European Patent Application EP 4 763 977 A1, published June 24, 2026. Title: EXTRACELLULAR VESICLES. Applicant: Fairway Lab AG. The sequence listing filed with the application follows.

SEQUENCE LISTING (56 sequences)

SEQ ID NO: 1 - DNA, 2409 bp, synthetic construct
  source 1..2409: mol_type = other DNA
atggatgagacctccccaaggctggaagaagactggaaaaaagtacttcagcgagaagcaggctggcagtgtgctgctctggttggtgaagaccagcctctttgcccagatcttcctgaacttgatctttctgaactagatgtgaacgacttggatacagacagctttctgggtggactcaagtggtgcagtgaccaatcagaaataatatccaatcagtacaacaatgagccttcaaacatatttgagaagatagatgaagagaatgaggcaaacttgctagcagtcctcacagagacactagacagtctccctgtggatgaagacggattgccctcatttgatgcgctgacagatggagacgtgaccactgacaatgaggctagtccttcctccatgcctgacggcacccctccaccccaggaggcagaagagccgtctctacttaagaagctcttactggcaccagccaacactcagctaagttataatgaatgcagtggtctcagtacccagaaccatgcaaatcacaatcacaggatcagaacaaaccctgcaattgttaagactgagaattcatggagcaataaagcgaagagtatttgtcaacagcaaaagccacaaagacgtccctgctcggagcttctcaaatatctgaccacaaacgatgaccctcctcacaccaaacccacagagaacagaaacagcagcagagacaaatgcacctccaaaaagaagtcccacacacagtcgcagtcacaacacttacaagccaaaccaacaactttatctcttcctctgaccccagagtcaccaaatgaccccaagggttccccatttgagaacaagactattgaacgcaccttaagtgtggaactctctggaactgcaggcctaactccacccaccactcctcctcataaagccaaccaagataacccttttagggcttctccaaagctgaagtcctcttgcaagactgtggtgccaccaccatcaaagaagcccaggtacagtgagtcttctggtacacaaggcaataactccaccaagaaagggccggagcaatccgagttgtatgcacaactcagcaagtcctcagtcctcactggtggacacgaggaaaggaagaccaagcggcccagtctgcggctgtttggtgaccatgactattgccagtcaattaattccaaaacagaaatactcattaatatatcacaggagctccaagactctagacaactagaaaataaagatgtctcctctgattggcaggggcagatttgttcttccacagattcagaccagtgctacctgagagagactttggaggcaagcaagcaggtctctccttgcagcacaagaaaacagctccaagaccaggaaatccgagccgagctgaacaagcacttcggtcatcccagtcaagctgtttttgacgacgaagcagacaagaccggtgaactgagggacagtgatttcagtaatgaacaattctccaaactacctatgtttataaattcaggactagccatggatggcctgtttgatgacagcgaagatgaaagtgataaactgagctacccttgggatggcacgcaatcctattcattgttcaatgtgtctccttcttgttcttcttttaactctccatgtagagattctgtgtcaccacccaaatccttattttctcaaagaccccaaaggatgcgctctcgttcaaggtccttttctcgacacaggtcgtgttcccgatcaccatattccaggtcaagatcaaggtctccaggcagtagatcctcttcaagatcctgctattactatgagtcaagccactacagacaccgcacgcaccgaaattctcccttgtatgtgagatcacgttcaagatcgccctacagccgtcggcccaggtatgacagctacgaggaatatcagcacgagaggctgaagagggaagaatatcgcagagagtatgagaagcgagagtctgagagggccaagcaaagggagaggcagaggcagaaggcaattgaagagcgccgtgtgatttatgtcggtaaaatcagacctgacacaacacggacagaactgagggaccgttttgaagtttttggtgaaattgaggagtgcacagtaaatctgcgggatgatggagacagctatggtttcattacctaccgttatacctgtgatgcttttgctgctcttgaaaatggatacactttgcgcaggtcaaacgaaactgactttgagctgtacttttgtggacgcaagcaatttttcaagtctaactatgcagacctagattcaaactcagatgactttgaccctgcttccaccaagagcaagtatgactctctggattttgatagtttactgaaagaagctcagagaagcttgcgcagg

SEQ ID NO: 2 - DNA, 3069 bp, synthetic construct
  source 1..3069: mol_type = other DNA
atggcggggaacgactgcggcgcgctgctggacgaagagctctcctccttcttcctcaactatctcgctgacacgcagggtggagggtccggggaggagcaactctatgctgactttccagaacttgacctctcccagctggatgccagcgactttgactcggccacctgctttggggagctgcagtggtgcccagagaactcagagactgaacccaaccagtacagccccgatgactccgagctcttccagattgacagtgagaatgaggccctcctggcagagctcaccaagaccctggatgacatccctgaagatgacgtgggtctggctgccttcccagccctggatggtggagacgctctatcatgcacctcagcttcgcctgccccctcatctgcaccccccagccctgccccggagaagccctcggccccagcccctgaggtggacgagctctcactgctgcagaagctcctcctggccacatcctacccaacatcaagctctgacacccagaaggaagggaccgcctggcgccaggcaggcctcagatctaaaagtcaacggccttgtgttaaggcggacagcacccaagacaagaaggctcccatgatgcagtctcagagccgaagttgtacagaactacataagcacctcacctcggcacagtgctgcctgcaggatcggggtctgcagccaccatgcctccagagtccccggctccctgccaaggaggacaaggagccgggtgaggactgcccgagcccccagccagctccagcctctccccgggactccctagctctgggcagggcagaccccggtgccccggtttcccaggaagacatgcaggcgatggtgcaactcatacgctacatgcacacctactgcctcccccagaggaagctgcccccacagacccctgagccactccccaaggcctgcagcaacccctcccagcaggtcagatcccggccctggtcccggcaccactccaaagcctcctgggctgagttctccattctgagggaacttctggctcaagacgtgctctgtgatgtcagcaaaccctaccgtctggccacgcctgtttatgcctccctcacacctcggtcaaggcccaggccccccaaagacagtcaggcctcccctggtcgcccgtcctcggtggaggaggtaaggatcgcagcttcacccaagagcaccgggcccagaccaagcctgcgcccactgcggctggaggtgaaaagggaggtccgccggcctgccagactgcagcagcaggaggaggaagacgaggaagaagaggaggaggaagaggaagaagaaaaagaggaggaggaggagtggggcaggaaaaggccaggccgaggcctgccatggacgaagctggggaggaagctggagagctctgtgtgccccgtgcggcgttctcggagactgaaccctgagctgggcccctggctgacatttgcagatgagccgctggtcccctcggagccccaaggtgctctgccctcactgtgcctggctcccaaggcctacgacgtagagcgggagctgggcagccccacggacgaggacagtggccaagaccagcagctcctacggggaccccagatccctgccctggagagcccctgtgagagtgggtgtggggacatggatgaggaccccagctgcccgcagctccctcccagagactctcccaggtgcctcatgctggccttgtcacaaagcgacccaacttttggcaagaagagctttgagcagaccttgacagtggagctctgtggcacagcaggactcaccccacccaccacaccaccgtacaagcccacagaggaggatcccttcaaaccagacatcaagcatagtctaggcaaagaaatagctctcagcctcccctcccctgagggcctctcactcaaggccaccccaggggctgcccacaagctgccaaagaagcacccagagcgaagtgagctcctgtcccacctgcgacatgccacagcccagccagcctcccaggctggccagaagcgtcccttctcctgttcctttggagaccatgactactgccaggtgctccgaccagaaggcgtcctgcaaaggaaggtgctgaggtcctgggagccgtctggggttcaccttgaggactggccccagcagggtgccccttgggctgaggcacaggcccctggcagggaggaagacagaagctgtgatgctggcgccccacccaaggacagcacgctgctgagagaccatgagatccgtgccagcctcaccaaacactttgggctgctggagaccgccctggaggaggaagacctggcctcctgcaagagccctgagtatgacactgtctttgaagacagcagcagcagcagcggcgagagcagcttcctcccagaggaggaagaggaagaaggggaggaggaggaggaggacgatgaagaagaggactcaggggtcagccccacttgctctgaccactgcccctaccagagcccaccaagcaaggccaaccggcagctctgttcccgcagccgctcaagctctggctcttcaccctgccactcctggtcaccagccactcgaaggaacttcagatgtgagagcagagggccgtgttcagacagaacgccaagcatccggcacgccaggaagcggcgggaaaaggccattggggaaggccgcgtggtgtacattcaaaatctctccagcgacatgagctcccgagagctgaagaggcgctttgaagtgtttggtgagattgaggagtgcgaggtgctgacaagaaataggagaggcgagaagtacggcttcatcacctaccggtgttctgagcacgcggccctctctttgacaaagggcgctgccctgaggaagcgcaacgagccctccttccagctgagctacggagggctccggcacttctgctggcccagatacactgactacgattccaattcagaagaggcccttcctgcgtcagggaaaagcaagtatgaagccatggattttgacagcttactgaaagaggcccagcagagcctgcat

SEQ ID NO: 3 - DNA, 3396 bp, synthetic construct
  source 1..3396: mol_type = other DNA
atgccgcgcgctccccgctgccgagccgtgcgctccctgctgcgcagccactaccgcgaggtgctgccgctggccacgttcgtgcggcgcctggggccccagggctggcggctggtgcagcgcggggacccggcggctttccgcgcgctggtggcccagtgcctggtgtgcgtgccctgggacgcacggccgccccccgccgccccctccttccgccaggtgtcctgcctgaaggagctggtggcccgagtgctgcagaggctgtgcgagcgcggcgcgaagaacgtgctggccttcggcttcgcgctgctggacggggcccgcgggggcccccccgaggccttcaccaccagcgtgcgcagctacctgcccaacacggtgaccgacgcactgcgggggagcggggcgtgggggctgctgctgcgccgcgtgggcgacgacgtgctggttcacctgctggcacgctgcgcgctctttgtgctggtggctcccagctgcgcctaccaggtgtgcgggccgccgctgtaccagctcggcgctgccactcaggcccggcccccgccacacgctagtggaccccgaaggcgtctgggatgcgaacgggcctggaaccatagcgtcagggaggccggggtccccctgggcctgccagccccgggtgcgaggaggcgcgggggcagtgccagccgaagtctgccgttgcccaagaggcccaggcgtggcgctgcccctgagccggagcggacgcccgttgggcaggggtcctgggcccacccgggcaggacgcgtggaccgagtgaccgtggtttctgtgtggtgtcacctgccagacccgccgaagaagccacctctttggagggtgcgctctctggcacgcgccactcccacccatccgtgggccgccagcaccacgcgggccccccatccacatcgcggccaccacgtccctgggacacgccttgtcccccggtgtacgccgagaccaagcacttcctctactcctcaggcgacaaggagcagctgcggccctccttcctactcagctctctgaggcccagcctgactggcgctcggaggctcgtggagaccatctttctgggttccaggccctggatgccagggactccccgcaggttgccccgcctgccccagcgctactggcaaatgcggcccctgtttctggagctgcttgggaaccacgcgcagtgcccctacggggtgctcctcaagacgcactgcccgctgcgagctgcggtcaccccagcagccggtgtctgtgcccgggagaagccccagggctctgtggcggcccccgaggaggaggacacagacccccgtcgcctggtgcagctgctccgccagcacagcagcccctggcaggtgtacggcttcgtgcgggcctgcctgcgccggctggtgcccccaggcctctggggctccaggcacaacgaacgccgcttcctcaggaacaccaagaagttcatctccctggggaagcatgccaagctctcgctgcaggagctgacgtggaagatgagcgtgcgggactgcgcttggctgcgcaggagcccaggggttggctgtgttccggccgcagagcaccgtctgcgtgaggagatcctggccaagttcctgcactggctgatgagtgtgtacgtcgtcgagctgctcaggtctttcttttatgtcacggagaccacgtttcaaaagaacaggctctttttctaccggaagagtgtctggagcaagttgcaaagcattggaatcagacagcacttgaagagggtgcagctgcgggagctgtcggaagcagaggtcaggcagcatcgggaagccaggcccgccctgctgacgtccagactccgcttcatccccaagcctgacgggctgcggccgattgtgaacatggactacgtcgtgggagccagaacgttccgcagagaaaagagggccgagcgtctcacctcgagggtgaaggcactgttcagcgtgctcaactacgagcgggcgcggcgccccggcctcctgggcgcctctgtgctgggcctggacgatatccacagggcctggcgcaccttcgtgctgcgtgtgcgggcccaggacccgccgcctgagctgtactttgtcaaggtggatgtgacgggcgcgtacgacaccatcccccaggacaggctcacggaggtcatcgccagcatcatcaaaccccagaacacgtactgcgtgcgtcggtatgccgtggtccagaaggccgcccatgggcacgtccgcaaggccttcaagagccacgtctctaccttgacagacctccagccgtacatgcgacagttcgtggctcacctgcaggagaccagcccgctgagggatgccgtcgtcatcgagcagagctcctccctgaatgaggccagcagtggcctcttcgacgtcttcctacgcttcatgtgccaccacgccgtgcgcatcaggggcaagtcctacgtccagtgccaggggatcccgcagggctccatcctctccacgctgctctgcagcctgtgctacggcgacatggagaacaagctgtttgcggggattcggcgggacgggctgctcctgcgtttggtggatgatttcttgttggtgacacctcacctcacccacgcgaaaaccttcctcaggaccctggtccgaggtgtccctgagtatggctgcgtggtgaacttgcggaagacagtggtgaacttccctgtagaagacgaggccctgggtggcacggcttttgttcagatgccggcccacggcctattcccctggtgcggcctgctgctggatacccggaccctggaggtgcagagcgactactccagctatgcccggacctccatcagagccagtctcaccttcaaccgcggcttcaaggctgggaggaacatgcgtcgcaaactctttggggtcttgcggctgaagtgtcacagcctgtttctggatttgcaggtgaacagcctccagacggtgtgcaccaacatctacaagatcctcctgctgcaggcgtacaggtttcacgcatgtgtgctgcagctcccatttcatcagcaagtttggaagaaccccacatttttcctgcgcgtcatctctgacacggcctccctctgctactccatcctgaaagccaagaacgcagggatgtcgctgggggccaagggcgccgccggccctctgccctccgaggccgtgcagtggctgtgccaccaagcattcctgctcaagctgactcgacaccgtgtcacctacgtgccactcctggggtcactcaggacagcccagacgcagctgagtcggaagctcccggggacgacgctgactgccctggaggccgcagccaacccggcactgccctcagacttcaagaccatcctggac

SEQ ID NO: 4 - DNA, 313 bp, synthetic construct
  source 1..313: mol_type = other DNA
ttaaccctagaaagatagtctgcgtaaaattgacgcatgcattcttgaaatattgctctctctttctaaatagcgcgaatccgtcgctgtgcatttaggacatctcagtcgccgcttggagctcccgtgaggcgtgcttgtcaatgcggtaagtgtcactgattttgaactataacgaccgcgtgagtcaaaatgacgcatgattatcttttacgtgacttttaagatttaactcatacgataattatattgttatttcatgttctacttacgtgataacttattatatatatattttcttgttatagatatc

SEQ ID NO: 5 - DNA, 235 bp, synthetic construct
  source 1..235: mol_type = other DNA
ttaaccctagaaagataatcatattgtgacgtacgttaaagataatcatgcgtaaaattgacgcatgtgttttatcggtctgtatatcgaggtttatttattaatttgaatagatattaagttttattatatttacacttacatactaataataaattcaacaaacaatttatttatgtttatttatttattaaaaaaaaacaaaaactcaaaatttcttctataaagtaacaaa

SEQ ID NO: 6 - DNA, 1176 bp, synthetic construct
  source 1..1176: mol_type = other DNA
ggctccggtgcccgtcagtgggcagagcgcacatcgcccacagtccccgagaagttggggggaggggtcggcaattgaaccggtgcctagagaaggtggcgcggggtaaactgggaaagtgatgtcgtgtactggctccgcctttttcccgagggtgggggagaaccgtatataagtgcagtagtcgccgtgaacgttctttttcgcaacgggtttgccgccagaacacaggtaagtgccgtgtgtggttcccgcgggcctggcctctttacgggttatggcccttgcgtgccttgaattacttccacctggctgcagtacgtgattcttgatcccgagcttcgggttggaagtgggtgggagagttcgaggccttgcgcttaaggagccccttcgcctcgtgcttgagttgaggcctggcctgggcgctggggccgccgcgtgcgaatctggtggcaccttcgcgcctgtctcgctgctttcgataagtctctagccatttaaaatttttgatgacctgctgcgacgctttttttctggcaagatagtcttgtaaatgcgggccaagatctgcacactggtatttcggtttttggggccgcgggcggcgacggggcccgtgcgtcccagcgcacatgttcggcgaggcggggcctgcgagcgcggccaccgagaatcggacgggggtagtctcaagctggccggcctgctctggtgcctggtctcgcgccgccgtgtatcgccccgccctgggcggcaaggctggcccggtcggcaccagttgcgtgagcggaaagatggccgcttcccggccctgctgcagggagctcaaaatggaggacgcggcgctcgggagagcgggcgggtgagtcacccacacaaaggaaaagggcctttccgtcctcagccgtcgcttcatgtgactccacggagtaccgggcgccgtccaggcacctcgattagttctcgagcttttggagtacgtcgtctttaggttggggggaggggttttatgcgatggagtttccccacactgagtgggtggagactgaagttaggccagcttggcacttgatgtaattctccttggaatttgccctttttgagtttggatcttggttcattctcaagcctcagacagtggttcaaagtttttttcttccatttcaggtgtcg

SEQ ID NO: 7 - DNA, 588 bp, cytomegalovirus humanbeta5
  source 1..588: mol_type = genomic DNA
gttgacattgattattgactagttattaatagtaatcaattacggggtcattagttcatagcccatatatggagttccgcgttacataacttacggtaaatggcccgcctggctgaccgcccaacgacccccgcccattgacgtcaataatgacgtatgttcccatagtaacgccaatagggactttccattgacgtcaatgggtggagtatttacggtaaactgcccacttggcagtacatcaagtgtatcatatgccaagtacgccccctattgacgtcaatgacggtaaatggcccgcctggcattatgcccagtacatgaccttatgggactttcctacttggcagtacatctacgtattagtcatcgctattaccatggtgatgcggttttggcagtacatcaatgggcgtggatagcggtttgactcacggggatttccaagtctccaccccattgacgtcaatgggagtttgttttggcaccaaaatcaacgggactttccaaaatgtcgtaacaactccgccccattgacgcaaatgggcggtaggcgtgtacggtgggaggtctatataagcagagctc

SEQ ID NO: 8 - DNA, 1242 bp, synthetic construct
  source 1..1242: mol_type = other DNA
gacattgattattgactagttattaatagtaatcaattacggggtcattagttcatagcccatatatggagttccgcgttacataacttacggtaaatggcccgcctggctgaccgcccaacgacccccgcccattgacgtcaataatgacgtatgttcccatagtaacgccaatagggactttccattgacgtcaatgggtggagtatttacggtaaactgcccacttggcagtacatcaagtgtatcatatgccaagtacgccccctattgacgtcaatgacggtaaatggcccgcctggcattatgcccagtacatgaccttatgggactttcctacttggcagtacatctacgtattagtcatcgctattaccatggtgatgcggttttggcagtacatcaatgggcgtggatagcggtttgactcacggggatttccaagtctccaccccattgacgtcaatgggagtttgttttggcaccaaaatcaacgggactttccaaaatgtcgtaacaactccgccccattgacgcaaatgggcggtaggcgtgtacggtgggaggtctatataagcagagctcgtttagtgaaccgtcagatcgcctggagacgccatccacgctgttttgacctccatagaagacaccgggaccgatccagcctcccctcgaagcttacatgtggtaccgagctcggatcctgagaacttcagggtgagtctatgggacccttgatgttttctttccccttcttttctatggttaagttcatgtcataggaaggggagaagtaacagggtacacatattgaccaaatcagggtaattttgcatttgtaattttaaaaaatgctttcttcttttaatatacttttttgtttatcttatttctaatactttccctaatctctttctttcagggcaataatgatacaatgtatcatgcctctttgcaccattctaaagaataacagtgataatttctgggttaaggcaatagcaatatttctgcatataaatatttctgcatataaattgtaactgatgtaagaggtttcatattgctaatagcagctacaatccagctaccattctgcttttattttatggttgggataaggctggattattctgagtccaagctaggcccttttgctaatcatgttcatacctcttatcttcctcccacagctcctgggcaacgtgctggtctgtgtgctggcccatcactttggcaaag

SEQ ID NO: 9 - DNA, 1733 bp, synthetic construct
  source 1..1733: mol_type = other DNA
ctcgacattgattattgactagttattaatagtaatcaattacggggtcattagttcatagcccatatatggagttccgcgttacataacttacggtaaatggcccgcctggctgaccgcccaacgacccccgcccattgacgtcaataatgacgtatgttcccatagtaacgccaatagggactttccattgacgtcaatgggtggagtatttacggtaaactgcccacttggcagtacatcaagtgtatcatatgccaagtacgccccctattgacgtcaatgacggtaaatggcccgcctggcattatgcccagtacatgaccttatgggactttcctacttggcagtacatctacgtattagtcatcgctattaccatggtcgaggtgagccccacgttctgcttcactctccccatctcccccccctccccacccccaattttgtatttatttattttttaattattttgtgcagcgatgggggcggggggggggggggggcgcgcgccaggcggggcggggcggggcgaggggcggggcggggcgaggcggagaggtgcggcggcagccaatcagagcggcgcgctccgaaagtttccttttatggcgaggcggcggcggcggcggccctataaaaagcgaagcgcgcggcgggcgggagtcgctgcgcgctgccttcgccccgtgccccgctccgccgccgcctcgcgccgcccgccccggctctgactgaccgcgttactcccacaggtgagcgggcgggacggcccttctcctccgggctgtaattagcgcttggtttaatgacggcttgtttcttttctgtggctgcgtgaaagccttgaggggctccgggagggccctttgtgcggggggagcggctcggggggtgcgtgcgtgtgtgtgtgcgtggggagcgccgcgtgcggctccgcgctgcccggcggctgtgagcgctgcgggcgcggcgcggggctttgtgcgctccgcagtgtgcgcgaggggagcgcggccgggggcggtgccccgcggtgcggggggggctgcgaggggaacaaaggctgcgtgcggggtgtgtgcgtgggggggtgagcagggggtgtgggcgcgtcggtcgggctgcaaccccccctgcacccccctccccgagttgctgagcacggcccggcttcgggtgcggggctccgtacggggcgtggcgcggggctcgccgtgccgggcggggggtggcggcaggtgggggtgccgggcggggcggggccgcctcgggccggggagggctcgggggaggggcgcggcggcccccggagcgccggcggctgtcgaggcgcggcgagccgcagccattgccttttatggtaatcgtgcgagagggcgcagggacttcctttgtcccaaatctgtgcggagccgaaatctgggaggcgccgccgcaccccctctagcgggcgcggggcgaagcggtgcggcgccggcaggaaggaaatgggcggggagggccttcgtgcgtcgccgcgccgccgtccccttctccctctccagcctcggggctgtccgcggggggacggctgccttcgggggggacggggcagggcggggttcggcttctggcgtgtgaccggcggctctagagcctctgctaaccatgttcatgccttcttctttttcctacagctcctgggcaacgtgctggttattgtgctgtctcatcattttggcaaagaattg

SEQ ID NO: 10 - DNA, 505 bp, Homo sapiens
  source 1..505: mol_type = genomic DNA
gggttgcgccttttccaaggcagccctgggtttgcgcagggacgcggctgctctgggcgtggttccgggaaacgcagcggcgccgaccctgggtctcgcacattcttcacgtccgttcgcagcgtcacccggatcttcgccgctacccttgtgggccccccggcgacgcttcctgctccgcccctaagtcgggaaggttccttgcggttcgcggcgtgccggacgtgacaaacggaagccgcacgtctcactagtaccctcgcagacggacagcgccagggagcaatggcagcgcgccgaccgcgatgggctgtggccaatagcggctgctcagcagggcgcgccgagagcagcggccgggaaggggcggtgcgggaggcggggtgtggggcggtagtgtgggccctgttcctgcccgcgcggtgttccgcattctgcaagcctccggagcgcacgtcggcagtcggctccctcgttgaccgaatcaccgacctctctccccagg

SEQ ID NO: 11 - DNA, 222 bp, Macaca mulatta polyomavirus 1
  source 1..222: mol_type = genomic DNA
cagacatgataagatacattgatgagtttggacaaaccacaactagaatgcagtgaaaaaaatgctttatttgtgaaatttgtgatgctattgctttatttgtaaccattataagctgcaataaacaagttaacaacaacaattgcattcattttatgtttcaggttcagggggaggtgtgggaggttttttaaagcaagtaaaacctctacaaatgtggta

SEQ ID NO: 12 - DNA, 522 bp, synthetic construct
  source 1..522: mol_type = other DNA
tcctcaggtgcaggctgcctatcagaaggtggtggctggtgtggccaatgccctggctcacaaataccactgagatctttttccctctgccaaaaattatggggacatcatgaagccccttgagcatctgacttctggctaataaaggaaatttattttcattgcaatagtgtgttggaattttttgtgtctctcactcggaaggacatatgggagggcaaatcatttaaaacatcagaatgagtatttggtttagagtttggcaacatatgcccatatgctggctgccatgaacaaaggttggctataaagaggtcatcagtatatgaaacagccccctgctgtccattccttattccatagaaaagccttgacttgaggttagattttttttatattttgttttgtgttatttttttctttaacatccctaaaattttccttacatgttttactagccagatttttcctcctctcctgactactcccagtcatagctgtccctcttctcttatggagatc

SEQ ID NO: 13 - skipped

SEQ ID NO: 14 - protein, 18 aa, Thosea asigna virus
EGRGSLLTCGDVEENPGP

SEQ ID NO: 15 - protein, 19 aa, Teschovirus A
ATNFSLLKQAGDVEENPGP

SEQ ID NO: 16 - protein, 20 aa, Equine rhinitis A virus
QCTNYALLKLAGDVESNPGP

SEQ ID NO: 17 - protein, 22 aa, Foot-and-mouth disease virus
VKQTLNFDLLKLAGDVESNPGP

SEQ ID NO: 18 - DNA, 63 bp, Thosea asigna virus
  source 1..63: mol_type = genomic DNA
ggaagcggagagggcaggggaagtcttctaacatgcggggacgtggaggaaaatcccggcccc

SEQ ID NO: 19 - DNA, 66 bp, Teschovirus A
  source 1..66: mol_type = genomic DNA
ggaagcggagccacgaacttctctctgttaaagcaagcaggagatgttgaagaaaaccccgggcct

SEQ ID NO: 20 - DNA, 69 bp, Equine rhinitis A virus
  source 1..69: mol_type = genomic DNA
ggaagcggacagtgtactaattatgctctcttgaaattggctggagatgttgagagcaacccaggtccc

SEQ ID NO: 21 - DNA, 75 bp, Foot-and-mouth disease virus
  source 1..75: mol_type = genomic DNA
ggaagcggagtgaaacagactttgaattttgaccttctgaagttggcaggagacgttgagtccaaccctgggccc

SEQ ID NO: 22 - DNA, 225 bp, synthetic construct
  source 1..225: mol_type = other DNA
ctgtgccttctagttgccagccatctgttgtttgcccctcccccgtgccttccttgaccctggaaggtgccactcccactgtcctttcctaataaaatgaggaaattgcatcgcattgtctgagtaggtgtcattctattctggggggtggggtggggcaggacagcaagggggaggattgggaagacaatagcaggcatgctggggatgcggtgggctctatgg

SEQ ID NO: 23 - DNA, 597 bp, synthetic construct
  source 1..597: mol_type = other DNA
atgaccgagtacaagcccacggtgcgcctcgccacccgcgacgacgtccccagggccgtacgcaccctcgccgccgcgttcgccgactaccccgccacgcgccacaccgtcgatccggaccgccacatcgagcgggtcaccgagctgcaagaactcttcctcacgcgcgtcgggctcgacatcggcaaggtgtgggtcgcggacgacggcgccgcggtggcggtctggaccacgccggagagcgtcgaagcgggggcggtgttcgccgagatcggcccgcgcatggccgagttgagcggttcccggctggccgcgcagcaacagatggaaggcctcctggcgccgcaccggcccaaggagcccgcgtggttcctggccaccgtcggcgtctcgcccgaccaccagggcaagggtctgggcagcgccgtcgtgctccccggagtggaggcggccgagcgcgccggggtgcccgccttcctggagacctccgcgccccgcaacctccccttctacgagcggctcggcttcaccgtcaccgccgacgtcgaggtgcccgaaggaccgcgcacctggtgcatgacccgcaagcccggtgcc

SEQ ID NO: 24 - DNA, 858 bp, synthetic construct
  source 1..858: mol_type = other DNA
atgagtattcaacatttccgtgtcgcccttattcccttttttgcggcattttgccttcctgtttttgctcacccagaaacgctggtgaaagtaaaagatgctgaagatcagttgggtgcacgagtgggttacatcgaactggatctcaacagcggtaagatccttgagagttttcgccccgaagaacgttttccaatgatgagcacttttaaagttctgctatgtggcgcggtattatcccgtattgacgccgggcaagagcaactcggtcgccgcatacactattctcagaatgacttggttgagtactcaccagtcacagaaaagcatcttacggatggcatgacagtaagagaattatgcagtgctgccataaccatgagtgataacactgcggccaacttacttctgacaacgatcggaggaccgaaggagctaaccgcttttttgcacaacatgggggatcatgtaactcgccttgatcgttgggaaccggagctgaatgaagccataccaaacgacgagcgtgacaccacgatgcctgtagcaatggcaacaacgttgcgcaaactattaactggcgaactacttactctagcttcccggcaacaattaatagactggatggaggcggataaagttgcaggaccacttctgcgctcggcccttccggctggctggtttattgctgataaatctggagccggtgagcgtgggtctcgcggtatcattgcagcactggggccagatggtaagccctcccgtatcgtagttatctacacgacggggagtcaggcaactatggatgaacgaaatagacagatcgctgagataggtgcctcactgattaagcattgg

SEQ ID NO: 25 - DNA, 589 bp, synthetic construct
  source 1..589: mol_type = other DNA
ttgagatcctttttttctgcgcgtaatctgctgcttgcaaacaaaaaaaccaccgctaccagcggtggtttgtttgccggatcaagagctaccaactctttttccgaaggtaactggcttcagcagagcgcagataccaaatactgttcttctagtgtagccgtagttaggccaccacttcaagaactctgtagcaccgcctacatacctcgctctgctaatcctgttaccagtggctgctgccagtggcgataagtcgtgtcttaccgggttggactcaagacgatagttaccggataaggcgcagcggtcgggctgaacggggggttcgtgcacacagcccagcttggagcgaacgacctacaccgaactgagatacctacagcgtgagctatgagaaagcgccacgcttcccgaagggagaaaggcggacaggtatccggtaagcggcagggtcggaacaggagagcgcacgagggagcttccagggggaaacgcctggtatctttatagtcctgtcgggtttcgccacctctgacttgagcgtcgatttttgtgatgctcgtcaggggggcggagcctatggaaa

SEQ ID NO: 26 - DNA, 717 bp, synthetic construct
  source 1..717: mol_type = other DNA
atggtgagcaagggcgaggagctgttcaccggggtggtgcccatcctggtcgagctggacggcgacgtaaacggccacaagttcagcgtgtccggcgagggcgagggcgatgccacctacggcaagctgaccctgaagttcatctgcaccaccggcaagctgcccgtgccctggcccaccctcgtgaccaccctgacctacggcgtgcagtgcttcagccgctaccccgaccacatgaagcagcacgacttcttcaagtccgccatgcccgaaggctacgtccaggagcgcaccatcttcttcaaggacgacggcaactacaagacccgcgccgaggtgaagttcgagggcgacaccctggtgaaccgcatcgagctgaagggcatcgacttcaaggaggacggcaacatcctggggcacaagctggagtacaactacaacagccacaacgtctatatcatggccgacaagcagaagaacggcatcaaggtgaacttcaagatccgccacaacatcgaggacggcagcgtgcagctcgccgaccactaccagcagaacacccccatcggcgacggccccgtgctgctgcccgacaaccactacctgagcacccagtccgccctgagcaaagaccccaacgagaagcgcgatcacatggtcctgctggagttcgtgaccgccgccgggatcactctcggcatggacgagctgtacaag

SEQ ID NO: 27 - DNA, 1650 bp, synthetic construct
  source 1..1650: mol_type = other DNA
atggaagacgccaaaaacataaagaaaggcccggcgccattctatccgctagaggatggaaccgctggagagcaactgcataaggctatgaagagatacgccctggttcctggaacaattgcttttacagatgcacatatcgaggtgaacatcacgtacgcggaatacttcgaaatgtccgttcggttggcagaagctatgaaacgatatgggctgaatacaaatcacagaatcgtcgtatgcagtgaaaactctcttcaattctttatgccggtgttgggcgcgttatttatcggagttgcagttgcgcccgcgaacgacatttataatgaacgtgaattgctcaacagtatgaacatttcgcagcctaccgtagtgtttgtttccaaaaaggggttgcaaaaaattttgaacgtgcaaaaaaaattaccaataatccagaaaattattatcatggattctaaaacggattaccagggatttcagtcgatgtacacgttcgtcacatctcatctacctcccggttttaatgaatacgattttgtaccagagtcctttgatcgtgacaaaacaattgcactgataatgaactcctctggatctactgggttacctaagggtgtggcccttccgcatagaactgcctgcgtcagattctcgcatgccagagatcctatttttggcaatcaaatcattccggatactgcgattttaagtgttgttccattccatcacggttttggaatgtttactacactcggatatttgatatgtggatttcgagtcgtcttaatgtatagatttgaagaagagctgtttttacgatcccttcaggattacaaaattcaaagtgcgttgctagtaccaaccctattttcattcttcgccaaaagcactctgattgacaaatacgatttatctaatttacacgaaattgcttctgggggcgcacctctttcgaaagaagtcggggaagcggttgcaaaacgcttccatcttccagggatacgacaaggatatgggctcactgagactacatcagctattctgattacacccgagggggatgataaaccgggcgcggtcggtaaagttgttccattttttgaagcgaaggttgtggatctggataccgggaaaacgctgggcgttaatcagagaggcgaattatgtgtcagaggacctatgattatgtccggttatgtaaacaatccggaagcgaccaacgccttgattgacaaggatggatggctacattctggagacatagcttactgggacgaagacgaacacttcttcatagttgaccgcttgaagtctttaattaaatacaaaggataccaggtggcccccgctgaattggagtcgatattgttacaacaccccaacatcttcgacgcgggcgtggcaggtcttcccgacgatgacgccggtgaacttcccgccgccgttgttgttttggagcacggaaagacgatgacggaaaaagagatcgtggattacgtcgccagtcaagtaacaaccgcgaaaaagttgcgcggaggagttgtgtttgtggacgaagtaccgaaaggtcttaccggaaaactcgacgcaagaaaaatcagagagatcctcataaaggccaagaagggcggaaagtccaaattg

SEQ ID NO: 28 - DNA, 708 bp, synthetic construct
  source 1..708: mol_type = other DNA
atggtgagcaagggcgaggaggataacatggccatcatcaaggagttcatgcgcttcaaggtgcacatggagggctccgtgaacggccacgagttcgagatcgagggcgagggcgagggccgcccctacgagggcacccagaccgccaagctgaaggtgaccaagggtggccccctgcccttcgcctgggacatcctgtcccctcagttcatgtacggctccaaggcctacgtgaagcaccccgccgacatccccgactacttgaagctgtccttccccgagggcttcaagtgggagcgcgtgatgaacttcgaggacggcggcgtggtgaccgtgacccaggactcctccctgcaggacggcgagttcatctacaaggtgaagctgcgcggcaccaacttcccctccgacggccccgtaatgcagaagaagaccatgggctgggaggcctcctccgagcggatgtaccccgaggacggcgccctgaagggcgagatcaagcagaggctgaagctgaaggacggcggccactacgacgctgaggtcaagaccacctacaaggccaagaagcccgtgcagctgcccggcgcctacaacgtcaacatcaagttggacatcacctcccacaacgaggactacaccatcgtggaacagtacgaacgcgccgagggccgccactccaccggcggcatggacgagctgtacaag

SEQ ID NO: 29 - DNA, 1782 bp, Trichoplusia ni
  source 1..1782: mol_type = genomic DNA
atgggtagttctttagacgatgagcatatcctctctgctcttctgcaaagcgatgacgagcttgttggtgaggattctgacagtgaaatatcagatcacgtaagtgaagatgacgtccagagcgatacagaagaagcgtttatagatgaggtacatgaagtgcagccaacgtcaagcggtagtgaaatattagacgaacaaaatgttattgaacaaccaggttcttcattggcttctaacagaatcttgaccttgccacagaggactattagaggtaagaataaacattgttggtcaacttcaaagtccacgaggcgtagccgagtctctgcactgaacattgtcagatctcaaagaggtccgacgcgtatgtgccgcaatatatatgacccacttttatgcttcaaactattttttactgatgagataatttcggaaattgtaaaatggacaaatgctgagatatcattgaaacgtcgggaatctatgacaggtgctacatttcgtgacacgaatgaagatgaaatctatgctttctttggtattctggtaatgacagcagtgagaaaagataaccacatgtccacagatgacctctttgatcgatctttgtcaatggtgtacgtctctgtaatgagtcgtgatcgttttgattttttgatacgatgtcttagaatggatgacaaaagtatacggcccacacttcgagaaaacgatgtatttactcctgttagaaaaatatgggatctctttatccatcagtgcatacaaaattacactccaggggctcatttgaccatagatgaacagttacttggttttagaggacggtgtccgtttaggatgtatatcccaaacaagccaagtaagtatggaataaaaatcctcatgatgtgtgacagtggtacgaagtatatgataaatggaatgccttatttgggaagaggaacacagaccaacggagtaccactcggtgaatactacgtgaaggagttatcaaagcctgtgcacggtagttgtcgtaatattacgtgtgacaattggttcacctcaatccctttggcaaaaaacttactacaagaaccgtataagttaaccattgtgggaaccgtgcgatcaaacaaacgcgagataccggaagtactgaaaaacagtcgctccaggccagtgggaacatcgatgttttgttttgacggaccccttactctcgtctcatataaaccgaagccagctaagatggtatacttattatcatcttgtgatgaggatgcttctatcaacgaaagtaccggtaaaccgcaaatggttatgtattataatcaaactaaaggcggagtggacacgctagaccaaatgtgttctgtgatgacctgcagtaggaagacgaataggtggcctatggcattattgtacggaatgataaacattgcctgcataaattcttttattatatacagccataatgtcagtagcaagggagaaaaggttcaaagtcgcaaaaaatttatgagaaacctttacatgagcctgacgtcatcgtttatgcgtaagcgtttagaagctcctactttgaagagatatttgcgcgataatatctctaatattttgccaaatgaagtgcctggtacatcagatgacagtactgaagagccagtaatgaaaaaacgtacttactgtacttactgcccctctaaaataaggcgaaaggcaaatgcatcgtgcaaaaaatgcaaaaaagttatttgtcgagagcataatattgatatgtgccaaagttgtttc

SEQ ID NO: 30 - DNA, 1782 bp, synthetic construct
  source 1..1782: mol_type = other DNA
atgggcagcagcctggacgacgagcacatcctgagcgccctgctgcagagcgacgacgagctggtcggcgaggacagcgacagcgaggtgagcgaccacgtgagcgaggacgacgtgcagtccgacaccgaggaggccttcatcgacgaggtgcacgaggtgcagcctaccagcagcggctccgagatcctggacgagcagaacgtgatcgagcagcccggcagctccctggccagcaacaggatcctgaccctgccccagaggaccatcaggggcaagaacaagcactgctggtccacctccaagcccaccaggcggagcagggtgtccgccctgaacatcgtgagaagccagaggggccccaccaggatgtgcaggaacatctacgaccccctgctgtgcttcaagctgttcttcaccgacgagatcatcagcgagatcgtgaagtggaccaacgccgagatcagcctgaagaggcgggagagcatgacctccgccaccttcagggacaccaacgaggacgagatctacgccttcttcggcatcctggtgatgaccgccgtgaggaaggacaaccacatgagcaccgacgacctgttcgacagatccctgagcatggtgtacgtgagcgtgatgagcagggacagattcgacttcctgatcagatgcctgaggatggacgacaagagcatcaggcccaccctgcgggagaacgacgtgttcacccccgtgagaaagatctgggacctgttcatccaccagtgcatccagaactacacccctggcgcccacctgaccatcgacgagcagctgctgggcttcaggggcaggtgccccttcagggtctatatccccaacaagcccagcaagtacggcatcaagatcctgatgatgtgcgacagcggcaccaagtacatgatcaacggcatgccctacctgggcaggggcacccagaccaacggcgtgcccctgggcgagtactacgtgaaggagctgtccaagcccgtccacggcagctgcagaaacatcacctgcgacaactggttcaccagcatccccctggccaagaacctgctgcaggagccctacaagctgaccatcgtgggcaccgtgagaagcaacaagagagagatccccgaggtcctgaagaacagcaggtccaggcccgtgggcaccagcatgttctgcttcgacggccccctgaccctggtgtcctacaagcccaagcccgccaagatggtgtacctgctgtccagctgcgacgaggacgccagcatcaacgagagcaccggcaagccccagatggtgatgtactacaaccagaccaagggcggcgtggacaccctggaccagatgtgcagcgtgatgacctgcagcagaaagaccaacaggtggcccatggccctgctgtacggcatgatcaacatcgcctgcatcaacagcttcatcatctacagccacaacgtgagcagcaagggcgagaaggtgcagagccggaaaaagttcatgcggaacctgtacatgggcctgacctccagcttcatgaggaagaggctggaggcccccaccctgaagagatacctgagggacaacatcagcaacatcctgcccaaagaggtgcccggcaccagcgacgacagcaccgaggagcccgtgatgaagaagaggacctactgcacctactgtcccagcaagatcagaagaaaggccagcgccagctgcaagaagtgtaagaaggtcatctgccgggagcacaacatcgacatgtgccagagctgtttc

SEQ ID NO: 31 - DNA, 17346 bp, synthetic construct
  source 1..17346: mol_type = other DNA
ttaaccctagaaagatagtctgcgtaaaattgacgcatgcattcttgaaatattgctctctctttctaaatagcgcgaatccgtcgctgtgcatttaggacatctcagtcgccgcttggagctcccgtgaggcgtgcttgtcaatgcggtaagtgtcactgattttgaactataacgaccgcgtgagtcaaaatgacgcatgattatcttttacgtgacttttaagatttaactcatacgataattatattgttatttcatgttctacttacgtgataacttattatatatatattttcttgttatagatatcatcaactttgtatagaaaagttgggctccggtgcccgtcagtgggcagagcgcacatcgcccacagtccccgagaagttggggggaggggtcggcaattgaaccggtgcctagagaaggtggcgcggggtaaactgggaaagtgatgtcgtgtactggctccgcctttttcccgagggtgggggagaaccgtatataagtgcagtagtcgccgtgaacgttctttttcgcaacgggtttgccgccagaacacaggtaagtgccgtgtgtggttcccgcgggcctggcctctttacgggttatggcccttgcgtgccttgaattacttccacctggctgcagtacgtgattcttgatcccgagcttcgggttggaagtgggtgggagagttcgaggccttgcgcttaaggagccccttcgcctcgtgcttgagttgaggcctggcctgggcgctggggccgccgcgtgcgaatctggtggcaccttcgcgcctgtctcgctgctttcgataagtctctagccatttaaaatttttgatgacctgctgcgacgctttttttctggcaagatagtcttgtaaatgcgggccaagatctgcacactggtatttcggtttttggggccgcgggcggcgacggggcccgtgcgtcccagcgcacatgttcggcgaggcggggcctgcgagcgcggccaccgagaatcggacgggggtagtctcaagctggccggcctgctctggtgcctggtctcgcgccgccgtgtatcgccccgccctgggcggcaaggctggcccggtcggcaccagttgcgtgagcggaaagatggccgcttcccggccctgctgcagggagctcaaaatggaggacgcggcgctcgggagagcgggcgggtgagtcacccacacaaaggaaaagggcctttccgtcctcagccgtcgcttcatgtgactccacggagtaccgggcgccgtccaggcacctcgattagttctcgagcttttggagtacgtcgtctttaggttggggggaggggttttatgcgatggagtttccccacactgagtgggtggagactgaagttaggccagcttggcacttgatgtaattctccttggaatttgccctttttgagtttggatcttggttcattctcaagcctcagacagtggttcaaagtttttttcttccatttcaggtgtcgtgacaagtttgtacaaaaaagcaggctgccaccatgccgcgcgctccccgctgccgagccgtgcgctccctgctgcgcagccactaccgcgaggtgctgccgctggccacgttcgtgcggcgcctggggccccagggctggcggctggtgcagcgcggggacccggcggctttccgcgcgctggtggcccagtgcctggtgtgcgtgccctgggacgcacggccgccccccgccgccccctccttccgccaggtgtcctgcctgaaggagctggtggcccgagtgctgcagaggctgtgcgagcgcggcgcgaagaacgtgctggccttcggcttcgcgctgctggacggggcccgcgggggcccccccgaggccttcaccaccagcgtgcgcagctacctgcccaacacggtgaccgacgcactgcgggggagcggggcgtgggggctgctgctgcgccgcgtgggcgacgacgtgctggttcacctgctggcacgctgcgcgctctttgtgctggtggctcccagctgcgcctaccaggtgtgcgggccgccgctgtaccagctcggcgctgccactcaggcccggcccccgccacacgctagtggaccccgaaggcgtctgggatgcgaacgggcctggaaccatagcgtcagggaggccggggtccccctgggcctgccagccccgggtgcgaggaggcgcgggggcagtgccagccgaagtctgccgttgcccaagaggcccaggcgtggcgctgcccctgagccggagcggacgcccgttgggcaggggtcctgggcccacccgggcaggacgcgtggaccgagtgaccgtggtttctgtgtggtgtcacctgccagacccgccgaagaagccacctctttggagggtgcgctctctggcacgcgccactcccacccatccgtgggccgccagcaccacgcgggccccccatccacatcgcggccaccacgtccctgggacacgccttgtcccccggtgtacgccgagaccaagcacttcctctactcctcaggcgacaaggagcagctgcggccctccttcctactcagctctctgaggcccagcctgactggcgctcggaggctcgtggagaccatctttctgggttccaggccctggatgccagggactccccgcaggttgccccgcctgccccagcgctactggcaaatgcggcccctgtttctggagctgcttgggaaccacgcgcagtgcccctacggggtgctcctcaagacgcactgcccgctgcgagctgcggtcaccccagcagccggtgtctgtgcccgggagaagccccagggctctgtggcggcccccgaggaggaggacacagacccccgtcgcctggtgcagctgctccgccagcacagcagcccctggcaggtgtacggcttcgtgcgggcctgcctgcgccggctggtgcccccaggcctctggggctccaggcacaacgaacgccgcttcctcaggaacaccaagaagttcatctccctggggaagcatgccaagctctcgctgcaggagctgacgtggaagatgagcgtgcgggactgcgcttggctgcgcaggagcccaggggttggctgtgttccggccgcagagcaccgtctgcgtgaggagatcctggccaagttcctgcactggctgatgagtgtgtacgtcgtcgagctgctcaggtctttcttttatgtcacggagaccacgtttcaaaagaacaggctctttttctaccggaagagtgtctggagcaagttgcaaagcattggaatcagacagcacttgaagagggtgcagctgcgggagctgtcggaagcagaggtcaggcagcatcgggaagccaggcccgccctgctgacgtccagactccgcttcatccccaagcctgacgggctgcggccgattgtgaacatggactacgtcgtgggagccagaacgttccgcagagaaaagagggccgagcgtctcacctcgagggtgaaggcactgttcagcgtgctcaactacgagcgggcgcggcgccccggcctcctgggcgcctctgtgctgggcctggacgatatccacagggcctggcgcaccttcgtgctgcgtgtgcgggcccaggacccgccgcctgagctgtactttgtcaaggtggatgtgacgggcgcgtacgacaccatcccccaggacaggctcacggaggtcatcgccagcatcatcaaaccccagaacacgtactgcgtgcgtcggtatgccgtggtccagaaggccgcccatgggcacgtccgcaaggccttcaagagccacgtctctaccttgacagacctccagccgtacatgcgacagttcgtggctcacctgcaggagaccagcccgctgagggatgccgtcgtcatcgagcagagctcctccctgaatgaggccagcagtggcctcttcgacgtcttcctacgcttcatgtgccaccacgccgtgcgcatcaggggcaagtcctacgtccagtgccaggggatcccgcagggctccatcctctccacgctgctctgcagcctgtgctacggcgacatggagaacaagctgtttgcggggattcggcgggacgggctgctcctgcgtttggtggatgatttcttgttggtgacacctcacctcacccacgcgaaaaccttcctcaggaccctggtccgaggtgtccctgagtatggctgcgtggtgaacttgcggaagacagtggtgaacttccctgtagaagacgaggccctgggtggcacggcttttgttcagatgccggcccacggcctattcccctggtgcggcctgctgctggatacccggaccctggaggtgcagagcgactactccagctatgcccggacctccatcagagccagtctcaccttcaaccgcggcttcaaggctgggaggaacatgcgtcgcaaactctttggggtcttgcggctgaagtgtcacagcctgtttctggatttgcaggtgaacagcctccagacggtgtgcaccaacatctacaagatcctcctgctgcaggcgtacaggtttcacgcatgtgtgctgcagctcccatttcatcagcaagtttggaagaaccccacatttttcctgcgcgtcatctctgacacggcctccctctgctactccatcctgaaagccaagaacgcagggatgtcgctgggggccaagggcgccgccggccctctgccctccgaggccgtgcagtggctgtgccaccaagcattcctgctcaagctgactcgacaccgtgtcacctacgtgccactcctggggtcactcaggacagcccagacgcagctgagtcggaagctcccggggacgacgctgactgccctggaggccgcagccaacccggcactgccctcagacttcaagaccatcctggactgactgtgccttctagttgccagccatctgttgtttgcccctcccccgtgccttccttgaccctggaaggtgccactcccactgtcctttcctaataaaatgaggaaattgcatcgcattgtctgagtaggtgtcattctattctggggggtggggtggggcaggacagcaagggggaggattgggaagacaatagcaggcatgctggggatgcggtgggctctatgggacattgattattgactagttattaatagtaatcaattacggggtcattagttcatagcccatatatggagttccgcgttacataacttacggtaaatggcccgcctggctgaccgcccaacgacccccgcccattgacgtcaataatgacgtatgttcccatagtaacgccaatagggactttccattgacgtcaatgggtggagtatttacggtaaactgcccacttggcagtacatcaagtgtatcatatgccaagtacgccccctattgacgtcaatgacggtaaatggcccgcctggcattatgcccagtacatgaccttatgggactttcctacttggcagtacatctacgtattagtcatcgctattaccatggtgatgcggttttggcagtacatcaatgggcgtggatagcggtttgactcacggggatttccaagtctccaccccattgacgtcaatgggagtttgttttggcaccaaaatcaacgggactttccaaaatgtcgtaacaactccgccccattgacgcaaatgggcggtaggcgtgtacggtgggaggtctatataagcagagctcgtttagtgaaccgtcagatcgcctggagacgccatccacgctgttttgacctccatagaagacaccgggaccgatccagcctcccctcgaagcttacatgtggtaccgagctcggatcctgagaacttcagggtgagtctatgggacccttgatgttttctttccccttcttttctatggttaagttcatgtcataggaaggggagaagtaacagggtacacatattgaccaaatcagggtaattttgcatttgtaattttaaaaaatgctttcttcttttaatatacttttttgtttatcttatttctaatactttccctaatctctttctttcagggcaataatgatacaatgtatcatgcctctttgcaccattctaaagaataacagtgataatttctgggttaaggcaatagcaatatttctgcatataaatatttctgcatataaattgtaactgatgtaagaggtttcatattgctaatagcagctacaatccagctaccattctgcttttattttatggttgggataaggctggattattctgagtccaagctaggcccttttgctaatcatgttcatacctcttatcttcctcccacagctcctgggcaacgtgctggtctgtgtgctggcccatcactttggcaaagacccagctttcttgtacaaagtgggccaccatggatgagacctccccaaggctggaagaagactggaaaaaagtacttcagcgagaagcaggctggcagtgtgctgctctggttggtgaagaccagcctctttgcccagatcttcctgaacttgatctttctgaactagatgtgaacgacttggatacagacagctttctgggtggactcaagtggtgcagtgaccaatcagaaataatatccaatcagtacaacaatgagccttcaaacatatttgagaagatagatgaagagaatgaggcaaacttgctagcagtcctcacagagacactagacagtctccctgtggatgaagacggattgccctcatttgatgcgctgacagatggagacgtgaccactgacaatgaggctagtccttcctccatgcctgacggcacccctccaccccaggaggcagaagagccgtctctacttaagaagctcttactggcaccagccaacactcagctaagttataatgaatgcagtggtctcagtacccagaaccatgcaaatcacaatcacaggatcagaacaaaccctgcaattgttaagactgagaattcatggagcaataaagcgaagagtatttgtcaacagcaaaagccacaaagacgtccctgctcggagcttctcaaatatctgaccacaaacgatgaccctcctcacaccaaacccacagagaacagaaacagcagcagagacaaatgcacctccaaaaagaagtcccacacacagtcgcagtcacaacacttacaagccaaaccaacaactttatctcttcctctgaccccagagtcaccaaatgaccccaagggttccccatttgagaacaagactattgaacgcaccttaagtgtggaactctctggaactgcaggcctaactccacccaccactcctcctcataaagccaaccaagataacccttttagggcttctccaaagctgaagtcctcttgcaagactgtggtgccaccaccatcaaagaagcccaggtacagtgagtcttctggtacacaaggcaataactccaccaagaaagggccggagcaatccgagttgtatgcacaactcagcaagtcctcagtcctcactggtggacacgaggaaaggaagaccaagcggcccagtctgcggctgtttggtgaccatgactattgccagtcaattaattccaaaacagaaatactcattaatatatcacaggagctccaagactctagacaactagaaaataaagatgtctcctctgattggcaggggcagatttgttcttccacagattcagaccagtgctacctgagagagactttggaggcaagcaagcaggtctctccttgcagcacaagaaaacagctccaagaccaggaaatccgagccgagctgaacaagcacttcggtcatcccagtcaagctgtttttgacgacgaagcagacaagaccggtgaactgagggacagtgatttcagtaatgaacaattctccaaactacctatgtttataaattcaggactagccatggatggcctgtttgatgacagcgaagatgaaagtgataaactgagctacccttgggatggcacgcaatcctattcattgttcaatgtgtctccttcttgttcttcttttaactctccatgtagagattctgtgtcaccacccaaatccttattttctcaaagaccccaaaggatgcgctctcgttcaaggtccttttctcgacacaggtcgtgttcccgatcaccatattccaggtcaagatcaaggtctccaggcagtagatcctcttcaagatcctgctattactatgagtcaagccactacagacaccgcacgcaccgaaattctcccttgtatgtgagatcacgttcaagatcgccctacagccgtcggcccaggtatgacagctacgaggaatatcagcacgagaggctgaagagggaagaatatcgcagagagtatgagaagcgagagtctgagagggccaagcaaagggagaggcagaggcagaaggcaattgaagagcgccgtgtgatttatgtcggtaaaatcagacctgacacaacacggacagaactgagggaccgttttgaagtttttggtgaaattgaggagtgcacagtaaatctgcgggatgatggagacagctatggtttcattacctaccgttatacctgtgatgcttttgctgctcttgaaaatggatacactttgcgcaggtcaaacgaaactgactttgagctgtacttttgtggacgcaagcaatttttcaagtctaactatgcagacctagattcaaactcagatgactttgaccctgcttccaccaagagcaagtatgactctctggattttgatagtttactgaaagaagctcagagaagcttgcgcaggggaagcggagccacgaacttctctctgttaaagcaagcaggagatgttgaagaaaaccccgggcctatggcggggaacgactgcggcgcgctgctggacgaagagctctcctccttcttcctcaactatctcgctgacacgcagggtggagggtccggggaggagcaactctatgctgactttccagaacttgacctctcccagctggatgccagcgactttgactcggccacctgctttggggagctgcagtggtgcccagagaactcagagactgaacccaaccagtacagccccgatgactccgagctcttccagattgacagtgagaatgaggccctcctggcagagctcaccaagaccctggatgacatccctgaagatgacgtgggtctggctgccttcccagccctggatggtggagacgctctatcatgcacctcagcttcgcctgccccctcatctgcaccccccagccctgccccggagaagccctcggccccagcccctgaggtggacgagctctcactgctgcagaagctcctcctggccacatcctacccaacatcaagctctgacacccagaaggaagggaccgcctggcgccaggcaggcctcagatctaaaagtcaacggccttgtgttaaggcggacagcacccaagacaagaaggctcccatgatgcagtctcagagccgaagttgtacagaactacataagcacctcacctcggcacagtgctgcctgcaggatcggggtctgcagccaccatgcctccagagtccccggctccctgccaaggaggacaaggagccgggtgaggactgcccgagcccccagccagctccagcctctccccgggactccctagctctgggcagggcagaccccggtgccccggtttcccaggaagacatgcaggcgatggtgcaactcatacgctacatgcacacctactgcctcccccagaggaagctgcccccacagacccctgagccactccccaaggcctgcagcaacccctcccagcaggtcagatcccggccctggtcccggcaccactccaaagcctcctgggctgagttctccattctgagggaacttctggctcaagacgtgctctgtgatgtcagcaaaccctaccgtctggccacgcctgtttatgcctccctcacacctcggtcaaggcccaggccccccaaagacagtcaggcctcccctggtcgcccgtcctcggtggaggaggtaaggatcgcagcttcacccaagagcaccgggcccagaccaagcctgcgcccactgcggctggaggtgaaaagggaggtccgccggcctgccagactgcagcagcaggaggaggaagacgaggaagaagaggaggaggaagaggaagaagaaaaagaggaggaggaggagtggggcaggaaaaggccaggccgaggcctgccatggacgaagctggggaggaagctggagagctctgtgtgccccgtgcggcgttctcggagactgaaccctgagctgggcccctggctgacatttgcagatgagccgctggtcccctcggagccccaaggtgctctgccctcactgtgcctggctcccaaggcctacgacgtagagcgggagctgggcagccccacggacgaggacagtggccaagaccagcagctcctacggggaccccagatccctgccctggagagcccctgtgagagtgggtgtggggacatggatgaggaccccagctgcccgcagctccctcccagagactctcccaggtgcctcatgctggccttgtcacaaagcgacccaacttttggcaagaagagctttgagcagaccttgacagtggagctctgtggcacagcaggactcaccccacccaccacaccaccgtacaagcccacagaggaggatcccttcaaaccagacatcaagcatagtctaggcaaagaaatagctctcagcctcccctcccctgagggcctctcactcaaggccaccccaggggctgcccacaagctgccaaagaagcacccagagcgaagtgagctcctgtcccacctgcgacatgccacagcccagccagcctcccaggctggccagaagcgtcccttctcctgttcctttggagaccatgactactgccaggtgctccgaccagaaggcgtcctgcaaaggaaggtgctgaggtcctgggagccgtctggggttcaccttgaggactggccccagcagggtgccccttgggctgaggcacaggcccctggcagggaggaagacagaagctgtgatgctggcgccccacccaaggacagcacgctgctgagagaccatgagatccgtgccagcctcaccaaacactttgggctgctggagaccgccctggaggaggaagacctggcctcctgcaagagccctgagtatgacactgtctttgaagacagcagcagcagcagcggcgagagcagcttcctcccagaggaggaagaggaagaaggggaggaggaggaggaggacgatgaagaagaggactcaggggtcagccccacttgctctgaccactgcccctaccagagcccaccaagcaaggccaaccggcagctctgttcccgcagccgctcaagctctggctcttcaccctgccactcctggtcaccagccactcgaaggaacttcagatgtgagagcagagggccgtgttcagacagaacgccaagcatccggcacgccaggaagcggcgggaaaaggccattggggaaggccgcgtggtgtacattcaaaatctctccagcgacatgagctcccgagagctgaagaggcgctttgaagtgtttggtgagattgaggagtgcgaggtgctgacaagaaataggagaggcgagaagtacggcttcatcacctaccggtgttctgagcacgcggccctctctttgacaaagggcgctgccctgaggaagcgcaacgagccctccttccagctgagctacggagggctccggcacttctgctggcccagatacactgactacgattccaattcagaagaggcccttcctgcgtcagggaaaagcaagtatgaagccatggattttgacagcttactgaaagaggcccagcagagcctgcattgacagacatgataagatacattgatgagtttggacaaaccacaactagaatgcagtgaaaaaaatgctttatttgtgaaatttgtgatgctattgctttatttgtaaccattataagctgcaataaacaagttaacaacaacaattgcattcattttatgtttcaggttcagggggaggtgtgggaggttttttaaagcaagtaaaacctctacaaatgtggtagggttgcgccttttccaaggcagccctgggtttgcgcagggacgcggctgctctgggcgtggttccgggaaacgcagcggcgccgaccctgggtctcgcacattcttcacgtccgttcgcagcgtcacccggatcttcgccgctacccttgtgggccccccggcgacgcttcctgctccgcccctaagtcgggaaggttccttgcggttcgcggcgtgccggacgtgacaaacggaagccgcacgtctcactagtaccctcgcagacggacagcgccagggagcaatggcagcgcgccgaccgcgatgggctgtggccaatagcggctgctcagcagggcgcgccgagagcagcggccgggaaggggcggtgcgggaggcggggtgtggggcggtagtgtgggccctgttcctgcccgcgcggtgttccgcattctgcaagcctccggagcgcacgtcggcagtcggctccctcgttgaccgaatcaccgacctctctccccagggccaccatgaccgagtacaagcccacggtgcgcctcgccacccgcgacgacgtccccagggccgtacgcaccctcgccgccgcgttcgccgactaccccgccacgcgccacaccgtcgatccggaccgccacatcgagcgggtcaccgagctgcaagaactcttcctcacgcgcgtcgggctcgacatcggcaaggtgtgggtcgcggacgacggcgccgcggtggcggtctggaccacgccggagagcgtcgaagcgggggcggtgttcgccgagatcggcccgcgcatggccgagttgagcggttcccggctggccgcgcagcaacagatggaaggcctcctggcgccgcaccggcccaaggagcccgcgtggttcctggccaccgtcggcgtctcgcccgaccaccagggcaagggtctgggcagcgccgtcgtgctccccggagtggaggcggccgagcgcgccggggtgcccgccttcctggagacctccgcgccccgcaacctccccttctacgagcggctcggcttcaccgtcaccgccgacgtcgaggtgcccgaaggaccgcgcacctggtgcatgacccgcaagcccggtgcctgacaactttattatacatagttgatcctcaggtgcaggctgcctatcagaaggtggtggctggtgtggccaatgccctggctcacaaataccactgagatctttttccctctgccaaaaattatggggacatcatgaagccccttgagcatctgacttctggctaataaaggaaatttattttcattgcaatagtgtgttggaattttttgtgtctctcactcggaaggacatatgggagggcaaatcatttaaaacatcagaatgagtatttggtttagagtttggcaacatatgcccatatgctggctgccatgaacaaaggttggctataaagaggtcatcagtatatgaaacagccccctgctgtccattccttattccatagaaaagccttgacttgaggttagattttttttatattttgttttgtgttatttttttctttaacatccctaaaattttccttacatgttttactagccagatttttcctcctctcctgactactcccagtcatagctgtccctcttctcttatggagatccctcgacctgcagcccaagcttggatccctcgagttaattaacgagagcataatattgatatgtgccaaagttgtttctgactgactaataagtataatttgtttctattatgtataggttaagctaattacttattttataatacaacatgactgtttttaaagtacaaaataagtttatttttgtaaaagagagaatgtttaaaagttttgttactttatagaagaaattttgagtttttgtttttttttaataaataaataaacataaataaattgtttgttgaatttattattagtatgtaagtgtaaatataataaaacttaatatctattcaaattaataaataaacctcgatatacagaccgataaaacacatgcgtcaattttacgcatgattatctttaacgtacgtcacaatatgattatctttctagggttaaataatagtttctaatttttttattattcagcctgctgtcgtgaataccgagctccaattcgccctatagtgagtcgtattacaattcactggccgtcgttttacaacgtcgtgactgggaaaaccctggcgttacccaacttaatcgccttgcagcacatccccctttcgccagctggcgtaatagcgaagaggcccgcaccgatcgcccttcccaacagttgcgcagcctgaatggcgaatgggacgcgccctgtagcggcgcattaagcgcggcgggtgtggtggttacgcgcagcgtgaccgctacacttgccagcgccctagcgcccgctcctttcgctttcttcccttcctttctcgccacgttcgccggctttccccgtcaagctctaaatcgggggctccctttagggttccgatttagtgctttacggcacctcgaccccaaaaaacttgattagggtgatggttcacgtagtgggccatcgccctgatagacggtttttcgccctttgacgttggagtccacgttctttaatagtggactcttgttccaaactggaacaacactcaaccctatctcggtctattcttttgatttataagggattttgccgatttcggcctattggttaaaaaatgagctgatttaacaaaaatttaacgcgaattttaacaaaatattaacgcttacaattttaggtggcacttttcggggaaatgtgcgcggaacccctatttgtttatttttctaaatacattcaaatatgtatccgctcatgagacaataaccctgataaatgcttcaataatattgaaaaaggaagagtatgagtattcaacatttccgtgtcgcccttattcccttttttgcggcattttgccttcctgtttttgctcacccagaaacgctggtgaaagtaaaagatgctgaagatcagttgggtgcacgagtgggttacatcgaactggatctcaacagcggtaagatccttgagagttttcgccccgaagaacgttttccaatgatgagcacttttaaagttctgctatgtggcgcggtattatcccgtattgacgccgggcaagagcaactcggtcgccgcatacactattctcagaatgacttggttgagtactcaccagtcacagaaaagcatcttacggatggcatgacagtaagagaattatgcagtgctgccataaccatgagtgataacactgcggccaacttacttctgacaacgatcggaggaccgaaggagctaaccgcttttttgcacaacatgggggatcatgtaactcgccttgatcgttgggaaccggagctgaatgaagccataccaaacgacgagcgtgacaccacgatgcctgtagcaatggcaacaacgttgcgcaaactattaactggcgaactacttactctagcttcccggcaacaattaatagactggatggaggcggataaagttgcaggaccacttctgcgctcggcccttccggctggctggtttattgctgataaatctggagccggtgagcgtgggtctcgcggtatcattgcagcactggggccagatggtaagccctcccgtatcgtagttatctacacgacggggagtcaggcaactatggatgaacgaaatagacagatcgctgagataggtgcctcactgattaagcattggtaactgtcagaccaagtttactcatatatactttagattgatttaaaacttcatttttaatttaaaaggatctaggtgaagatcctttttgataatctcatgaccaaaatcccttaacgtgagttttcgttccactgagcgtcagaccccgtagaaaagatcaaaggatcttcttgagatcctttttttctgcgcgtaatctgctgcttgcaaacaaaaaaaccaccgctaccagcggtggtttgtttgccggatcaagagctaccaactctttttccgaaggtaactggcttcagcagagcgcagataccaaatactgttcttctagtgtagccgtagttaggccaccacttcaagaactctgtagcaccgcctacatacctcgctctgctaatcctgttaccagtggctgctgccagtggcgataagtcgtgtcttaccgggttggactcaagacgatagttaccggataaggcgcagcggtcgggctgaacggggggttcgtgcacacagcccagcttggagcgaacgacctacaccgaactgagatacctacagcgtgagctatgagaaagcgccacgcttcccgaagggagaaaggcggacaggtatccggtaagcggcagggtcggaacaggagagcgcacgagggagcttccagggggaaacgcctggtatctttatagtcctgtcgggtttcgccacctctgacttgagcgtcgatttttgtgatgctcgtcaggggggcggagcctatggaaaaacgccagcaacgcggcctttttacggttcctggccttttgctggccttttgctcacatgttctttcctgcgttatcccctgattctgtggataaccgtattaccgcctttgagtgagctgataccgctcgccgcagccgaacgaccgagcgcagcgagtcagtgagcgaggaagcggaagagcgcccaatacgcaaaccgcctctccccgcgcgttggccgattcattaatgcagctggcacgacaggtttcccgactggaaagcgggcagtgagcgcaacgcaattaatgtgagttagctcactcattaggcaccccaggctttacactttatgcttccggctcgtatgttgtgtggaattgtgagcggataacaatttcacacaggaaacagctatgaccatgattacgccaagctcgaaattaaccctcactaaagggaacaaaagctggtacctcgcgcgacttggtttgccattctttagcgcgcgtcgcgtcacacagcttggccacaatgtggtttttgtcaaacgaagattctatgacgtgtttaaagtttaggtcgagtaaagcgcaaatctttt

SEQ ID NO: 32 - DNA, 16782 bp, synthetic construct
  source 1..16782: mol_type = other DNA
ttaaccctagaaagatagtctgcgtaaaattgacgcatgcattcttgaaatattgctctctctttctaaatagcgcgaatccgtcgctgtgcatttaggacatctcagtcgccgcttggagctcccgtgaggcgtgcttgtcaatgcggtaagtgtcactgattttgaactataacgaccgcgtgagtcaaaatgacgcatgattatcttttacgtgacttttaagatttaactcatacgataattatattgttatttcatgttctacttacgtgataacttattatatatatattttcttgttatagatatcatcaactttgtatagaaaagttggacattgattattgactagttattaatagtaatcaattacggggtcattagttcatagcccatatatggagttccgcgttacataacttacggtaaatggcccgcctggctgaccgcccaacgacccccgcccattgacgtcaataatgacgtatgttcccatagtaacgccaatagggactttccattgacgtcaatgggtggagtatttacggtaaactgcccacttggcagtacatcaagtgtatcatatgccaagtacgccccctattgacgtcaatgacggtaaatggcccgcctggcattatgcccagtacatgaccttatgggactttcctacttggcagtacatctacgtattagtcatcgctattaccatggtgatgcggttttggcagtacatcaatgggcgtggatagcggtttgactcacggggatttccaagtctccaccccattgacgtcaatgggagtttgttttggcaccaaaatcaacgggactttccaaaatgtcgtaacaactccgccccattgacgcaaatgggcggtaggcgtgtacggtgggaggtctatataagcagagctcgtttagtgaaccgtcagatcgcctggagacgccatccacgctgttttgacctccatagaagacaccgggaccgatccagcctcccctcgaagcttacatgtggtaccgagctcggatcctgagaacttcagggtgagtctatgggacccttgatgttttctttccccttcttttctatggttaagttcatgtcataggaaggggagaagtaacagggtacacatattgaccaaatcagggtaattttgcatttgtaattttaaaaaatgctttcttcttttaatatacttttttgtttatcttatttctaatactttccctaatctctttctttcagggcaataatgatacaatgtatcatgcctctttgcaccattctaaagaataacagtgataatttctgggttaaggcaatagcaatatttctgcatataaatatttctgcatataaattgtaactgatgtaagaggtttcatattgctaatagcagctacaatccagctaccattctgcttttattttatggttgggataaggctggattattctgagtccaagctaggcccttttgctaatcatgttcatacctcttatcttcctcccacagctcctgggcaacgtgctggtctgtgtgctggcccatcactttggcaaagcaagtttgtacaaaaaagcaggctgccaccatgccgcgcgctccccgctgccgagccgtgcgctccctgctgcgcagccactaccgcgaggtgctgccgctggccacgttcgtgcggcgcctggggccccagggctggcggctggtgcagcgcggggacccggcggctttccgcgcgctggtggcccagtgcctggtgtgcgtgccctgggacgcacggccgccccccgccgccccctccttccgccaggtgtcctgcctgaaggagctggtggcccgagtgctgcagaggctgtgcgagcgcggcgcgaagaacgtgctggccttcggcttcgcgctgctggacggggcccgcgggggcccccccgaggccttcaccaccagcgtgcgcagctacctgcccaacacggtgaccgacgcactgcgggggagcggggcgtgggggctgctgctgcgccgcgtgggcgacgacgtgctggttcacctgctggcacgctgcgcgctctttgtgctggtggctcccagctgcgcctaccaggtgtgcgggccgccgctgtaccagctcggcgctgccactcaggcccggcccccgccacacgctagtggaccccgaaggcgtctgggatgcgaacgggcctggaaccatagcgtcagggaggccggggtccccctgggcctgccagccccgggtgcgaggaggcgcgggggcagtgccagccgaagtctgccgttgcccaagaggcccaggcgtggcgctgcccctgagccggagcggacgcccgttgggcaggggtcctgggcccacccgggcaggacgcgtggaccgagtgaccgtggtttctgtgtggtgtcacctgccagacccgccgaagaagccacctctttggagggtgcgctctctggcacgcgccactcccacccatccgtgggccgccagcaccacgcgggccccccatccacatcgcggccaccacgtccctgggacacgccttgtcccccggtgtacgccgagaccaagcacttcctctactcctcaggcgacaaggagcagctgcggccctccttcctactcagctctctgaggcccagcctgactggcgctcggaggctcgtggagaccatctttctgggttccaggccctggatgccagggactccccgcaggttgccccgcctgccccagcgctactggcaaatgcggcccctgtttctggagctgcttgggaaccacgcgcagtgcccctacggggtgctcctcaagacgcactgcccgctgcgagctgcggtcaccccagcagccggtgtctgtgcccgggagaagccccagggctctgtggcggcccccgaggaggaggacacagacccccgtcgcctggtgcagctgctccgccagcacagcagcccctggcaggtgtacggcttcgtgcgggcctgcctgcgccggctggtgcccccaggcctctggggctccaggcacaacgaacgccgcttcctcaggaacaccaagaagttcatctccctggggaagcatgccaagctctcgctgcaggagctgacgtggaagatgagcgtgcgggactgcgcttggctgcgcaggagcccaggggttggctgtgttccggccgcagagcaccgtctgcgtgaggagatcctggccaagttcctgcactggctgatgagtgtgtacgtcgtcgagctgctcaggtctttcttttatgtcacggagaccacgtttcaaaagaacaggctctttttctaccggaagagtgtctggagcaagttgcaaagcattggaatcagacagcacttgaagagggtgcagctgcgggagctgtcggaagcagaggtcaggcagcatcgggaagccaggcccgccctgctgacgtccagactccgcttcatccccaagcctgacgggctgcggccgattgtgaacatggactacgtcgtgggagccagaacgttccgcagagaaaagagggccgagcgtctcacctcgagggtgaaggcactgttcagcgtgctcaactacgagcgggcgcggcgccccggcctcctgggcgcctctgtgctgggcctggacgatatccacagggcctggcgcaccttcgtgctgcgtgtgcgggcccaggacccgccgcctgagctgtactttgtcaaggtggatgtgacgggcgcgtacgacaccatcccccaggacaggctcacggaggtcatcgccagcatcatcaaaccccagaacacgtactgcgtgcgtcggtatgccgtggtccagaaggccgcccatgggcacgtccgcaaggccttcaagagccacgtctctaccttgacagacctccagccgtacatgcgacagttcgtggctcacctgcaggagaccagcccgctgagggatgccgtcgtcatcgagcagagctcctccctgaatgaggccagcagtggcctcttcgacgtcttcctacgcttcatgtgccaccacgccgtgcgcatcaggggcaagtcctacgtccagtgccaggggatcccgcagggctccatcctctccacgctgctctgcagcctgtgctacggcgacatggagaacaagctgtttgcggggattcggcgggacgggctgctcctgcgtttggtggatgatttcttgttggtgacacctcacctcacccacgcgaaaaccttcctcaggaccctggtccgaggtgtccctgagtatggctgcgtggtgaacttgcggaagacagtggtgaacttccctgtagaagacgaggccctgggtggcacggcttttgttcagatgccggcccacggcctattcccctggtgcggcctgctgctggatacccggaccctggaggtgcagagcgactactccagctatgcccggacctccatcagagccagtctcaccttcaaccgcggcttcaaggctgggaggaacatgcgtcgcaaactctttggggtcttgcggctgaagtgtcacagcctgtttctggatttgcaggtgaacagcctccagacggtgtgcaccaacatctacaagatcctcctgctgcaggcgtacaggtttcacgcatgtgtgctgcagctcccatttcatcagcaagtttggaagaaccccacatttttcctgcgcgtcatctctgacacggcctccctctgctactccatcctgaaagccaagaacgcagggatgtcgctgggggccaagggcgccgccggccctctgccctccgaggccgtgcagtggctgtgccaccaagcattcctgctcaagctgactcgacaccgtgtcacctacgtgccactcctggggtcactcaggacagcccagacgcagctgagtcggaagctcccggggacgacgctgactgccctggaggccgcagccaacccggcactgccctcagacttcaagaccatcctggacggaagcggagccacgaacttctctctgttaaagcaagcaggagatgttgaagaaaaccccgggcctatggatgagacctccccaaggctggaagaagactggaaaaaagtacttcagcgagaagcaggctggcagtgtgctgctctggttggtgaagaccagcctctttgcccagatcttcctgaacttgatctttctgaactagatgtgaacgacttggatacagacagctttctgggtggactcaagtggtgcagtgaccaatcagaaataatatccaatcagtacaacaatgagccttcaaacatatttgagaagatagatgaagagaatgaggcaaacttgctagcagtcctcacagagacactagacagtctccctgtggatgaagacggattgccctcatttgatgcgctgacagatggagacgtgaccactgacaatgaggctagtccttcctccatgcctgacggcacccctccaccccaggaggcagaagagccgtctctacttaagaagctcttactggcaccagccaacactcagctaagttataatgaatgcagtggtctcagtacccagaaccatgcaaatcacaatcacaggatcagaacaaaccctgcaattgttaagactgagaattcatggagcaataaagcgaagagtatttgtcaacagcaaaagccacaaagacgtccctgctcggagcttctcaaatatctgaccacaaacgatgaccctcctcacaccaaacccacagagaacagaaacagcagcagagacaaatgcacctccaaaaagaagtcccacacacagtcgcagtcacaacacttacaagccaaaccaacaactttatctcttcctctgaccccagagtcaccaaatgaccccaagggttccccatttgagaacaagactattgaacgcaccttaagtgtggaactctctggaactgcaggcctaactccacccaccactcctcctcataaagccaaccaagataacccttttagggcttctccaaagctgaagtcctcttgcaagactgtggtgccaccaccatcaaagaagcccaggtacagtgagtcttctggtacacaaggcaataactccaccaagaaagggccggagcaatccgagttgtatgcacaactcagcaagtcctcagtcctcactggtggacacgaggaaaggaagaccaagcggcccagtctgcggctgtttggtgaccatgactattgccagtcaattaattccaaaacagaaatactcattaatatatcacaggagctccaagactctagacaactagaaaataaagatgtctcctctgattggcaggggcagatttgttcttccacagattcagaccagtgctacctgagagagactttggaggcaagcaagcaggtctctccttgcagcacaagaaaacagctccaagaccaggaaatccgagccgagctgaacaagcacttcggtcatcccagtcaagctgtttttgacgacgaagcagacaagaccggtgaactgagggacagtgatttcagtaatgaacaattctccaaactacctatgtttataaattcaggactagccatggatggcctgtttgatgacagcgaagatgaaagtgataaactgagctacccttgggatggcacgcaatcctattcattgttcaatgtgtctccttcttgttcttcttttaactctccatgtagagattctgtgtcaccacccaaatccttattttctcaaagaccccaaaggatgcgctctcgttcaaggtccttttctcgacacaggtcgtgttcccgatcaccatattccaggtcaagatcaaggtctccaggcagtagatcctcttcaagatcctgctattactatgagtcaagccactacagacaccgcacgcaccgaaattctcccttgtatgtgagatcacgttcaagatcgccctacagccgtcggcccaggtatgacagctacgaggaatatcagcacgagaggctgaagagggaagaatatcgcagagagtatgagaagcgagagtctgagagggccaagcaaagggagaggcagaggcagaaggcaattgaagagcgccgtgtgatttatgtcggtaaaatcagacctgacacaacacggacagaactgagggaccgttttgaagtttttggtgaaattgaggagtgcacagtaaatctgcgggatgatggagacagctatggtttcattacctaccgttatacctgtgatgcttttgctgctcttgaaaatggatacactttgcgcaggtcaaacgaaactgactttgagctgtacttttgtggacgcaagcaatttttcaagtctaactatgcagacctagattcaaactcagatgactttgaccctgcttccaccaagagcaagtatgactctctggattttgatagtttactgaaagaagctcagagaagcttgcgcaggggaagcggagagggcaggggaagtcttctaacatgcggggacgtggaggaaaatcccggccccatggcggggaacgactgcggcgcgctgctggacgaagagctctcctccttcttcctcaactatctcgctgacacgcagggtggagggtccggggaggagcaactctatgctgactttccagaacttgacctctcccagctggatgccagcgactttgactcggccacctgctttggggagctgcagtggtgcccagagaactcagagactgaacccaaccagtacagccccgatgactccgagctcttccagattgacagtgagaatgaggccctcctggcagagctcaccaagaccctggatgacatccctgaagatgacgtgggtctggctgccttcccagccctggatggtggagacgctctatcatgcacctcagcttcgcctgccccctcatctgcaccccccagccctgccccggagaagccctcggccccagcccctgaggtggacgagctctcactgctgcagaagctcctcctggccacatcctacccaacatcaagctctgacacccagaaggaagggaccgcctggcgccaggcaggcctcagatctaaaagtcaacggccttgtgttaaggcggacagcacccaagacaagaaggctcccatgatgcagtctcagagccgaagttgtacagaactacataagcacctcacctcggcacagtgctgcctgcaggatcggggtctgcagccaccatgcctccagagtccccggctccctgccaaggaggacaaggagccgggtgaggactgcccgagcccccagccagctccagcctctccccgggactccctagctctgggcagggcagaccccggtgccccggtttcccaggaagacatgcaggcgatggtgcaactcatacgctacatgcacacctactgcctcccccagaggaagctgcccccacagacccctgagccactccccaaggcctgcagcaacccctcccagcaggtcagatcccggccctggtcccggcaccactccaaagcctcctgggctgagttctccattctgagggaacttctggctcaagacgtgctctgtgatgtcagcaaaccctaccgtctggccacgcctgtttatgcctccctcacacctcggtcaaggcccaggccccccaaagacagtcaggcctcccctggtcgcccgtcctcggtggaggaggtaaggatcgcagcttcacccaagagcaccgggcccagaccaagcctgcgcccactgcggctggaggtgaaaagggaggtccgccggcctgccagactgcagcagcaggaggaggaagacgaggaagaagaggaggaggaagaggaagaagaaaaagaggaggaggaggagtggggcaggaaaaggccaggccgaggcctgccatggacgaagctggggaggaagctggagagctctgtgtgccccgtgcggcgttctcggagactgaaccctgagctgggcccctggctgacatttgcagatgagccgctggtcccctcggagccccaaggtgctctgccctcactgtgcctggctcccaaggcctacgacgtagagcgggagctgggcagccccacggacgaggacagtggccaagaccagcagctcctacggggaccccagatccctgccctggagagcccctgtgagagtgggtgtggggacatggatgaggaccccagctgcccgcagctccctcccagagactctcccaggtgcctcatgctggccttgtcacaaagcgacccaacttttggcaagaagagctttgagcagaccttgacagtggagctctgtggcacagcaggactcaccccacccaccacaccaccgtacaagcccacagaggaggatcccttcaaaccagacatcaagcatagtctaggcaaagaaatagctctcagcctcccctcccctgagggcctctcactcaaggccaccccaggggctgcccacaagctgccaaagaagcacccagagcgaagtgagctcctgtcccacctgcgacatgccacagcccagccagcctcccaggctggccagaagcgtcccttctcctgttcctttggagaccatgactactgccaggtgctccgaccagaaggcgtcctgcaaaggaaggtgctgaggtcctgggagccgtctggggttcaccttgaggactggccccagcagggtgccccttgggctgaggcacaggcccctggcagggaggaagacagaagctgtgatgctggcgccccacccaaggacagcacgctgctgagagaccatgagatccgtgccagcctcaccaaacactttgggctgctggagaccgccctggaggaggaagacctggcctcctgcaagagccctgagtatgacactgtctttgaagacagcagcagcagcagcggcgagagcagcttcctcccagaggaggaagaggaagaaggggaggaggaggaggaggacgatgaagaagaggactcaggggtcagccccacttgctctgaccactgcccctaccagagcccaccaagcaaggccaaccggcagctctgttcccgcagccgctcaagctctggctcttcaccctgccactcctggtcaccagccactcgaaggaacttcagatgtgagagcagagggccgtgttcagacagaacgccaagcatccggcacgccaggaagcggcgggaaaaggccattggggaaggccgcgtggtgtacattcaaaatctctccagcgacatgagctcccgagagctgaagaggcgctttgaagtgtttggtgagattgaggagtgcgaggtgctgacaagaaataggagaggcgagaagtacggcttcatcacctaccggtgttctgagcacgcggccctctctttgacaaagggcgctgccctgaggaagcgcaacgagccctccttccagctgagctacggagggctccggcacttctgctggcccagatacactgactacgattccaattcagaagaggcccttcctgcgtcagggaaaagcaagtatgaagccatggattttgacagcttactgaaagaggcccagcagagcctgcattgactgtgccttctagttgccagccatctgttgtttgcccctcccccgtgccttccttgaccctggaaggtgccactcccactgtcctttcctaataaaatgaggaaattgcatcgcattgtctgagtaggtgtcattctattctggggggtggggtggggcaggacagcaagggggaggattgggaagacaatagcaggcatgctggggatgcggtgggctctatggacccagctttcttgtacaaagtgggggttgcgccttttccaaggcagccctgggtttgcgcagggacgcggctgctctgggcgtggttccgggaaacgcagcggcgccgaccctgggtctcgcacattcttcacgtccgttcgcagcgtcacccggatcttcgccgctacccttgtgggccccccggcgacgcttcctgctccgcccctaagtcgggaaggttccttgcggttcgcggcgtgccggacgtgacaaacggaagccgcacgtctcactagtaccctcgcagacggacagcgccagggagcaatggcagcgcgccgaccgcgatgggctgtggccaatagcggctgctcagcagggcgcgccgagagcagcggccgggaaggggcggtgcgggaggcggggtgtggggcggtagtgtgggccctgttcctgcccgcgcggtgttccgcattctgcaagcctccggagcgcacgtcggcagtcggctccctcgttgaccgaatcaccgacctctctccccagggccaccatggtgagcaagggcgaggagctgttcaccggggtggtgcccatcctggtcgagctggacggcgacgtaaacggccacaagttcagcgtgtccggcgagggcgagggcgatgccacctacggcaagctgaccctgaagttcatctgcaccaccggcaagctgcccgtgccctggcccaccctcgtgaccaccctgacctacggcgtgcagtgcttcagccgctaccccgaccacatgaagcagcacgacttcttcaagtccgccatgcccgaaggctacgtccaggagcgcaccatcttcttcaaggacgacggcaactacaagacccgcgccgaggtgaagttcgagggcgacaccctggtgaaccgcatcgagctgaagggcatcgacttcaaggaggacggcaacatcctggggcacaagctggagtacaactacaacagccacaacgtctatatcatggccgacaagcagaagaacggcatcaaggtgaacttcaagatccgccacaacatcgaggacggcagcgtgcagctcgccgaccactaccagcagaacacccccatcggcgacggccccgtgctgctgcccgacaaccactacctgagcacccagtccgccctgagcaaagaccccaacgagaagcgcgatcacatggtcctgctggagttcgtgaccgccgccgggatcactctcggcatggacgagctgtacaagggaagcggagccacgaacttctctctgttaaagcaagcaggagatgttgaagaaaaccccgggcctatgaccgagtacaagcccacggtgcgcctcgccacccgcgacgacgtccccagggccgtacgcaccctcgccgccgcgttcgccgactaccccgccacgcgccacaccgtcgatccggaccgccacatcgagcgggtcaccgagctgcaagaactcttcctcacgcgcgtcgggctcgacatcggcaaggtgtgggtcgcggacgacggcgccgcggtggcggtctggaccacgccggagagcgtcgaagcgggggcggtgttcgccgagatcggcccgcgcatggccgagttgagcggttcccggctggccgcgcagcaacagatggaaggcctcctggcgccgcaccggcccaaggagcccgcgtggttcctggccaccgtcggcgtctcgcccgaccaccagggcaagggtctgggcagcgccgtcgtgctccccggagtggaggcggccgagcgcgccggggtgcccgccttcctggagacctccgcgccccgcaacctccccttctacgagcggctcggcttcaccgtcaccgccgacgtcgaggtgcccgaaggaccgcgcacctggtgcatgacccgcaagcccggtgcctgacaactttattatacatagttgatcctcaggtgcaggctgcctatcagaaggtggtggctggtgtggccaatgccctggctcacaaataccactgagatctttttccctctgccaaaaattatggggacatcatgaagccccttgagcatctgacttctggctaataaaggaaatttattttcattgcaatagtgtgttggaattttttgtgtctctcactcggaaggacatatgggagggcaaatcatttaaaacatcagaatgagtatttggtttagagtttggcaacatatgcccatatgctggctgccatgaacaaaggttggctataaagaggtcatcagtatatgaaacagccccctgctgtccattccttattccatagaaaagccttgacttgaggttagattttttttatattttgttttgtgttatttttttctttaacatccctaaaattttccttacatgttttactagccagatttttcctcctctcctgactactcccagtcatagctgtccctcttctcttatggagatccctcgacctgcagcccaagcttggatccctcgagttaattaacgagagcataatattgatatgtgccaaagttgtttctgactgactaataagtataatttgtttctattatgtataggttaagctaattacttattttataatacaacatgactgtttttaaagtacaaaataagtttatttttgtaaaagagagaatgtttaaaagttttgttactttatagaagaaattttgagtttttgtttttttttaataaataaataaacataaataaattgtttgttgaatttattattagtatgtaagtgtaaatataataaaacttaatatctattcaaattaataaataaacctcgatatacagaccgataaaacacatgcgtcaattttacgcatgattatctttaacgtacgtcacaatatgattatctttctagggttaaataatagtttctaatttttttattattcagcctgctgtcgtgaataccgagctccaattcgccctatagtgagtcgtattacaattcactggccgtcgttttacaacgtcgtgactgggaaaaccctggcgttacccaacttaatcgccttgcagcacatccccctttcgccagctggcgtaatagcgaagaggcccgcaccgatcgcccttcccaacagttgcgcagcctgaatggcgaatgggacgcgccctgtagcggcgcattaagcgcggcgggtgtggtggttacgcgcagcgtgaccgctacacttgccagcgccctagcgcccgctcctttcgctttcttcccttcctttctcgccacgttcgccggctttccccgtcaagctctaaatcgggggctccctttagggttccgatttagtgctttacggcacctcgaccccaaaaaacttgattagggtgatggttcacgtagtgggccatcgccctgatagacggtttttcgccctttgacgttggagtccacgttctttaatagtggactcttgttccaaactggaacaacactcaaccctatctcggtctattcttttgatttataagggattttgccgatttcggcctattggttaaaaaatgagctgatttaacaaaaatttaacgcgaattttaacaaaatattaacgcttacaattttaggtggcacttttcggggaaatgtgcgcggaacccctatttgtttatttttctaaatacattcaaatatgtatccgctcatgagacaataaccctgataaatgcttcaataatattgaaaaaggaagagtatgagtattcaacatttccgtgtcgcccttattcccttttttgcggcattttgccttcctgtttttgctcacccagaaacgctggtgaaagtaaaagatgctgaagatcagttgggtgcacgagtgggttacatcgaactggatctcaacagcggtaagatccttgagagttttcgccccgaagaacgttttccaatgatgagcacttttaaagttctgctatgtggcgcggtattatcccgtattgacgccgggcaagagcaactcggtcgccgcatacactattctcagaatgacttggttgagtactcaccagtcacagaaaagcatcttacggatggcatgacagtaagagaattatgcagtgctgccataaccatgagtgataacactgcggccaacttacttctgacaacgatcggaggaccgaaggagctaaccgcttttttgcacaacatgggggatcatgtaactcgccttgatcgttgggaaccggagctgaatgaagccataccaaacgacgagcgtgacaccacgatgcctgtagcaatggcaacaacgttgcgcaaactattaactggcgaactacttactctagcttcccggcaacaattaatagactggatggaggcggataaagttgcaggaccacttctgcgctcggcccttccggctggctggtttattgctgataaatctggagccggtgagcgtgggtctcgcggtatcattgcagcactggggccagatggtaagccctcccgtatcgtagttatctacacgacggggagtcaggcaactatggatgaacgaaatagacagatcgctgagataggtgcctcactgattaagcattggtaactgtcagaccaagtttactcatatatactttagattgatttaaaacttcatttttaatttaaaaggatctaggtgaagatcctttttgataatctcatgaccaaaatcccttaacgtgagttttcgttccactgagcgtcagaccccgtagaaaagatcaaaggatcttcttgagatcctttttttctgcgcgtaatctgctgcttgcaaacaaaaaaaccaccgctaccagcggtggtttgtttgccggatcaagagctaccaactctttttccgaaggtaactggcttcagcagagcgcagataccaaatactgttcttctagtgtagccgtagttaggccaccacttcaagaactctgtagcaccgcctacatacctcgctctgctaatcctgttaccagtggctgctgccagtggcgataagtcgtgtcttaccgggttggactcaagacgatagttaccggataaggcgcagcggtcgggctgaacggggggttcgtgcacacagcccagcttggagcgaacgacctacaccgaactgagatacctacagcgtgagctatgagaaagcgccacgcttcccgaagggagaaaggcggacaggtatccggtaagcggcagggtcggaacaggagagcgcacgagggagcttccagggggaaacgcctggtatctttatagtcctgtcgggtttcgccacctctgacttgagcgtcgatttttgtgatgctcgtcaggggggcggagcctatggaaaaacgccagcaacgcggcctttttacggttcctggccttttgctggccttttgctcacatgttctttcctgcgttatcccctgattctgtggataaccgtattaccgcctttgagtgagctgataccgctcgccgcagccgaacgaccgagcgcagcgagtcagtgagcgaggaagcggaagagcgcccaatacgcaaaccgcctctccccgcgcgttggccgattcattaatgcagctggcacgacaggtttcccgactggaaagcgggcagtgagcgcaacgcaattaatgtgagttagctcactcattaggcaccccaggctttacactttatgcttccggctcgtatgttgtgtggaattgtgagcggataacaatttcacacaggaaacagctatgaccatgattacgccaagctcgaaattaaccctcactaaagggaacaaaagctggtacctcgcgcgacttggtttgccattctttagcgcgcgtcgcgtcacacagcttggccacaatgtggtttttgtcaaacgaagattctatgacgtgtttaaagtttaggtcgagtaaagcgcaaatctttt

SEQ ID NO: 33 - DNA, 15999 bp, synthetic construct
  source 1..15999: mol_type = other DNA
ttaaccctagaaagatagtctgcgtaaaattgacgcatgcattcttgaaatattgctctctctttctaaatagcgcgaatccgtcgctgtgcatttaggacatctcagtcgccgcttggagctcccgtgaggcgtgcttgtcaatgcggtaagtgtcactgattttgaactataacgaccgcgtgagtcaaaatgacgcatgattatcttttacgtgacttttaagatttaactcatacgataattatattgttatttcatgttctacttacgtgataacttattatatatatattttcttgttatagatatcatcaactttgtatagaaaagttggacattgattattgactagttattaatagtaatcaattacggggtcattagttcatagcccatatatggagttccgcgttacataacttacggtaaatggcccgcctggctgaccgcccaacgacccccgcccattgacgtcaataatgacgtatgttcccatagtaacgccaatagggactttccattgacgtcaatgggtggagtatttacggtaaactgcccacttggcagtacatcaagtgtatcatatgccaagtacgccccctattgacgtcaatgacggtaaatggcccgcctggcattatgcccagtacatgaccttatgggactttcctacttggcagtacatctacgtattagtcatcgctattaccatggtgatgcggttttggcagtacatcaatgggcgtggatagcggtttgactcacggggatttccaagtctccaccccattgacgtcaatgggagtttgttttggcaccaaaatcaacgggactttccaaaatgtcgtaacaactccgccccattgacgcaaatgggcggtaggcgtgtacggtgggaggtctatataagcagagctcgtttagtgaaccgtcagatcgcctggagacgccatccacgctgttttgacctccatagaagacaccgggaccgatccagcctcccctcgaagcttacatgtggtaccgagctcggatcctgagaacttcagggtgagtctatgggacccttgatgttttctttccccttcttttctatggttaagttcatgtcataggaaggggagaagtaacagggtacacatattgaccaaatcagggtaattttgcatttgtaattttaaaaaatgctttcttcttttaatatacttttttgtttatcttatttctaatactttccctaatctctttctttcagggcaataatgatacaatgtatcatgcctctttgcaccattctaaagaataacagtgataatttctgggttaaggcaatagcaatatttctgcatataaatatttctgcatataaattgtaactgatgtaagaggtttcatattgctaatagcagctacaatccagctaccattctgcttttattttatggttgggataaggctggattattctgagtccaagctaggcccttttgctaatcatgttcatacctcttatcttcctcccacagctcctgggcaacgtgctggtctgtgtgctggcccatcactttggcaaagcaagtttgtacaaaaaagcaggctgccaccatgccgcgcgctccccgctgccgagccgtgcgctccctgctgcgcagccactaccgcgaggtgctgccgctggccacgttcgtgcggcgcctggggccccagggctggcggctggtgcagcgcggggacccggcggctttccgcgcgctggtggcccagtgcctggtgtgcgtgccctgggacgcacggccgccccccgccgccccctccttccgccaggtgtcctgcctgaaggagctggtggcccgagtgctgcagaggctgtgcgagcgcggcgcgaagaacgtgctggccttcggcttcgcgctgctggacggggcccgcgggggcccccccgaggccttcaccaccagcgtgcgcagctacctgcccaacacggtgaccgacgcactgcgggggagcggggcgtgggggctgctgctgcgccgcgtgggcgacgacgtgctggttcacctgctggcacgctgcgcgctctttgtgctggtggctcccagctgcgcctaccaggtgtgcgggccgccgctgtaccagctcggcgctgccactcaggcccggcccccgccacacgctagtggaccccgaaggcgtctgggatgcgaacgggcctggaaccatagcgtcagggaggccggggtccccctgggcctgccagccccgggtgcgaggaggcgcgggggcagtgccagccgaagtctgccgttgcccaagaggcccaggcgtggcgctgcccctgagccggagcggacgcccgttgggcaggggtcctgggcccacccgggcaggacgcgtggaccgagtgaccgtggtttctgtgtggtgtcacctgccagacccgccgaagaagccacctctttggagggtgcgctctctggcacgcgccactcccacccatccgtgggccgccagcaccacgcgggccccccatccacatcgcggccaccacgtccctgggacacgccttgtcccccggtgtacgccgagaccaagcacttcctctactcctcaggcgacaaggagcagctgcggccctccttcctactcagctctctgaggcccagcctgactggcgctcggaggctcgtggagaccatctttctgggttccaggccctggatgccagggactccccgcaggttgccccgcctgccccagcgctactggcaaatgcggcccctgtttctggagctgcttgggaaccacgcgcagtgcccctacggggtgctcctcaagacgcactgcccgctgcgagctgcggtcaccccagcagccggtgtctgtgcccgggagaagccccagggctctgtggcggcccccgaggaggaggacacagacccccgtcgcctggtgcagctgctccgccagcacagcagcccctggcaggtgtacggcttcgtgcgggcctgcctgcgccggctggtgcccccaggcctctggggctccaggcacaacgaacgccgcttcctcaggaacaccaagaagttcatctccctggggaagcatgccaagctctcgctgcaggagctgacgtggaagatgagcgtgcgggactgcgcttggctgcgcaggagcccaggggttggctgtgttccggccgcagagcaccgtctgcgtgaggagatcctggccaagttcctgcactggctgatgagtgtgtacgtcgtcgagctgctcaggtctttcttttatgtcacggagaccacgtttcaaaagaacaggctctttttctaccggaagagtgtctggagcaagttgcaaagcattggaatcagacagcacttgaagagggtgcagctgcgggagctgtcggaagcagaggtcaggcagcatcgggaagccaggcccgccctgctgacgtccagactccgcttcatccccaagcctgacgggctgcggccgattgtgaacatggactacgtcgtgggagccagaacgttccgcagagaaaagagggccgagcgtctcacctcgagggtgaaggcactgttcagcgtgctcaactacgagcgggcgcggcgccccggcctcctgggcgcctctgtgctgggcctggacgatatccacagggcctggcgcaccttcgtgctgcgtgtgcgggcccaggacccgccgcctgagctgtactttgtcaaggtggatgtgacgggcgcgtacgacaccatcccccaggacaggctcacggaggtcatcgccagcatcatcaaaccccagaacacgtactgcgtgcgtcggtatgccgtggtccagaaggccgcccatgggcacgtccgcaaggccttcaagagccacgtctctaccttgacagacctccagccgtacatgcgacagttcgtggctcacctgcaggagaccagcccgctgagggatgccgtcgtcatcgagcagagctcctccctgaatgaggccagcagtggcctcttcgacgtcttcctacgcttcatgtgccaccacgccgtgcgcatcaggggcaagtcctacgtccagtgccaggggatcccgcagggctccatcctctccacgctgctctgcagcctgtgctacggcgacatggagaacaagctgtttgcggggattcggcgggacgggctgctcctgcgtttggtggatgatttcttgttggtgacacctcacctcacccacgcgaaaaccttcctcaggaccctggtccgaggtgtccctgagtatggctgcgtggtgaacttgcggaagacagtggtgaacttccctgtagaagacgaggccctgggtggcacggcttttgttcagatgccggcccacggcctattcccctggtgcggcctgctgctggatacccggaccctggaggtgcagagcgactactccagctatgcccggacctccatcagagccagtctcaccttcaaccgcggcttcaaggctgggaggaacatgcgtcgcaaactctttggggtcttgcggctgaagtgtcacagcctgtttctggatttgcaggtgaacagcctccagacggtgtgcaccaacatctacaagatcctcctgctgcaggcgtacaggtttcacgcatgtgtgctgcagctcccatttcatcagcaagtttggaagaaccccacatttttcctgcgcgtcatctctgacacggcctccctctgctactccatcctgaaagccaagaacgcagggatgtcgctgggggccaagggcgccgccggccctctgccctccgaggccgtgcagtggctgtgccaccaagcattcctgctcaagctgactcgacaccgtgtcacctacgtgccactcctggggtcactcaggacagcccagacgcagctgagtcggaagctcccggggacgacgctgactgccctggaggccgcagccaacccggcactgccctcagacttcaagaccatcctggacggaagcggagccacgaacttctctctgttaaagcaagcaggagatgttgaagaaaaccccgggcctatggatgagacctccccaaggctggaagaagactggaaaaaagtacttcagcgagaagcaggctggcagtgtgctgctctggttggtgaagaccagcctctttgcccagatcttcctgaacttgatctttctgaactagatgtgaacgacttggatacagacagctttctgggtggactcaagtggtgcagtgaccaatcagaaataatatccaatcagtacaacaatgagccttcaaacatatttgagaagatagatgaagagaatgaggcaaacttgctagcagtcctcacagagacactagacagtctccctgtggatgaagacggattgccctcatttgatgcgctgacagatggagacgtgaccactgacaatgaggctagtccttcctccatgcctgacggcacccctccaccccaggaggcagaagagccgtctctacttaagaagctcttactggcaccagccaacactcagctaagttataatgaatgcagtggtctcagtacccagaaccatgcaaatcacaatcacaggatcagaacaaaccctgcaattgttaagactgagaattcatggagcaataaagcgaagagtatttgtcaacagcaaaagccacaaagacgtccctgctcggagcttctcaaatatctgaccacaaacgatgaccctcctcacaccaaacccacagagaacagaaacagcagcagagacaaatgcacctccaaaaagaagtcccacacacagtcgcagtcacaacacttacaagccaaaccaacaactttatctcttcctctgaccccagagtcaccaaatgaccccaagggttccccatttgagaacaagactattgaacgcaccttaagtgtggaactctctggaactgcaggcctaactccacccaccactcctcctcataaagccaaccaagataacccttttagggcttctccaaagctgaagtcctcttgcaagactgtggtgccaccaccatcaaagaagcccaggtacagtgagtcttctggtacacaaggcaataactccaccaagaaagggccggagcaatccgagttgtatgcacaactcagcaagtcctcagtcctcactggtggacacgaggaaaggaagaccaagcggcccagtctgcggctgtttggtgaccatgactattgccagtcaattaattccaaaacagaaatactcattaatatatcacaggagctccaagactctagacaactagaaaataaagatgtctcctctgattggcaggggcagatttgttcttccacagattcagaccagtgctacctgagagagactttggaggcaagcaagcaggtctctccttgcagcacaagaaaacagctccaagaccaggaaatccgagccgagctgaacaagcacttcggtcatcccagtcaagctgtttttgacgacgaagcagacaagaccggtgaactgagggacagtgatttcagtaatgaacaattctccaaactacctatgtttataaattcaggactagccatggatggcctgtttgatgacagcgaagatgaaagtgataaactgagctacccttgggatggcacgcaatcctattcattgttcaatgtgtctccttcttgttcttcttttaactctccatgtagagattctgtgtcaccacccaaatccttattttctcaaagaccccaaaggatgcgctctcgttcaaggtccttttctcgacacaggtcgtgttcccgatcaccatattccaggtcaagatcaaggtctccaggcagtagatcctcttcaagatcctgctattactatgagtcaagccactacagacaccgcacgcaccgaaattctcccttgtatgtgagatcacgttcaagatcgccctacagccgtcggcccaggtatgacagctacgaggaatatcagcacgagaggctgaagagggaagaatatcgcagagagtatgagaagcgagagtctgagagggccaagcaaagggagaggcagaggcagaaggcaattgaagagcgccgtgtgatttatgtcggtaaaatcagacctgacacaacacggacagaactgagggaccgttttgaagtttttggtgaaattgaggagtgcacagtaaatctgcgggatgatggagacagctatggtttcattacctaccgttatacctgtgatgcttttgctgctcttgaaaatggatacactttgcgcaggtcaaacgaaactgactttgagctgtacttttgtggacgcaagcaatttttcaagtctaactatgcagacctagattcaaactcagatgactttgaccctgcttccaccaagagcaagtatgactctctggattttgatagtttactgaaagaagctcagagaagcttgcgcaggggaagcggagagggcaggggaagtcttctaacatgcggggacgtggaggaaaatcccggccccatggcggggaacgactgcggcgcgctgctggacgaagagctctcctccttcttcctcaactatctcgctgacacgcagggtggagggtccggggaggagcaactctatgctgactttccagaacttgacctctcccagctggatgccagcgactttgactcggccacctgctttggggagctgcagtggtgcccagagaactcagagactgaacccaaccagtacagccccgatgactccgagctcttccagattgacagtgagaatgaggccctcctggcagagctcaccaagaccctggatgacatccctgaagatgacgtgggtctggctgccttcccagccctggatggtggagacgctctatcatgcacctcagcttcgcctgccccctcatctgcaccccccagccctgccccggagaagccctcggccccagcccctgaggtggacgagctctcactgctgcagaagctcctcctggccacatcctacccaacatcaagctctgacacccagaaggaagggaccgcctggcgccaggcaggcctcagatctaaaagtcaacggccttgtgttaaggcggacagcacccaagacaagaaggctcccatgatgcagtctcagagccgaagttgtacagaactacataagcacctcacctcggcacagtgctgcctgcaggatcggggtctgcagccaccatgcctccagagtccccggctccctgccaaggaggacaaggagccgggtgaggactgcccgagcccccagccagctccagcctctccccgggactccctagctctgggcagggcagaccccggtgccccggtttcccaggaagacatgcaggcgatggtgcaactcatacgctacatgcacacctactgcctcccccagaggaagctgcccccacagacccctgagccactccccaaggcctgcagcaacccctcccagcaggtcagatcccggccctggtcccggcaccactccaaagcctcctgggctgagttctccattctgagggaacttctggctcaagacgtgctctgtgatgtcagcaaaccctaccgtctggccacgcctgtttatgcctccctcacacctcggtcaaggcccaggccccccaaagacagtcaggcctcccctggtcgcccgtcctcggtggaggaggtaaggatcgcagcttcacccaagagcaccgggcccagaccaagcctgcgcccactgcggctggaggtgaaaagggaggtccgccggcctgccagactgcagcagcaggaggaggaagacgaggaagaagaggaggaggaagaggaagaagaaaaagaggaggaggaggagtggggcaggaaaaggccaggccgaggcctgccatggacgaagctggggaggaagctggagagctctgtgtgccccgtgcggcgttctcggagactgaaccctgagctgggcccctggctgacatttgcagatgagccgctggtcccctcggagccccaaggtgctctgccctcactgtgcctggctcccaaggcctacgacgtagagcgggagctgggcagccccacggacgaggacagtggccaagaccagcagctcctacggggaccccagatccctgccctggagagcccctgtgagagtgggtgtggggacatggatgaggaccccagctgcccgcagctccctcccagagactctcccaggtgcctcatgctggccttgtcacaaagcgacccaacttttggcaagaagagctttgagcagaccttgacagtggagctctgtggcacagcaggactcaccccacccaccacaccaccgtacaagcccacagaggaggatcccttcaaaccagacatcaagcatagtctaggcaaagaaatagctctcagcctcccctcccctgagggcctctcactcaaggccaccccaggggctgcccacaagctgccaaagaagcacccagagcgaagtgagctcctgtcccacctgcgacatgccacagcccagccagcctcccaggctggccagaagcgtcccttctcctgttcctttggagaccatgactactgccaggtgctccgaccagaaggcgtcctgcaaaggaaggtgctgaggtcctgggagccgtctggggttcaccttgaggactggccccagcagggtgccccttgggctgaggcacaggcccctggcagggaggaagacagaagctgtgatgctggcgccccacccaaggacagcacgctgctgagagaccatgagatccgtgccagcctcaccaaacactttgggctgctggagaccgccctggaggaggaagacctggcctcctgcaagagccctgagtatgacactgtctttgaagacagcagcagcagcagcggcgagagcagcttcctcccagaggaggaagaggaagaaggggaggaggaggaggaggacgatgaagaagaggactcaggggtcagccccacttgctctgaccactgcccctaccagagcccaccaagcaaggccaaccggcagctctgttcccgcagccgctcaagctctggctcttcaccctgccactcctggtcaccagccactcgaaggaacttcagatgtgagagcagagggccgtgttcagacagaacgccaagcatccggcacgccaggaagcggcgggaaaaggccattggggaaggccgcgtggtgtacattcaaaatctctccagcgacatgagctcccgagagctgaagaggcgctttgaagtgtttggtgagattgaggagtgcgaggtgctgacaagaaataggagaggcgagaagtacggcttcatcacctaccggtgttctgagcacgcggccctctctttgacaaagggcgctgccctgaggaagcgcaacgagccctccttccagctgagctacggagggctccggcacttctgctggcccagatacactgactacgattccaattcagaagaggcccttcctgcgtcagggaaaagcaagtatgaagccatggattttgacagcttactgaaagaggcccagcagagcctgcattgactgtgccttctagttgccagccatctgttgtttgcccctcccccgtgccttccttgaccctggaaggtgccactcccactgtcctttcctaataaaatgaggaaattgcatcgcattgtctgagtaggtgtcattctattctggggggtggggtggggcaggacagcaagggggaggattgggaagacaatagcaggcatgctggggatgcggtgggctctatggacccagctttcttgtacaaagtgggggttgcgccttttccaaggcagccctgggtttgcgcagggacgcggctgctctgggcgtggttccgggaaacgcagcggcgccgaccctgggtctcgcacattcttcacgtccgttcgcagcgtcacccggatcttcgccgctacccttgtgggccccccggcgacgcttcctgctccgcccctaagtcgggaaggttccttgcggttcgcggcgtgccggacgtgacaaacggaagccgcacgtctcactagtaccctcgcagacggacagcgccagggagcaatggcagcgcgccgaccgcgatgggctgtggccaatagcggctgctcagcagggcgcgccgagagcagcggccgggaaggggcggtgcgggaggcggggtgtggggcggtagtgtgggccctgttcctgcccgcgcggtgttccgcattctgcaagcctccggagcgcacgtcggcagtcggctccctcgttgaccgaatcaccgacctctctccccagggccaccatgaccgagtacaagcccacggtgcgcctcgccacccgcgacgacgtccccagggccgtacgcaccctcgccgccgcgttcgccgactaccccgccacgcgccacaccgtcgatccggaccgccacatcgagcgggtcaccgagctgcaagaactcttcctcacgcgcgtcgggctcgacatcggcaaggtgtgggtcgcggacgacggcgccgcggtggcggtctggaccacgccggagagcgtcgaagcgggggcggtgttcgccgagatcggcccgcgcatggccgagttgagcggttcccggctggccgcgcagcaacagatggaaggcctcctggcgccgcaccggcccaaggagcccgcgtggttcctggccaccgtcggcgtctcgcccgaccaccagggcaagggtctgggcagcgccgtcgtgctccccggagtggaggcggccgagcgcgccggggtgcccgccttcctggagacctccgcgccccgcaacctccccttctacgagcggctcggcttcaccgtcaccgccgacgtcgaggtgcccgaaggaccgcgcacctggtgcatgacccgcaagcccggtgcctgacaactttattatacatagttgatcctcaggtgcaggctgcctatcagaaggtggtggctggtgtggccaatgccctggctcacaaataccactgagatctttttccctctgccaaaaattatggggacatcatgaagccccttgagcatctgacttctggctaataaaggaaatttattttcattgcaatagtgtgttggaattttttgtgtctctcactcggaaggacatatgggagggcaaatcatttaaaacatcagaatgagtatttggtttagagtttggcaacatatgcccatatgctggctgccatgaacaaaggttggctataaagaggtcatcagtatatgaaacagccccctgctgtccattccttattccatagaaaagccttgacttgaggttagattttttttatattttgttttgtgttatttttttctttaacatccctaaaattttccttacatgttttactagccagatttttcctcctctcctgactactcccagtcatagctgtccctcttctcttatggagatccctcgacctgcagcccaagcttggatccctcgagttaattaacgagagcataatattgatatgtgccaaagttgtttctgactgactaataagtataatttgtttctattatgtataggttaagctaattacttattttataatacaacatgactgtttttaaagtacaaaataagtttatttttgtaaaagagagaatgtttaaaagttttgttactttatagaagaaattttgagtttttgtttttttttaataaataaataaacataaataaattgtttgttgaatttattattagtatgtaagtgtaaatataataaaacttaatatctattcaaattaataaataaacctcgatatacagaccgataaaacacatgcgtcaattttacgcatgattatctttaacgtacgtcacaatatgattatctttctagggttaaataatagtttctaatttttttattattcagcctgctgtcgtgaataccgagctccaattcgccctatagtgagtcgtattacaattcactggccgtcgttttacaacgtcgtgactgggaaaaccctggcgttacccaacttaatcgccttgcagcacatccccctttcgccagctggcgtaatagcgaagaggcccgcaccgatcgcccttcccaacagttgcgcagcctgaatggcgaatgggacgcgccctgtagcggcgcattaagcgcggcgggtgtggtggttacgcgcagcgtgaccgctacacttgccagcgccctagcgcccgctcctttcgctttcttcccttcctttctcgccacgttcgccggctttccccgtcaagctctaaatcgggggctccctttagggttccgatttagtgctttacggcacctcgaccccaaaaaacttgattagggtgatggttcacgtagtgggccatcgccctgatagacggtttttcgccctttgacgttggagtccacgttctttaatagtggactcttgttccaaactggaacaacactcaaccctatctcggtctattcttttgatttataagggattttgccgatttcggcctattggttaaaaaatgagctgatttaacaaaaatttaacgcgaattttaacaaaatattaacgcttacaattttaggtggcacttttcggggaaatgtgcgcggaacccctatttgtttatttttctaaatacattcaaatatgtatccgctcatgagacaataaccctgataaatgcttcaataatattgaaaaaggaagagtatgagtattcaacatttccgtgtcgcccttattcccttttttgcggcattttgccttcctgtttttgctcacccagaaacgctggtgaaagtaaaagatgctgaagatcagttgggtgcacgagtgggttacatcgaactggatctcaacagcggtaagatccttgagagttttcgccccgaagaacgttttccaatgatgagcacttttaaagttctgctatgtggcgcggtattatcccgtattgacgccgggcaagagcaactcggtcgccgcatacactattctcagaatgacttggttgagtactcaccagtcacagaaaagcatcttacggatggcatgacagtaagagaattatgcagtgctgccataaccatgagtgataacactgcggccaacttacttctgacaacgatcggaggaccgaaggagctaaccgcttttttgcacaacatgggggatcatgtaactcgccttgatcgttgggaaccggagctgaatgaagccataccaaacgacgagcgtgacaccacgatgcctgtagcaatggcaacaacgttgcgcaaactattaactggcgaactacttactctagcttcccggcaacaattaatagactggatggaggcggataaagttgcaggaccacttctgcgctcggcccttccggctggctggtttattgctgataaatctggagccggtgagcgtgggtctcgcggtatcattgcagcactggggccagatggtaagccctcccgtatcgtagttatctacacgacggggagtcaggcaactatggatgaacgaaatagacagatcgctgagataggtgcctcactgattaagcattggtaactgtcagaccaagtttactcatatatactttagattgatttaaaacttcatttttaatttaaaaggatctaggtgaagatcctttttgataatctcatgaccaaaatcccttaacgtgagttttcgttccactgagcgtcagaccccgtagaaaagatcaaaggatcttcttgagatcctttttttctgcgcgtaatctgctgcttgcaaacaaaaaaaccaccgctaccagcggtggtttgtttgccggatcaagagctaccaactctttttccgaaggtaactggcttcagcagagcgcagataccaaatactgttcttctagtgtagccgtagttaggccaccacttcaagaactctgtagcaccgcctacatacctcgctctgctaatcctgttaccagtggctgctgccagtggcgataagtcgtgtcttaccgggttggactcaagacgatagttaccggataaggcgcagcggtcgggctgaacggggggttcgtgcacacagcccagcttggagcgaacgacctacaccgaactgagatacctacagcgtgagctatgagaaagcgccacgcttcccgaagggagaaaggcggacaggtatccggtaagcggcagggtcggaacaggagagcgcacgagggagcttccagggggaaacgcctggtatctttatagtcctgtcgggtttcgccacctctgacttgagcgtcgatttttgtgatgctcgtcaggggggcggagcctatggaaaaacgccagcaacgcggcctttttacggttcctggccttttgctggccttttgctcacatgttctttcctgcgttatcccctgattctgtggataaccgtattaccgcctttgagtgagctgataccgctcgccgcagccgaacgaccgagcgcagcgagtcagtgagcgaggaagcggaagagcgcccaatacgcaaaccgcctctccccgcgcgttggccgattcattaatgcagctggcacgacaggtttcccgactggaaagcgggcagtgagcgcaacgcaattaatgtgagttagctcactcattaggcaccccaggctttacactttatgcttccggctcgtatgttgtgtggaattgtgagcggataacaatttcacacaggaaacagctatgaccatgattacgccaagctcgaaattaaccctcactaaagggaacaaaagctggtacctcgcgcgacttggtttgccattctttagcgcgcgtcgcgtcacacagcttggccacaatgtggtttttgtcaaacgaagattctatgacgtgtttaaagtttaggtcgagtaaagcgcaaatctttt

SEQ ID NO: 34 - DNA, 17715 bp, synthetic construct
  source 1..17715: mol_type = other DNA
ttaaccctagaaagatagtctgcgtaaaattgacgcatgcattcttgaaatattgctctctctttctaaatagcgcgaatccgtcgctgtgcatttaggacatctcagtcgccgcttggagctcccgtgaggcgtgcttgtcaatgcggtaagtgtcactgattttgaactataacgaccgcgtgagtcaaaatgacgcatgattatcttttacgtgacttttaagatttaactcatacgataattatattgttatttcatgttctacttacgtgataacttattatatatatattttcttgttatagatatcatcaactttgtatagaaaagttggacattgattattgactagttattaatagtaatcaattacggggtcattagttcatagcccatatatggagttccgcgttacataacttacggtaaatggcccgcctggctgaccgcccaacgacccccgcccattgacgtcaataatgacgtatgttcccatagtaacgccaatagggactttccattgacgtcaatgggtggagtatttacggtaaactgcccacttggcagtacatcaagtgtatcatatgccaagtacgccccctattgacgtcaatgacggtaaatggcccgcctggcattatgcccagtacatgaccttatgggactttcctacttggcagtacatctacgtattagtcatcgctattaccatggtgatgcggttttggcagtacatcaatgggcgtggatagcggtttgactcacggggatttccaagtctccaccccattgacgtcaatgggagtttgttttggcaccaaaatcaacgggactttccaaaatgtcgtaacaactccgccccattgacgcaaatgggcggtaggcgtgtacggtgggaggtctatataagcagagctcgtttagtgaaccgtcagatcgcctggagacgccatccacgctgttttgacctccatagaagacaccgggaccgatccagcctcccctcgaagcttacatgtggtaccgagctcggatcctgagaacttcagggtgagtctatgggacccttgatgttttctttccccttcttttctatggttaagttcatgtcataggaaggggagaagtaacagggtacacatattgaccaaatcagggtaattttgcatttgtaattttaaaaaatgctttcttcttttaatatacttttttgtttatcttatttctaatactttccctaatctctttctttcagggcaataatgatacaatgtatcatgcctctttgcaccattctaaagaataacagtgataatttctgggttaaggcaatagcaatatttctgcatataaatatttctgcatataaattgtaactgatgtaagaggtttcatattgctaatagcagctacaatccagctaccattctgcttttattttatggttgggataaggctggattattctgagtccaagctaggcccttttgctaatcatgttcatacctcttatcttcctcccacagctcctgggcaacgtgctggtctgtgtgctggcccatcactttggcaaagcaagtttgtacaaaaaagcaggctgccaccatgccgcgcgctccccgctgccgagccgtgcgctccctgctgcgcagccactaccgcgaggtgctgccgctggccacgttcgtgcggcgcctggggccccagggctggcggctggtgcagcgcggggacccggcggctttccgcgcgctggtggcccagtgcctggtgtgcgtgccctgggacgcacggccgccccccgccgccccctccttccgccaggtgtcctgcctgaaggagctggtggcccgagtgctgcagaggctgtgcgagcgcggcgcgaagaacgtgctggccttcggcttcgcgctgctggacggggcccgcgggggcccccccgaggccttcaccaccagcgtgcgcagctacctgcccaacacggtgaccgacgcactgcgggggagcggggcgtgggggctgctgctgcgccgcgtgggcgacgacgtgctggttcacctgctggcacgctgcgcgctctttgtgctggtggctcccagctgcgcctaccaggtgtgcgggccgccgctgtaccagctcggcgctgccactcaggcccggcccccgccacacgctagtggaccccgaaggcgtctgggatgcgaacgggcctggaaccatagcgtcagggaggccggggtccccctgggcctgccagccccgggtgcgaggaggcgcgggggcagtgccagccgaagtctgccgttgcccaagaggcccaggcgtggcgctgcccctgagccggagcggacgcccgttgggcaggggtcctgggcccacccgggcaggacgcgtggaccgagtgaccgtggtttctgtgtggtgtcacctgccagacccgccgaagaagccacctctttggagggtgcgctctctggcacgcgccactcccacccatccgtgggccgccagcaccacgcgggccccccatccacatcgcggccaccacgtccctgggacacgccttgtcccccggtgtacgccgagaccaagcacttcctctactcctcaggcgacaaggagcagctgcggccctccttcctactcagctctctgaggcccagcctgactggcgctcggaggctcgtggagaccatctttctgggttccaggccctggatgccagggactccccgcaggttgccccgcctgccccagcgctactggcaaatgcggcccctgtttctggagctgcttgggaaccacgcgcagtgcccctacggggtgctcctcaagacgcactgcccgctgcgagctgcggtcaccccagcagccggtgtctgtgcccgggagaagccccagggctctgtggcggcccccgaggaggaggacacagacccccgtcgcctggtgcagctgctccgccagcacagcagcccctggcaggtgtacggcttcgtgcgggcctgcctgcgccggctggtgcccccaggcctctggggctccaggcacaacgaacgccgcttcctcaggaacaccaagaagttcatctccctggggaagcatgccaagctctcgctgcaggagctgacgtggaagatgagcgtgcgggactgcgcttggctgcgcaggagcccaggggttggctgtgttccggccgcagagcaccgtctgcgtgaggagatcctggccaagttcctgcactggctgatgagtgtgtacgtcgtcgagctgctcaggtctttcttttatgtcacggagaccacgtttcaaaagaacaggctctttttctaccggaagagtgtctggagcaagttgcaaagcattggaatcagacagcacttgaagagggtgcagctgcgggagctgtcggaagcagaggtcaggcagcatcgggaagccaggcccgccctgctgacgtccagactccgcttcatccccaagcctgacgggctgcggccgattgtgaacatggactacgtcgtgggagccagaacgttccgcagagaaaagagggccgagcgtctcacctcgagggtgaaggcactgttcagcgtgctcaactacgagcgggcgcggcgccccggcctcctgggcgcctctgtgctgggcctggacgatatccacagggcctggcgcaccttcgtgctgcgtgtgcgggcccaggacccgccgcctgagctgtactttgtcaaggtggatgtgacgggcgcgtacgacaccatcccccaggacaggctcacggaggtcatcgccagcatcatcaaaccccagaacacgtactgcgtgcgtcggtatgccgtggtccagaaggccgcccatgggcacgtccgcaaggccttcaagagccacgtctctaccttgacagacctccagccgtacatgcgacagttcgtggctcacctgcaggagaccagcccgctgagggatgccgtcgtcatcgagcagagctcctccctgaatgaggccagcagtggcctcttcgacgtcttcctacgcttcatgtgccaccacgccgtgcgcatcaggggcaagtcctacgtccagtgccaggggatcccgcagggctccatcctctccacgctgctctgcagcctgtgctacggcgacatggagaacaagctgtttgcggggattcggcgggacgggctgctcctgcgtttggtggatgatttcttgttggtgacacctcacctcacccacgcgaaaaccttcctcaggaccctggtccgaggtgtccctgagtatggctgcgtggtgaacttgcggaagacagtggtgaacttccctgtagaagacgaggccctgggtggcacggcttttgttcagatgccggcccacggcctattcccctggtgcggcctgctgctggatacccggaccctggaggtgcagagcgactactccagctatgcccggacctccatcagagccagtctcaccttcaaccgcggcttcaaggctgggaggaacatgcgtcgcaaactctttggggtcttgcggctgaagtgtcacagcctgtttctggatttgcaggtgaacagcctccagacggtgtgcaccaacatctacaagatcctcctgctgcaggcgtacaggtttcacgcatgtgtgctgcagctcccatttcatcagcaagtttggaagaaccccacatttttcctgcgcgtcatctctgacacggcctccctctgctactccatcctgaaagccaagaacgcagggatgtcgctgggggccaagggcgccgccggccctctgccctccgaggccgtgcagtggctgtgccaccaagcattcctgctcaagctgactcgacaccgtgtcacctacgtgccactcctggggtcactcaggacagcccagacgcagctgagtcggaagctcccggggacgacgctgactgccctggaggccgcagccaacccggcactgccctcagacttcaagaccatcctggacggaagcggagccacgaacttctctctgttaaagcaagcaggagatgttgaagaaaaccccgggcctatggatgagacctccccaaggctggaagaagactggaaaaaagtacttcagcgagaagcaggctggcagtgtgctgctctggttggtgaagaccagcctctttgcccagatcttcctgaacttgatctttctgaactagatgtgaacgacttggatacagacagctttctgggtggactcaagtggtgcagtgaccaatcagaaataatatccaatcagtacaacaatgagccttcaaacatatttgagaagatagatgaagagaatgaggcaaacttgctagcagtcctcacagagacactagacagtctccctgtggatgaagacggattgccctcatttgatgcgctgacagatggagacgtgaccactgacaatgaggctagtccttcctccatgcctgacggcacccctccaccccaggaggcagaagagccgtctctacttaagaagctcttactggcaccagccaacactcagctaagttataatgaatgcagtggtctcagtacccagaaccatgcaaatcacaatcacaggatcagaacaaaccctgcaattgttaagactgagaattcatggagcaataaagcgaagagtatttgtcaacagcaaaagccacaaagacgtccctgctcggagcttctcaaatatctgaccacaaacgatgaccctcctcacaccaaacccacagagaacagaaacagcagcagagacaaatgcacctccaaaaagaagtcccacacacagtcgcagtcacaacacttacaagccaaaccaacaactttatctcttcctctgaccccagagtcaccaaatgaccccaagggttccccatttgagaacaagactattgaacgcaccttaagtgtggaactctctggaactgcaggcctaactccacccaccactcctcctcataaagccaaccaagataacccttttagggcttctccaaagctgaagtcctcttgcaagactgtggtgccaccaccatcaaagaagcccaggtacagtgagtcttctggtacacaaggcaataactccaccaagaaagggccggagcaatccgagttgtatgcacaactcagcaagtcctcagtcctcactggtggacacgaggaaaggaagaccaagcggcccagtctgcggctgtttggtgaccatgactattgccagtcaattaattccaaaacagaaatactcattaatatatcacaggagctccaagactctagacaactagaaaataaagatgtctcctctgattggcaggggcagatttgttcttccacagattcagaccagtgctacctgagagagactttggaggcaagcaagcaggtctctccttgcagcacaagaaaacagctccaagaccaggaaatccgagccgagctgaacaagcacttcggtcatcccagtcaagctgtttttgacgacgaagcagacaagaccggtgaactgagggacagtgatttcagtaatgaacaattctccaaactacctatgtttataaattcaggactagccatggatggcctgtttgatgacagcgaagatgaaagtgataaactgagctacccttgggatggcacgcaatcctattcattgttcaatgtgtctccttcttgttcttcttttaactctccatgtagagattctgtgtcaccacccaaatccttattttctcaaagaccccaaaggatgcgctctcgttcaaggtccttttctcgacacaggtcgtgttcccgatcaccatattccaggtcaagatcaaggtctccaggcagtagatcctcttcaagatcctgctattactatgagtcaagccactacagacaccgcacgcaccgaaattctcccttgtatgtgagatcacgttcaagatcgccctacagccgtcggcccaggtatgacagctacgaggaatatcagcacgagaggctgaagagggaagaatatcgcagagagtatgagaagcgagagtctgagagggccaagcaaagggagaggcagaggcagaaggcaattgaagagcgccgtgtgatttatgtcggtaaaatcagacctgacacaacacggacagaactgagggaccgttttgaagtttttggtgaaattgaggagtgcacagtaaatctgcgggatgatggagacagctatggtttcattacctaccgttatacctgtgatgcttttgctgctcttgaaaatggatacactttgcgcaggtcaaacgaaactgactttgagctgtacttttgtggacgcaagcaatttttcaagtctaactatgcagacctagattcaaactcagatgactttgaccctgcttccaccaagagcaagtatgactctctggattttgatagtttactgaaagaagctcagagaagcttgcgcaggggaagcggagagggcaggggaagtcttctaacatgcggggacgtggaggaaaatcccggccccatggcggggaacgactgcggcgcgctgctggacgaagagctctcctccttcttcctcaactatctcgctgacacgcagggtggagggtccggggaggagcaactctatgctgactttccagaacttgacctctcccagctggatgccagcgactttgactcggccacctgctttggggagctgcagtggtgcccagagaactcagagactgaacccaaccagtacagccccgatgactccgagctcttccagattgacagtgagaatgaggccctcctggcagagctcaccaagaccctggatgacatccctgaagatgacgtgggtctggctgccttcccagccctggatggtggagacgctctatcatgcacctcagcttcgcctgccccctcatctgcaccccccagccctgccccggagaagccctcggccccagcccctgaggtggacgagctctcactgctgcagaagctcctcctggccacatcctacccaacatcaagctctgacacccagaaggaagggaccgcctggcgccaggcaggcctcagatctaaaagtcaacggccttgtgttaaggcggacagcacccaagacaagaaggctcccatgatgcagtctcagagccgaagttgtacagaactacataagcacctcacctcggcacagtgctgcctgcaggatcggggtctgcagccaccatgcctccagagtccccggctccctgccaaggaggacaaggagccgggtgaggactgcccgagcccccagccagctccagcctctccccgggactccctagctctgggcagggcagaccccggtgccccggtttcccaggaagacatgcaggcgatggtgcaactcatacgctacatgcacacctactgcctcccccagaggaagctgcccccacagacccctgagccactccccaaggcctgcagcaacccctcccagcaggtcagatcccggccctggtcccggcaccactccaaagcctcctgggctgagttctccattctgagggaacttctggctcaagacgtgctctgtgatgtcagcaaaccctaccgtctggccacgcctgtttatgcctccctcacacctcggtcaaggcccaggccccccaaagacagtcaggcctcccctggtcgcccgtcctcggtggaggaggtaaggatcgcagcttcacccaagagcaccgggcccagaccaagcctgcgcccactgcggctggaggtgaaaagggaggtccgccggcctgccagactgcagcagcaggaggaggaagacgaggaagaagaggaggaggaagaggaagaagaaaaagaggaggaggaggagtggggcaggaaaaggccaggccgaggcctgccatggacgaagctggggaggaagctggagagctctgtgtgccccgtgcggcgttctcggagactgaaccctgagctgggcccctggctgacatttgcagatgagccgctggtcccctcggagccccaaggtgctctgccctcactgtgcctggctcccaaggcctacgacgtagagcgggagctgggcagccccacggacgaggacagtggccaagaccagcagctcctacggggaccccagatccctgccctggagagcccctgtgagagtgggtgtggggacatggatgaggaccccagctgcccgcagctccctcccagagactctcccaggtgcctcatgctggccttgtcacaaagcgacccaacttttggcaagaagagctttgagcagaccttgacagtggagctctgtggcacagcaggactcaccccacccaccacaccaccgtacaagcccacagaggaggatcccttcaaaccagacatcaagcatagtctaggcaaagaaatagctctcagcctcccctcccctgagggcctctcactcaaggccaccccaggggctgcccacaagctgccaaagaagcacccagagcgaagtgagctcctgtcccacctgcgacatgccacagcccagccagcctcccaggctggccagaagcgtcccttctcctgttcctttggagaccatgactactgccaggtgctccgaccagaaggcgtcctgcaaaggaaggtgctgaggtcctgggagccgtctggggttcaccttgaggactggccccagcagggtgccccttgggctgaggcacaggcccctggcagggaggaagacagaagctgtgatgctggcgccccacccaaggacagcacgctgctgagagaccatgagatccgtgccagcctcaccaaacactttgggctgctggagaccgccctggaggaggaagacctggcctcctgcaagagccctgagtatgacactgtctttgaagacagcagcagcagcagcggcgagagcagcttcctcccagaggaggaagaggaagaaggggaggaggaggaggaggacgatgaagaagaggactcaggggtcagccccacttgctctgaccactgcccctaccagagcccaccaagcaaggccaaccggcagctctgttcccgcagccgctcaagctctggctcttcaccctgccactcctggtcaccagccactcgaaggaacttcagatgtgagagcagagggccgtgttcagacagaacgccaagcatccggcacgccaggaagcggcgggaaaaggccattggggaaggccgcgtggtgtacattcaaaatctctccagcgacatgagctcccgagagctgaagaggcgctttgaagtgtttggtgagattgaggagtgcgaggtgctgacaagaaataggagaggcgagaagtacggcttcatcacctaccggtgttctgagcacgcggccctctctttgacaaagggcgctgccctgaggaagcgcaacgagccctccttccagctgagctacggagggctccggcacttctgctggcccagatacactgactacgattccaattcagaagaggcccttcctgcgtcagggaaaagcaagtatgaagccatggattttgacagcttactgaaagaggcccagcagagcctgcattgactgtgccttctagttgccagccatctgttgtttgcccctcccccgtgccttccttgaccctggaaggtgccactcccactgtcctttcctaataaaatgaggaaattgcatcgcattgtctgagtaggtgtcattctattctggggggtggggtggggcaggacagcaagggggaggattgggaagacaatagcaggcatgctggggatgcggtgggctctatggacccagctttcttgtacaaagtgggggttgcgccttttccaaggcagccctgggtttgcgcagggacgcggctgctctgggcgtggttccgggaaacgcagcggcgccgaccctgggtctcgcacattcttcacgtccgttcgcagcgtcacccggatcttcgccgctacccttgtgggccccccggcgacgcttcctgctccgcccctaagtcgggaaggttccttgcggttcgcggcgtgccggacgtgacaaacggaagccgcacgtctcactagtaccctcgcagacggacagcgccagggagcaatggcagcgcgccgaccgcgatgggctgtggccaatagcggctgctcagcagggcgcgccgagagcagcggccgggaaggggcggtgcgggaggcggggtgtggggcggtagtgtgggccctgttcctgcccgcgcggtgttccgcattctgcaagcctccggagcgcacgtcggcagtcggctccctcgttgaccgaatcaccgacctctctccccagggccaccatggaagacgccaaaaacataaagaaaggcccggcgccattctatccgctagaggatggaaccgctggagagcaactgcataaggctatgaagagatacgccctggttcctggaacaattgcttttacagatgcacatatcgaggtgaacatcacgtacgcggaatacttcgaaatgtccgttcggttggcagaagctatgaaacgatatgggctgaatacaaatcacagaatcgtcgtatgcagtgaaaactctcttcaattctttatgccggtgttgggcgcgttatttatcggagttgcagttgcgcccgcgaacgacatttataatgaacgtgaattgctcaacagtatgaacatttcgcagcctaccgtagtgtttgtttccaaaaaggggttgcaaaaaattttgaacgtgcaaaaaaaattaccaataatccagaaaattattatcatggattctaaaacggattaccagggatttcagtcgatgtacacgttcgtcacatctcatctacctcccggttttaatgaatacgattttgtaccagagtcctttgatcgtgacaaaacaattgcactgataatgaactcctctggatctactgggttacctaagggtgtggcccttccgcatagaactgcctgcgtcagattctcgcatgccagagatcctatttttggcaatcaaatcattccggatactgcgattttaagtgttgttccattccatcacggttttggaatgtttactacactcggatatttgatatgtggatttcgagtcgtcttaatgtatagatttgaagaagagctgtttttacgatcccttcaggattacaaaattcaaagtgcgttgctagtaccaaccctattttcattcttcgccaaaagcactctgattgacaaatacgatttatctaatttacacgaaattgcttctgggggcgcacctctttcgaaagaagtcggggaagcggttgcaaaacgcttccatcttccagggatacgacaaggatatgggctcactgagactacatcagctattctgattacacccgagggggatgataaaccgggcgcggtcggtaaagttgttccattttttgaagcgaaggttgtggatctggataccgggaaaacgctgggcgttaatcagagaggcgaattatgtgtcagaggacctatgattatgtccggttatgtaaacaatccggaagcgaccaacgccttgattgacaaggatggatggctacattctggagacatagcttactgggacgaagacgaacacttcttcatagttgaccgcttgaagtctttaattaaatacaaaggataccaggtggcccccgctgaattggagtcgatattgttacaacaccccaacatcttcgacgcgggcgtggcaggtcttcccgacgatgacgccggtgaacttcccgccgccgttgttgttttggagcacggaaagacgatgacggaaaaagagatcgtggattacgtcgccagtcaagtaacaaccgcgaaaaagttgcgcggaggagttgtgtttgtggacgaagtaccgaaaggtcttaccggaaaactcgacgcaagaaaaatcagagagatcctcataaaggccaagaagggcggaaagtccaaattgggaagcggagccacgaacttctctctgttaaagcaagcaggagatgttgaagaaaaccccgggcctatgaccgagtacaagcccacggtgcgcctcgccacccgcgacgacgtccccagggccgtacgcaccctcgccgccgcgttcgccgactaccccgccacgcgccacaccgtcgatccggaccgccacatcgagcgggtcaccgagctgcaagaactcttcctcacgcgcgtcgggctcgacatcggcaaggtgtgggtcgcggacgacggcgccgcggtggcggtctggaccacgccggagagcgtcgaagcgggggcggtgttcgccgagatcggcccgcgcatggccgagttgagcggttcccggctggccgcgcagcaacagatggaaggcctcctggcgccgcaccggcccaaggagcccgcgtggttcctggccaccgtcggcgtctcgcccgaccaccagggcaagggtctgggcagcgccgtcgtgctccccggagtggaggcggccgagcgcgccggggtgcccgccttcctggagacctccgcgccccgcaacctccccttctacgagcggctcggcttcaccgtcaccgccgacgtcgaggtgcccgaaggaccgcgcacctggtgcatgacccgcaagcccggtgcctgacaactttattatacatagttgatcctcaggtgcaggctgcctatcagaaggtggtggctggtgtggccaatgccctggctcacaaataccactgagatctttttccctctgccaaaaattatggggacatcatgaagccccttgagcatctgacttctggctaataaaggaaatttattttcattgcaatagtgtgttggaattttttgtgtctctcactcggaaggacatatgggagggcaaatcatttaaaacatcagaatgagtatttggtttagagtttggcaacatatgcccatatgctggctgccatgaacaaaggttggctataaagaggtcatcagtatatgaaacagccccctgctgtccattccttattccatagaaaagccttgacttgaggttagattttttttatattttgttttgtgttatttttttctttaacatccctaaaattttccttacatgttttactagccagatttttcctcctctcctgactactcccagtcatagctgtccctcttctcttatggagatccctcgacctgcagcccaagcttggatccctcgagttaattaacgagagcataatattgatatgtgccaaagttgtttctgactgactaataagtataatttgtttctattatgtataggttaagctaattacttattttataatacaacatgactgtttttaaagtacaaaataagtttatttttgtaaaagagagaatgtttaaaagttttgttactttatagaagaaattttgagtttttgtttttttttaataaataaataaacataaataaattgtttgttgaatttattattagtatgtaagtgtaaatataataaaacttaatatctattcaaattaataaataaacctcgatatacagaccgataaaacacatgcgtcaattttacgcatgattatctttaacgtacgtcacaatatgattatctttctagggttaaataatagtttctaatttttttattattcagcctgctgtcgtgaataccgagctccaattcgccctatagtgagtcgtattacaattcactggccgtcgttttacaacgtcgtgactgggaaaaccctggcgttacccaacttaatcgccttgcagcacatccccctttcgccagctggcgtaatagcgaagaggcccgcaccgatcgcccttcccaacagttgcgcagcctgaatggcgaatgggacgcgccctgtagcggcgcattaagcgcggcgggtgtggtggttacgcgcagcgtgaccgctacacttgccagcgccctagcgcccgctcctttcgctttcttcccttcctttctcgccacgttcgccggctttccccgtcaagctctaaatcgggggctccctttagggttccgatttagtgctttacggcacctcgaccccaaaaaacttgattagggtgatggttcacgtagtgggccatcgccctgatagacggtttttcgccctttgacgttggagtccacgttctttaatagtggactcttgttccaaactggaacaacactcaaccctatctcggtctattcttttgatttataagggattttgccgatttcggcctattggttaaaaaatgagctgatttaacaaaaatttaacgcgaattttaacaaaatattaacgcttacaattttaggtggcacttttcggggaaatgtgcgcggaacccctatttgtttatttttctaaatacattcaaatatgtatccgctcatgagacaataaccctgataaatgcttcaataatattgaaaaaggaagagtatgagtattcaacatttccgtgtcgcccttattcccttttttgcggcattttgccttcctgtttttgctcacccagaaacgctggtgaaagtaaaagatgctgaagatcagttgggtgcacgagtgggttacatcgaactggatctcaacagcggtaagatccttgagagttttcgccccgaagaacgttttccaatgatgagcacttttaaagttctgctatgtggcgcggtattatcccgtattgacgccgggcaagagcaactcggtcgccgcatacactattctcagaatgacttggttgagtactcaccagtcacagaaaagcatcttacggatggcatgacagtaagagaattatgcagtgctgccataaccatgagtgataacactgcggccaacttacttctgacaacgatcggaggaccgaaggagctaaccgcttttttgcacaacatgggggatcatgtaactcgccttgatcgttgggaaccggagctgaatgaagccataccaaacgacgagcgtgacaccacgatgcctgtagcaatggcaacaacgttgcgcaaactattaactggcgaactacttactctagcttcccggcaacaattaatagactggatggaggcggataaagttgcaggaccacttctgcgctcggcccttccggctggctggtttattgctgataaatctggagccggtgagcgtgggtctcgcggtatcattgcagcactggggccagatggtaagccctcccgtatcgtagttatctacacgacggggagtcaggcaactatggatgaacgaaatagacagatcgctgagataggtgcctcactgattaagcattggtaactgtcagaccaagtttactcatatatactttagattgatttaaaacttcatttttaatttaaaaggatctaggtgaagatcctttttgataatctcatgaccaaaatcccttaacgtgagttttcgttccactgagcgtcagaccccgtagaaaagatcaaaggatcttcttgagatcctttttttctgcgcgtaatctgctgcttgcaaacaaaaaaaccaccgctaccagcggtggtttgtttgccggatcaagagctaccaactctttttccgaaggtaactggcttcagcagagcgcagataccaaatactgttcttctagtgtagccgtagttaggccaccacttcaagaactctgtagcaccgcctacatacctcgctctgctaatcctgttaccagtggctgctgccagtggcgataagtcgtgtcttaccgggttggactcaagacgatagttaccggataaggcgcagcggtcgggctgaacggggggttcgtgcacacagcccagcttggagcgaacgacctacaccgaactgagatacctacagcgtgagctatgagaaagcgccacgcttcccgaagggagaaaggcggacaggtatccggtaagcggcagggtcggaacaggagagcgcacgagggagcttccagggggaaacgcctggtatctttatagtcctgtcgggtttcgccacctctgacttgagcgtcgatttttgtgatgctcgtcaggggggcggagcctatggaaaaacgccagcaacgcggcctttttacggttcctggccttttgctggccttttgctcacatgttctttcctgcgttatcccctgattctgtggataaccgtattaccgcctttgagtgagctgataccgctcgccgcagccgaacgaccgagcgcagcgagtcagtgagcgaggaagcggaagagcgcccaatacgcaaaccgcctctccccgcgcgttggccgattcattaatgcagctggcacgacaggtttcccgactggaaagcgggcagtgagcgcaacgcaattaatgtgagttagctcactcattaggcaccccaggctttacactttatgcttccggctcgtatgttgtgtggaattgtgagcggataacaatttcacacaggaaacagctatgaccatgattacgccaagctcgaaattaaccctcactaaagggaacaaaagctggtacctcgcgcgacttggtttgccattctttagcgcgcgtcgcgtcacacagcttggccacaatgtggtttttgtcaaacgaagattctatgacgtgtttaaagtttaggtcgagtaaagcgcaaatctttt

SEQ ID NO: 35 - DNA, 17346 bp, synthetic construct
  source 1..17346: mol_type = other DNA
ttaaccctagaaagatagtctgcgtaaaattgacgcatgcattcttgaaatattgctctctctttctaaatagcgcgaatccgtcgctgtgcatttaggacatctcagtcgccgcttggagctcccgtgaggcgtgcttgtcaatgcggtaagtgtcactgattttgaactataacgaccgcgtgagtcaaaatgacgcatgattatcttttacgtgacttttaagatttaactcatacgataattatattgttatttcatgttctacttacgtgataacttattatatatatattttcttgttatagatatcatcaactttgtatagaaaagttggacattgattattgactagttattaatagtaatcaattacggggtcattagttcatagcccatatatggagttccgcgttacataacttacggtaaatggcccgcctggctgaccgcccaacgacccccgcccattgacgtcaataatgacgtatgttcccatagtaacgccaatagggactttccattgacgtcaatgggtggagtatttacggtaaactgcccacttggcagtacatcaagtgtatcatatgccaagtacgccccctattgacgtcaatgacggtaaatggcccgcctggcattatgcccagtacatgaccttatgggactttcctacttggcagtacatctacgtattagtcatcgctattaccatggtgatgcggttttggcagtacatcaatgggcgtggatagcggtttgactcacggggatttccaagtctccaccccattgacgtcaatgggagtttgttttggcaccaaaatcaacgggactttccaaaatgtcgtaacaactccgccccattgacgcaaatgggcggtaggcgtgtacggtgggaggtctatataagcagagctcgtttagtgaaccgtcagatcgcctggagacgccatccacgctgttttgacctccatagaagacaccgggaccgatccagcctcccctcgaagcttacatgtggtaccgagctcggatcctgagaacttcagggtgagtctatgggacccttgatgttttctttccccttcttttctatggttaagttcatgtcataggaaggggagaagtaacagggtacacatattgaccaaatcagggtaattttgcatttgtaattttaaaaaatgctttcttcttttaatatacttttttgtttatcttatttctaatactttccctaatctctttctttcagggcaataatgatacaatgtatcatgcctctttgcaccattctaaagaataacagtgataatttctgggttaaggcaatagcaatatttctgcatataaatatttctgcatataaattgtaactgatgtaagaggtttcatattgctaatagcagctacaatccagctaccattctgcttttattttatggttgggataaggctggattattctgagtccaagctaggcccttttgctaatcatgttcatacctcttatcttcctcccacagctcctgggcaacgtgctggtctgtgtgctggcccatcactttggcaaagcaagtttgtacaaaaaagcaggctgccaccatgccgcgcgctccccgctgccgagccgtgcgctccctgctgcgcagccactaccgcgaggtgctgccgctggccacgttcgtgcggcgcctggggccccagggctggcggctggtgcagcgcggggacccggcggctttccgcgcgctggtggcccagtgcctggtgtgcgtgccctgggacgcacggccgccccccgccgccccctccttccgccaggtgtcctgcctgaaggagctggtggcccgagtgctgcagaggctgtgcgagcgcggcgcgaagaacgtgctggccttcggcttcgcgctgctggacggggcccgcgggggcccccccgaggccttcaccaccagcgtgcgcagctacctgcccaacacggtgaccgacgcactgcgggggagcggggcgtgggggctgctgctgcgccgcgtgggcgacgacgtgctggttcacctgctggcacgctgcgcgctctttgtgctggtggctcccagctgcgcctaccaggtgtgcgggccgccgctgtaccagctcggcgctgccactcaggcccggcccccgccacacgctagtggaccccgaaggcgtctgggatgcgaacgggcctggaaccatagcgtcagggaggccggggtccccctgggcctgccagccccgggtgcgaggaggcgcgggggcagtgccagccgaagtctgccgttgcccaagaggcccaggcgtggcgctgcccctgagccggagcggacgcccgttgggcaggggtcctgggcccacccgggcaggacgcgtggaccgagtgaccgtggtttctgtgtggtgtcacctgccagacccgccgaagaagccacctctttggagggtgcgctctctggcacgcgccactcccacccatccgtgggccgccagcaccacgcgggccccccatccacatcgcggccaccacgtccctgggacacgccttgtcccccggtgtacgccgagaccaagcacttcctctactcctcaggcgacaaggagcagctgcggccctccttcctactcagctctctgaggcccagcctgactggcgctcggaggctcgtggagaccatctttctgggttccaggccctggatgccagggactccccgcaggttgccccgcctgccccagcgctactggcaaatgcggcccctgtttctggagctgcttgggaaccacgcgcagtgcccctacggggtgctcctcaagacgcactgcccgctgcgagctgcggtcaccccagcagccggtgtctgtgcccgggagaagccccagggctctgtggcggcccccgaggaggaggacacagacccccgtcgcctggtgcagctgctccgccagcacagcagcccctggcaggtgtacggcttcgtgcgggcctgcctgcgccggctggtgcccccaggcctctggggctccaggcacaacgaacgccgcttcctcaggaacaccaagaagttcatctccctggggaagcatgccaagctctcgctgcaggagctgacgtggaagatgagcgtgcgggactgcgcttggctgcgcaggagcccaggggttggctgtgttccggccgcagagcaccgtctgcgtgaggagatcctggccaagttcctgcactggctgatgagtgtgtacgtcgtcgagctgctcaggtctttcttttatgtcacggagaccacgtttcaaaagaacaggctctttttctaccggaagagtgtctggagcaagttgcaaagcattggaatcagacagcacttgaagagggtgcagctgcgggagctgtcggaagcagaggtcaggcagcatcgggaagccaggcccgccctgctgacgtccagactccgcttcatccccaagcctgacgggctgcggccgattgtgaacatggactacgtcgtgggagccagaacgttccgcagagaaaagagggccgagcgtctcacctcgagggtgaaggcactgttcagcgtgctcaactacgagcgggcgcggcgccccggcctcctgggcgcctctgtgctgggcctggacgatatccacagggcctggcgcaccttcgtgctgcgtgtgcgggcccaggacccgccgcctgagctgtactttgtcaaggtggatgtgacgggcgcgtacgacaccatcccccaggacaggctcacggaggtcatcgccagcatcatcaaaccccagaacacgtactgcgtgcgtcggtatgccgtggtccagaaggccgcccatgggcacgtccgcaaggccttcaagagccacgtctctaccttgacagacctccagccgtacatgcgacagttcgtggctcacctgcaggagaccagcccgctgagggatgccgtcgtcatcgagcagagctcctccctgaatgaggccagcagtggcctcttcgacgtcttcctacgcttcatgtgccaccacgccgtgcgcatcaggggcaagtcctacgtccagtgccaggggatcccgcagggctccatcctctccacgctgctctgcagcctgtgctacggcgacatggagaacaagctgtttgcggggattcggcgggacgggctgctcctgcgtttggtggatgatttcttgttggtgacacctcacctcacccacgcgaaaaccttcctcaggaccctggtccgaggtgtccctgagtatggctgcgtggtgaacttgcggaagacagtggtgaacttccctgtagaagacgaggccctgggtggcacggcttttgttcagatgccggcccacggcctattcccctggtgcggcctgctgctggatacccggaccctggaggtgcagagcgactactccagctatgcccggacctccatcagagccagtctcaccttcaaccgcggcttcaaggctgggaggaacatgcgtcgcaaactctttggggtcttgcggctgaagtgtcacagcctgtttctggatttgcaggtgaacagcctccagacggtgtgcaccaacatctacaagatcctcctgctgcaggcgtacaggtttcacgcatgtgtgctgcagctcccatttcatcagcaagtttggaagaaccccacatttttcctgcgcgtcatctctgacacggcctccctctgctactccatcctgaaagccaagaacgcagggatgtcgctgggggccaagggcgccgccggccctctgccctccgaggccgtgcagtggctgtgccaccaagcattcctgctcaagctgactcgacaccgtgtcacctacgtgccactcctggggtcactcaggacagcccagacgcagctgagtcggaagctcccggggacgacgctgactgccctggaggccgcagccaacccggcactgccctcagacttcaagaccatcctggacggaagcggagccacgaacttctctctgttaaagcaagcaggagatgttgaagaaaaccccgggcctatggatgagacctccccaaggctggaagaagactggaaaaaagtacttcagcgagaagcaggctggcagtgtgctgctctggttggtgaagaccagcctctttgcccagatcttcctgaacttgatctttctgaactagatgtgaacgacttggatacagacagctttctgggtggactcaagtggtgcagtgaccaatcagaaataatatccaatcagtacaacaatgagccttcaaacatatttgagaagatagatgaagagaatgaggcaaacttgctagcagtcctcacagagacactagacagtctccctgtggatgaagacggattgccctcatttgatgcgctgacagatggagacgtgaccactgacaatgaggctagtccttcctccatgcctgacggcacccctccaccccaggaggcagaagagccgtctctacttaagaagctcttactggcaccagccaacactcagctaagttataatgaatgcagtggtctcagtacccagaaccatgcaaatcacaatcacaggatcagaacaaaccctgcaattgttaagactgagaattcatggagcaataaagcgaagagtatttgtcaacagcaaaagccacaaagacgtccctgctcggagcttctcaaatatctgaccacaaacgatgaccctcctcacaccaaacccacagagaacagaaacagcagcagagacaaatgcacctccaaaaagaagtcccacacacagtcgcagtcacaacacttacaagccaaaccaacaactttatctcttcctctgaccccagagtcaccaaatgaccccaagggttccccatttgagaacaagactattgaacgcaccttaagtgtggaactctctggaactgcaggcctaactccacccaccactcctcctcataaagccaaccaagataacccttttagggcttctccaaagctgaagtcctcttgcaagactgtggtgccaccaccatcaaagaagcccaggtacagtgagtcttctggtacacaaggcaataactccaccaagaaagggccggagcaatccgagttgtatgcacaactcagcaagtcctcagtcctcactggtggacacgaggaaaggaagaccaagcggcccagtctgcggctgtttggtgaccatgactattgccagtcaattaattccaaaacagaaatactcattaatatatcacaggagctccaagactctagacaactagaaaataaagatgtctcctctgattggcaggggcagatttgttcttccacagattcagaccagtgctacctgagagagactttggaggcaagcaagcaggtctctccttgcagcacaagaaaacagctccaagaccaggaaatccgagccgagctgaacaagcacttcggtcatcccagtcaagctgtttttgacgacgaagcagacaagaccggtgaactgagggacagtgatttcagtaatgaacaattctccaaactacctatgtttataaattcaggactagccatggatggcctgtttgatgacagcgaagatgaaagtgataaactgagctacccttgggatggcacgcaatcctattcattgttcaatgtgtctccttcttgttcttcttttaactctccatgtagagattctgtgtcaccacccaaatccttattttctcaaagaccccaaaggatgcgctctcgttcaaggtccttttctcgacacaggtcgtgttcccgatcaccatattccaggtcaagatcaaggtctccaggcagtagatcctcttcaagatcctgctattactatgagtcaagccactacagacaccgcacgcaccgaaattctcccttgtatgtgagatcacgttcaagatcgccctacagccgtcggcccaggtatgacagctacgaggaatatcagcacgagaggctgaagagggaagaatatcgcagagagtatgagaagcgagagtctgagagggccaagcaaagggagaggcagaggcagaaggcaattgaagagcgccgtgtgatttatgtcggtaaaatcagacctgacacaacacggacagaactgagggaccgttttgaagtttttggtgaaattgaggagtgcacagtaaatctgcgggatgatggagacagctatggtttcattacctaccgttatacctgtgatgcttttgctgctcttgaaaatggatacactttgcgcaggtcaaacgaaactgactttgagctgtacttttgtggacgcaagcaatttttcaagtctaactatgcagacctagattcaaactcagatgactttgaccctgcttccaccaagagcaagtatgactctctggattttgatagtttactgaaagaagctcagagaagcttgcgcaggtaactgtgccttctagttgccagccatctgttgtttgcccctcccccgtgccttccttgaccctggaaggtgccactcccactgtcctttcctaataaaatgaggaaattgcatcgcattgtctgagtaggtgtcattctattctggggggtggggtggggcaggacagcaagggggaggattgggaagacaatagcaggcatgctggggatgcggtgggctctatggggctccggtgcccgtcagtgggcagagcgcacatcgcccacagtccccgagaagttggggggaggggtcggcaattgaaccggtgcctagagaaggtggcgcggggtaaactgggaaagtgatgtcgtgtactggctccgcctttttcccgagggtgggggagaaccgtatataagtgcagtagtcgccgtgaacgttctttttcgcaacgggtttgccgccagaacacaggtaagtgccgtgtgtggttcccgcgggcctggcctctttacgggttatggcccttgcgtgccttgaattacttccacctggctgcagtacgtgattcttgatcccgagcttcgggttggaagtgggtgggagagttcgaggccttgcgcttaaggagccccttcgcctcgtgcttgagttgaggcctggcctgggcgctggggccgccgcgtgcgaatctggtggcaccttcgcgcctgtctcgctgctttcgataagtctctagccatttaaaatttttgatgacctgctgcgacgctttttttctggcaagatagtcttgtaaatgcgggccaagatctgcacactggtatttcggtttttggggccgcgggcggcgacggggcccgtgcgtcccagcgcacatgttcggcgaggcggggcctgcgagcgcggccaccgagaatcggacgggggtagtctcaagctggccggcctgctctggtgcctggtctcgcgccgccgtgtatcgccccgccctgggcggcaaggctggcccggtcggcaccagttgcgtgagcggaaagatggccgcttcccggccctgctgcagggagctcaaaatggaggacgcggcgctcgggagagcgggcgggtgagtcacccacacaaaggaaaagggcctttccgtcctcagccgtcgcttcatgtgactccacggagtaccgggcgccgtccaggcacctcgattagttctcgagcttttggagtacgtcgtctttaggttggggggaggggttttatgcgatggagtttccccacactgagtgggtggagactgaagttaggccagcttggcacttgatgtaattctccttggaatttgccctttttgagtttggatcttggttcattctcaagcctcagacagtggttcaaagtttttttcttccatttcaggtgtcgtgaacccagctttcttgtacaaagtgggccaccatggcggggaacgactgcggcgcgctgctggacgaagagctctcctccttcttcctcaactatctcgctgacacgcagggtggagggtccggggaggagcaactctatgctgactttccagaacttgacctctcccagctggatgccagcgactttgactcggccacctgctttggggagctgcagtggtgcccagagaactcagagactgaacccaaccagtacagccccgatgactccgagctcttccagattgacagtgagaatgaggccctcctggcagagctcaccaagaccctggatgacatccctgaagatgacgtgggtctggctgccttcccagccctggatggtggagacgctctatcatgcacctcagcttcgcctgccccctcatctgcaccccccagccctgccccggagaagccctcggccccagcccctgaggtggacgagctctcactgctgcagaagctcctcctggccacatcctacccaacatcaagctctgacacccagaaggaagggaccgcctggcgccaggcaggcctcagatctaaaagtcaacggccttgtgttaaggcggacagcacccaagacaagaaggctcccatgatgcagtctcagagccgaagttgtacagaactacataagcacctcacctcggcacagtgctgcctgcaggatcggggtctgcagccaccatgcctccagagtccccggctccctgccaaggaggacaaggagccgggtgaggactgcccgagcccccagccagctccagcctctccccgggactccctagctctgggcagggcagaccccggtgccccggtttcccaggaagacatgcaggcgatggtgcaactcatacgctacatgcacacctactgcctcccccagaggaagctgcccccacagacccctgagccactccccaaggcctgcagcaacccctcccagcaggtcagatcccggccctggtcccggcaccactccaaagcctcctgggctgagttctccattctgagggaacttctggctcaagacgtgctctgtgatgtcagcaaaccctaccgtctggccacgcctgtttatgcctccctcacacctcggtcaaggcccaggccccccaaagacagtcaggcctcccctggtcgcccgtcctcggtggaggaggtaaggatcgcagcttcacccaagagcaccgggcccagaccaagcctgcgcccactgcggctggaggtgaaaagggaggtccgccggcctgccagactgcagcagcaggaggaggaagacgaggaagaagaggaggaggaagaggaagaagaaaaagaggaggaggaggagtggggcaggaaaaggccaggccgaggcctgccatggacgaagctggggaggaagctggagagctctgtgtgccccgtgcggcgttctcggagactgaaccctgagctgggcccctggctgacatttgcagatgagccgctggtcccctcggagccccaaggtgctctgccctcactgtgcctggctcccaaggcctacgacgtagagcgggagctgggcagccccacggacgaggacagtggccaagaccagcagctcctacggggaccccagatccctgccctggagagcccctgtgagagtgggtgtggggacatggatgaggaccccagctgcccgcagctccctcccagagactctcccaggtgcctcatgctggccttgtcacaaagcgacccaacttttggcaagaagagctttgagcagaccttgacagtggagctctgtggcacagcaggactcaccccacccaccacaccaccgtacaagcccacagaggaggatcccttcaaaccagacatcaagcatagtctaggcaaagaaatagctctcagcctcccctcccctgagggcctctcactcaaggccaccccaggggctgcccacaagctgccaaagaagcacccagagcgaagtgagctcctgtcccacctgcgacatgccacagcccagccagcctcccaggctggccagaagcgtcccttctcctgttcctttggagaccatgactactgccaggtgctccgaccagaaggcgtcctgcaaaggaaggtgctgaggtcctgggagccgtctggggttcaccttgaggactggccccagcagggtgccccttgggctgaggcacaggcccctggcagggaggaagacagaagctgtgatgctggcgccccacccaaggacagcacgctgctgagagaccatgagatccgtgccagcctcaccaaacactttgggctgctggagaccgccctggaggaggaagacctggcctcctgcaagagccctgagtatgacactgtctttgaagacagcagcagcagcagcggcgagagcagcttcctcccagaggaggaagaggaagaaggggaggaggaggaggaggacgatgaagaagaggactcaggggtcagccccacttgctctgaccactgcccctaccagagcccaccaagcaaggccaaccggcagctctgttcccgcagccgctcaagctctggctcttcaccctgccactcctggtcaccagccactcgaaggaacttcagatgtgagagcagagggccgtgttcagacagaacgccaagcatccggcacgccaggaagcggcgggaaaaggccattggggaaggccgcgtggtgtacattcaaaatctctccagcgacatgagctcccgagagctgaagaggcgctttgaagtgtttggtgagattgaggagtgcgaggtgctgacaagaaataggagaggcgagaagtacggcttcatcacctaccggtgttctgagcacgcggccctctctttgacaaagggcgctgccctgaggaagcgcaacgagccctccttccagctgagctacggagggctccggcacttctgctggcccagatacactgactacgattccaattcagaagaggcccttcctgcgtcagggaaaagcaagtatgaagccatggattttgacagcttactgaaagaggcccagcagagcctgcattgacagacatgataagatacattgatgagtttggacaaaccacaactagaatgcagtgaaaaaaatgctttatttgtgaaatttgtgatgctattgctttatttgtaaccattataagctgcaataaacaagttaacaacaacaattgcattcattttatgtttcaggttcagggggaggtgtgggaggttttttaaagcaagtaaaacctctacaaatgtggtagggttgcgccttttccaaggcagccctgggtttgcgcagggacgcggctgctctgggcgtggttccgggaaacgcagcggcgccgaccctgggtctcgcacattcttcacgtccgttcgcagcgtcacccggatcttcgccgctacccttgtgggccccccggcgacgcttcctgctccgcccctaagtcgggaaggttccttgcggttcgcggcgtgccggacgtgacaaacggaagccgcacgtctcactagtaccctcgcagacggacagcgccagggagcaatggcagcgcgccgaccgcgatgggctgtggccaatagcggctgctcagcagggcgcgccgagagcagcggccgggaaggggcggtgcgggaggcggggtgtggggcggtagtgtgggccctgttcctgcccgcgcggtgttccgcattctgcaagcctccggagcgcacgtcggcagtcggctccctcgttgaccgaatcaccgacctctctccccagggccaccatgaccgagtacaagcccacggtgcgcctcgccacccgcgacgacgtccccagggccgtacgcaccctcgccgccgcgttcgccgactaccccgccacgcgccacaccgtcgatccggaccgccacatcgagcgggtcaccgagctgcaagaactcttcctcacgcgcgtcgggctcgacatcggcaaggtgtgggtcgcggacgacggcgccgcggtggcggtctggaccacgccggagagcgtcgaagcgggggcggtgttcgccgagatcggcccgcgcatggccgagttgagcggttcccggctggccgcgcagcaacagatggaaggcctcctggcgccgcaccggcccaaggagcccgcgtggttcctggccaccgtcggcgtctcgcccgaccaccagggcaagggtctgggcagcgccgtcgtgctccccggagtggaggcggccgagcgcgccggggtgcccgccttcctggagacctccgcgccccgcaacctccccttctacgagcggctcggcttcaccgtcaccgccgacgtcgaggtgcccgaaggaccgcgcacctggtgcatgacccgcaagcccggtgcctgacaactttattatacatagttgatcctcaggtgcaggctgcctatcagaaggtggtggctggtgtggccaatgccctggctcacaaataccactgagatctttttccctctgccaaaaattatggggacatcatgaagccccttgagcatctgacttctggctaataaaggaaatttattttcattgcaatagtgtgttggaattttttgtgtctctcactcggaaggacatatgggagggcaaatcatttaaaacatcagaatgagtatttggtttagagtttggcaacatatgcccatatgctggctgccatgaacaaaggttggctataaagaggtcatcagtatatgaaacagccccctgctgtccattccttattccatagaaaagccttgacttgaggttagattttttttatattttgttttgtgttatttttttctttaacatccctaaaattttccttacatgttttactagccagatttttcctcctctcctgactactcccagtcatagctgtccctcttctcttatggagatccctcgacctgcagcccaagcttggatccctcgagttaattaacgagagcataatattgatatgtgccaaagttgtttctgactgactaataagtataatttgtttctattatgtataggttaagctaattacttattttataatacaacatgactgtttttaaagtacaaaataagtttatttttgtaaaagagagaatgtttaaaagttttgttactttatagaagaaattttgagtttttgtttttttttaataaataaataaacataaataaattgtttgttgaatttattattagtatgtaagtgtaaatataataaaacttaatatctattcaaattaataaataaacctcgatatacagaccgataaaacacatgcgtcaattttacgcatgattatctttaacgtacgtcacaatatgattatctttctagggttaaataatagtttctaatttttttattattcagcctgctgtcgtgaataccgagctccaattcgccctatagtgagtcgtattacaattcactggccgtcgttttacaacgtcgtgactgggaaaaccctggcgttacccaacttaatcgccttgcagcacatccccctttcgccagctggcgtaatagcgaagaggcccgcaccgatcgcccttcccaacagttgcgcagcctgaatggcgaatgggacgcgccctgtagcggcgcattaagcgcggcgggtgtggtggttacgcgcagcgtgaccgctacacttgccagcgccctagcgcccgctcctttcgctttcttcccttcctttctcgccacgttcgccggctttccccgtcaagctctaaatcgggggctccctttagggttccgatttagtgctttacggcacctcgaccccaaaaaacttgattagggtgatggttcacgtagtgggccatcgccctgatagacggtttttcgccctttgacgttggagtccacgttctttaatagtggactcttgttccaaactggaacaacactcaaccctatctcggtctattcttttgatttataagggattttgccgatttcggcctattggttaaaaaatgagctgatttaacaaaaatttaacgcgaattttaacaaaatattaacgcttacaattttaggtggcacttttcggggaaatgtgcgcggaacccctatttgtttatttttctaaatacattcaaatatgtatccgctcatgagacaataaccctgataaatgcttcaataatattgaaaaaggaagagtatgagtattcaacatttccgtgtcgcccttattcccttttttgcggcattttgccttcctgtttttgctcacccagaaacgctggtgaaagtaaaagatgctgaagatcagttgggtgcacgagtgggttacatcgaactggatctcaacagcggtaagatccttgagagttttcgccccgaagaacgttttccaatgatgagcacttttaaagttctgctatgtggcgcggtattatcccgtattgacgccgggcaagagcaactcggtcgccgcatacactattctcagaatgacttggttgagtactcaccagtcacagaaaagcatcttacggatggcatgacagtaagagaattatgcagtgctgccataaccatgagtgataacactgcggccaacttacttctgacaacgatcggaggaccgaaggagctaaccgcttttttgcacaacatgggggatcatgtaactcgccttgatcgttgggaaccggagctgaatgaagccataccaaacgacgagcgtgacaccacgatgcctgtagcaatggcaacaacgttgcgcaaactattaactggcgaactacttactctagcttcccggcaacaattaatagactggatggaggcggataaagttgcaggaccacttctgcgctcggcccttccggctggctggtttattgctgataaatctggagccggtgagcgtgggtctcgcggtatcattgcagcactggggccagatggtaagccctcccgtatcgtagttatctacacgacggggagtcaggcaactatggatgaacgaaatagacagatcgctgagataggtgcctcactgattaagcattggtaactgtcagaccaagtttactcatatatactttagattgatttaaaacttcatttttaatttaaaaggatctaggtgaagatcctttttgataatctcatgaccaaaatcccttaacgtgagttttcgttccactgagcgtcagaccccgtagaaaagatcaaaggatcttcttgagatcctttttttctgcgcgtaatctgctgcttgcaaacaaaaaaaccaccgctaccagcggtggtttgtttgccggatcaagagctaccaactctttttccgaaggtaactggcttcagcagagcgcagataccaaatactgttcttctagtgtagccgtagttaggccaccacttcaagaactctgtagcaccgcctacatacctcgctctgctaatcctgttaccagtggctgctgccagtggcgataagtcgtgtcttaccgggttggactcaagacgatagttaccggataaggcgcagcggtcgggctgaacggggggttcgtgcacacagcccagcttggagcgaacgacctacaccgaactgagatacctacagcgtgagctatgagaaagcgccacgcttcccgaagggagaaaggcggacaggtatccggtaagcggcagggtcggaacaggagagcgcacgagggagcttccagggggaaacgcctggtatctttatagtcctgtcgggtttcgccacctctgacttgagcgtcgatttttgtgatgctcgtcaggggggcggagcctatggaaaaacgccagcaacgcggcctttttacggttcctggccttttgctggccttttgctcacatgttctttcctgcgttatcccctgattctgtggataaccgtattaccgcctttgagtgagctgataccgctcgccgcagccgaacgaccgagcgcagcgagtcagtgagcgaggaagcggaagagcgcccaatacgcaaaccgcctctccccgcgcgttggccgattcattaatgcagctggcacgacaggtttcccgactggaaagcgggcagtgagcgcaacgcaattaatgtgagttagctcactcattaggcaccccaggctttacactttatgcttccggctcgtatgttgtgtggaattgtgagcggataacaatttcacacaggaaacagctatgaccatgattacgccaagctcgaaattaaccctcactaaagggaacaaaagctggtacctcgcgcgacttggtttgccattctttagcgcgcgtcgcgtcacacagcttggccacaatgtggtttttgtcaaacgaagattctatgacgtgtttaaagtttaggtcgagtaaagcgcaaatctttt

SEQ ID NO: 36 - DNA, 7356 bp, synthetic construct
  source 1..7356: mol_type = other DNA
caactttgtatagaaaagttgctcgacattgattattgactagttattaatagtaatcaattacggggtcattagttcatagcccatatatggagttccgcgttacataacttacggtaaatggcccgcctggctgaccgcccaacgacccccgcccattgacgtcaataatgacgtatgttcccatagtaacgccaatagggactttccattgacgtcaatgggtggagtatttacggtaaactgcccacttggcagtacatcaagtgtatcatatgccaagtacgccccctattgacgtcaatgacggtaaatggcccgcctggcattatgcccagtacatgaccttatgggactttcctacttggcagtacatctacgtattagtcatcgctattaccatggtcgaggtgagccccacgttctgcttcactctccccatctcccccccctccccacccccaattttgtatttatttattttttaattattttgtgcagcgatgggggcggggggggggggggggcgcgcgccaggcggggcggggcggggcgaggggcggggcggggcgaggcggagaggtgcggcggcagccaatcagagcggcgcgctccgaaagtttccttttatggcgaggcggcggcggcggcggccctataaaaagcgaagcgcgcggcgggcgggagtcgctgcgcgctgccttcgccccgtgccccgctccgccgccgcctcgcgccgcccgccccggctctgactgaccgcgttactcccacaggtgagcgggcgggacggcccttctcctccgggctgtaattagcgcttggtttaatgacggcttgtttcttttctgtggctgcgtgaaagccttgaggggctccgggagggccctttgtgcggggggagcggctcggggggtgcgtgcgtgtgtgtgtgcgtggggagcgccgcgtgcggctccgcgctgcccggcggctgtgagcgctgcgggcgcggcgcggggctttgtgcgctccgcagtgtgcgcgaggggagcgcggccgggggcggtgccccgcggtgcggggggggctgcgaggggaacaaaggctgcgtgcggggtgtgtgcgtgggggggtgagcagggggtgtgggcgcgtcggtcgggctgcaaccccccctgcacccccctccccgagttgctgagcacggcccggcttcgggtgcggggctccgtacggggcgtggcgcggggctcgccgtgccgggcggggggtggcggcaggtgggggtgccgggcggggcggggccgcctcgggccggggagggctcgggggaggggcgcggcggcccccggagcgccggcggctgtcgaggcgcggcgagccgcagccattgccttttatggtaatcgtgcgagagggcgcagggacttcctttgtcccaaatctgtgcggagccgaaatctgggaggcgccgccgcaccccctctagcgggcgcggggcgaagcggtgcggcgccggcaggaaggaaatgggcggggagggccttcgtgcgtcgccgcgccgccgtccccttctccctctccagcctcggggctgtccgcggggggacggctgccttcgggggggacggggcagggcggggttcggcttctggcgtgtgaccggcggctctagagcctctgctaaccatgttcatgccttcttctttttcctacagctcctgggcaacgtgctggttattgtgctgtctcatcattttggcaaagaattgcaagtttgtacaaaaaagcaggctgccaccatgggtagttctttagacgatgagcatatcctctctgctcttctgcaaagcgatgacgagcttgttggtgaggattctgacagtgaaatatcagatcacgtaagtgaagatgacgtccagagcgatacagaagaagcgtttatagatgaggtacatgaagtgcagccaacgtcaagcggtagtgaaatattagacgaacaaaatgttattgaacaaccaggttcttcattggcttctaacagaatcttgaccttgccacagaggactattagaggtaagaataaacattgttggtcaacttcaaagtccacgaggcgtagccgagtctctgcactgaacattgtcagatctcaaagaggtccgacgcgtatgtgccgcaatatatatgacccacttttatgcttcaaactattttttactgatgagataatttcggaaattgtaaaatggacaaatgctgagatatcattgaaacgtcgggaatctatgacaggtgctacatttcgtgacacgaatgaagatgaaatctatgctttctttggtattctggtaatgacagcagtgagaaaagataaccacatgtccacagatgacctctttgatcgatctttgtcaatggtgtacgtctctgtaatgagtcgtgatcgttttgattttttgatacgatgtcttagaatggatgacaaaagtatacggcccacacttcgagaaaacgatgtatttactcctgttagaaaaatatgggatctctttatccatcagtgcatacaaaattacactccaggggctcatttgaccatagatgaacagttacttggttttagaggacggtgtccgtttaggatgtatatcccaaacaagccaagtaagtatggaataaaaatcctcatgatgtgtgacagtggtacgaagtatatgataaatggaatgccttatttgggaagaggaacacagaccaacggagtaccactcggtgaatactacgtgaaggagttatcaaagcctgtgcacggtagttgtcgtaatattacgtgtgacaattggttcacctcaatccctttggcaaaaaacttactacaagaaccgtataagttaaccattgtgggaaccgtgcgatcaaacaaacgcgagataccggaagtactgaaaaacagtcgctccaggccagtgggaacatcgatgttttgttttgacggaccccttactctcgtctcatataaaccgaagccagctaagatggtatacttattatcatcttgtgatgaggatgcttctatcaacgaaagtaccggtaaaccgcaaatggttatgtattataatcaaactaaaggcggagtggacacgctagaccaaatgtgttctgtgatgacctgcagtaggaagacgaataggtggcctatggcattattgtacggaatgataaacattgcctgcataaattcttttattatatacagccataatgtcagtagcaagggagaaaaggttcaaagtcgcaaaaaatttatgagaaacctttacatgagcctgacgtcatcgtttatgcgtaagcgtttagaagctcctactttgaagagatatttgcgcgataatatctctaatattttgccaaatgaagtgcctggtacatcagatgacagtactgaagagccagtaatgaaaaaacgtacttactgtacttactgcccctctaaaataaggcgaaaggcaaatgcatcgtgcaaaaaatgcaaaaaagttatttgtcgagagcataatattgatatgtgccaaagttgtttctgaacccagctttcttgtacaaagtggtgatggccggccgcttcgagcagacatgataagatacattgatgagtttggacaaaccacaactagaatgcagtgaaaaaaatgctttatttgtgaaatttgtgatgctattgctttatttgtaaccattataagctgcaataaacaagttaacaacaacaattgcattcattttatgtttcaggttcagggggaggtgtgggaggttttttaaagcaagtaaaacctctacaaatgtggtacgcgttgacattgattattgactagttattaatagtaatcaattacggggtcattagttcatagcccatatatggagttccgcgttacataacttacggtaaatggcccgcctggctgaccgcccaacgacccccgcccattgacgtcaataatgacgtatgttcccatagtaacgccaatagggactttccattgacgtcaatgggtggagtatttacggtaaactgcccacttggcagtacatcaagtgtatcatatgccaagtacgccccctattgacgtcaatgacggtaaatggcccgcctggcattatgcccagtacatgaccttatgggactttcctacttggcagtacatctacgtattagtcatcgctattaccatggtgatgcggttttggcagtacatcaatgggcgtggatagcggtttgactcacggggatttccaagtctccaccccattgacgtcaatgggagtttgttttggcaccaaaatcaacgggactttccaaaatgtcgtaacaactccgccccattgacgcaaatgggcggtaggcgtgtacggtgggaggtctatataagcagagctctctggctaactagagaacccactgcgccaccatgaccgagtacaagcccacggtgcgcctcgccacccgcgacgacgtccccagggccgtacgcaccctcgccgccgcgttcgccgactaccccgccacgcgccacaccgtcgatccggaccgccacatcgagcgggtcaccgagctgcaagaactcttcctcacgcgcgtcgggctcgacatcggcaaggtgtgggtcgcggacgacggcgccgcggtggcggtctggaccacgccggagagcgtcgaagcgggggcggtgttcgccgagatcggcccgcgcatggccgagttgagcggttcccggctggccgcgcagcaacagatggaaggcctcctggcgccgcaccggcccaaggagcccgcgtggttcctggccaccgtcggcgtctcgcccgaccaccagggcaagggtctgggcagcgccgtcgtgctccccggagtggaggcggccgagcgcgccggggtgcccgccttcctggagacctccgcgccccgcaacctccccttctacgagcggctcggcttcaccgtcaccgccgacgtcgaggtgcccgaaggaccgcgcacctggtgcatgacccgcaagcccggtgcctgactcgagtctagagggcccgtttaaacccgctgatcagcctcgactgtgccttctagttgccagccatctgttgtttgcccctcccccgtgccttccttgaccctggaaggtgccactcccactgtcctttcctaataaaatgaggaaattgcatcgcattgtctgagtaggtgtcattctattctggggggtggggtggggcaggacagcaagggggaggattgggaagacaatagcaggcatgctggggatgcggtgggctctatgggcggccgcggcgctcttccgcttcctcgctcactgactcgctgcgctcggtcgttcggctgcggcgagcggtatcagctcactcaaaggcggtaatacggttatccacagaatcaggggataacgcaggaaagaacatgtgagcaaaaggccagcaaaaggccaggaaccgtaaaaaggccgcgttgctggcgtttttccataggctccgcccccctgacgagcatcacaaaaatcgacgctcaagtcagaggtggcgaaacccgacaggactataaagataccaggcgtttccccctggaagctccctcgtgcgctctcctgttccgaccctgccgcttaccggatacctgtccgcctttctctcttcgggaagcgtggcgctttctcatagctcacgctgtaggtatctcagttcggtgtaggtcgttcgctccaagctgggctgtgtgcacgaaccccccgttcagcccgaccgctgcgccttatccggtaactatcgtcttgagtccaacccggtaagacacgacttatcgccactggcagcagccactggtaacaggattagcagagcgaggtatgtaggcggtgctacagagttcttgaagtggtggcctaactacggctacactagaagaacagtatttggtatctgcgctctgctgaagccagttaccttcggaaaaagagttggtagctcttgatccggcaaacaaaccaccgctggtagcggtggtttttttgtttgcaagcagcagattacgcgcagaaaaaaaggatctcaagaagatcctttgatcttttctacggggtctgacgctcagtggaacgaaaactcacgttaagggattttggtcatgagattatcaaaaaggatcttcacctagatccttttaaattaaaaatgaagttttaaatcaatctaaagtatatatgagtaaacttggtctgacagttaccaatgcttaatcagtgaggcacctatctcagcgatctgtctatttcgttcatccatagttgcctgactccccgtcgtgtagataactacgatacgggagggcttaccatctggccccagtgctgcaatgataccgcgagacccacgctcaccggctccagatttatcagcaataaaccagccagccggaagggccgagcgcagaagtggtcctgcaactttatccgcctccatccagtctattaattgttgccgggaagctagagtaagtagttcgccagttaatagtttgcgcaacgttgttgccattgctacaggcatcgtggtgtcacgctcgtcgtttggtatggcttcattcagctccggttcccaacgatcaaggcgagttacatgatcccccatgttgtgcaaaaaagcggttagctccttcggtcctccgatcgttgtcagaagtaagttggccgcagtgttatcactcatggttatggcagcactgcataattctcttactgtcatgccatccgtaagatgcttttctgtgactggtgagtactcaaccaagtcattctgagaatagtgtatgcggcgaccgagttgctcttgcccggcgtcaatacgggataataccgcgccacatagcagaactttaaaagtgctcatcattggaaaacgttcttcggggcgaaaactctcaaggatcttaccgctgttgagatccagttcgatgtaacccactcgtgcacccaactgatcttcagcatcttttactttcaccagcgtttctgggtgagcaaaaacaggaaggcaaaatgccgcaaaaaagggaataagggcgacacggaaatgttgaatactcatactcttcctttttcaatattattgaagcatttatcagggttattgtctcatgagcggatacatatttgaatgtatttagaaaaataaacaaataggggttccgcgcacatttccccgaaaagtgccacctgacgtctaagaaaccattattatcatgacattaacctataaaaataggcgtatcacgaggccctttcgtcggcgcgccgcggccgc

SEQ ID NO: 37 - DNA, 7467 bp, synthetic construct
  source 1..7467: mol_type = other DNA
caactttgtatagaaaagttgctcgacattgattattgactagttattaatagtaatcaattacggggtcattagttcatagcccatatatggagttccgcgttacataacttacggtaaatggcccgcctggctgaccgcccaacgacccccgcccattgacgtcaataatgacgtatgttcccatagtaacgccaatagggactttccattgacgtcaatgggtggagtatttacggtaaactgcccacttggcagtacatcaagtgtatcatatgccaagtacgccccctattgacgtcaatgacggtaaatggcccgcctggcattatgcccagtacatgaccttatgggactttcctacttggcagtacatctacgtattagtcatcgctattaccatggtcgaggtgagccccacgttctgcttcactctccccatctcccccccctccccacccccaattttgtatttatttattttttaattattttgtgcagcgatgggggcggggggggggggggggcgcgcgccaggcggggcggggcggggcgaggggcggggcggggcgaggcggagaggtgcggcggcagccaatcagagcggcgcgctccgaaagtttccttttatggcgaggcggcggcggcggcggccctataaaaagcgaagcgcgcggcgggcgggagtcgctgcgcgctgccttcgccccgtgccccgctccgccgccgcctcgcgccgcccgccccggctctgactgaccgcgttactcccacaggtgagcgggcgggacggcccttctcctccgggctgtaattagcgcttggtttaatgacggcttgtttcttttctgtggctgcgtgaaagccttgaggggctccgggagggccctttgtgcggggggagcggctcggggggtgcgtgcgtgtgtgtgtgcgtggggagcgccgcgtgcggctccgcgctgcccggcggctgtgagcgctgcgggcgcggcgcggggctttgtgcgctccgcagtgtgcgcgaggggagcgcggccgggggcggtgccccgcggtgcggggggggctgcgaggggaacaaaggctgcgtgcggggtgtgtgcgtgggggggtgagcagggggtgtgggcgcgtcggtcgggctgcaaccccccctgcacccccctccccgagttgctgagcacggcccggcttcgggtgcggggctccgtacggggcgtggcgcggggctcgccgtgccgggcggggggtggcggcaggtgggggtgccgggcggggcggggccgcctcgggccggggagggctcgggggaggggcgcggcggcccccggagcgccggcggctgtcgaggcgcggcgagccgcagccattgccttttatggtaatcgtgcgagagggcgcagggacttcctttgtcccaaatctgtgcggagccgaaatctgggaggcgccgccgcaccccctctagcgggcgcggggcgaagcggtgcggcgccggcaggaaggaaatgggcggggagggccttcgtgcgtcgccgcgccgccgtccccttctccctctccagcctcggggctgtccgcggggggacggctgccttcgggggggacggggcagggcggggttcggcttctggcgtgtgaccggcggctctagagcctctgctaaccatgttcatgccttcttctttttcctacagctcctgggcaacgtgctggttattgtgctgtctcatcattttggcaaagaattgcaagtttgtacaaaaaagcaggctgccaccatgggcagcagcctggacgacgagcacatcctgagcgccctgctgcagagcgacgacgagctggtcggcgaggacagcgacagcgaggtgagcgaccacgtgagcgaggacgacgtgcagtccgacaccgaggaggccttcatcgacgaggtgcacgaggtgcagcctaccagcagcggctccgagatcctggacgagcagaacgtgatcgagcagcccggcagctccctggccagcaacaggatcctgaccctgccccagaggaccatcaggggcaagaacaagcactgctggtccacctccaagcccaccaggcggagcagggtgtccgccctgaacatcgtgagaagccagaggggccccaccaggatgtgcaggaacatctacgaccccctgctgtgcttcaagctgttcttcaccgacgagatcatcagcgagatcgtgaagtggaccaacgccgagatcagcctgaagaggcgggagagcatgacctccgccaccttcagggacaccaacgaggacgagatctacgccttcttcggcatcctggtgatgaccgccgtgaggaaggacaaccacatgagcaccgacgacctgttcgacagatccctgagcatggtgtacgtgagcgtgatgagcagggacagattcgacttcctgatcagatgcctgaggatggacgacaagagcatcaggcccaccctgcgggagaacgacgtgttcacccccgtgagaaagatctgggacctgttcatccaccagtgcatccagaactacacccctggcgcccacctgaccatcgacgagcagctgctgggcttcaggggcaggtgccccttcagggtctatatccccaacaagcccagcaagtacggcatcaagatcctgatgatgtgcgacagcggcaccaagtacatgatcaacggcatgccctacctgggcaggggcacccagaccaacggcgtgcccctgggcgagtactacgtgaaggagctgtccaagcccgtccacggcagctgcagaaacatcacctgcgacaactggttcaccagcatccccctggccaagaacctgctgcaggagccctacaagctgaccatcgtgggcaccgtgagaagcaacaagagagagatccccgaggtcctgaagaacagcaggtccaggcccgtgggcaccagcatgttctgcttcgacggccccctgaccctggtgtcctacaagcccaagcccgccaagatggtgtacctgctgtccagctgcgacgaggacgccagcatcaacgagagcaccggcaagccccagatggtgatgtactacaaccagaccaagggcggcgtggacaccctggaccagatgtgcagcgtgatgacctgcagcagaaagaccaacaggtggcccatggccctgctgtacggcatgatcaacatcgcctgcatcaacagcttcatcatctacagccacaacgtgagcagcaagggcgagaaggtgcagagccggaaaaagttcatgcggaacctgtacatgggcctgacctccagcttcatgaggaagaggctggaggcccccaccctgaagagatacctgagggacaacatcagcaacatcctgcccaaagaggtgcccggcaccagcgacgacagcaccgaggagcccgtgatgaagaagaggacctactgcacctactgtcccagcaagatcagaagaaaggccagcgccagctgcaagaagtgtaagaaggtcatctgccgggagcacaacatcgacatgtgccagagctgtttctgaacccagctttcttgtacaaagtggtgatggccggccgcttcgagcagacatgataagatacattgatgagtttggacaaaccacaactagaatgcagtgaaaaaaatgctttatttgtgaaatttgtgatgctattgctttatttgtaaccattataagctgcaataaacaagttaacaacaacaattgcattcattttatgtttcaggttcagggggaggtgtgggaggttttttaaagcaagtaaaacctctacaaatgtggtacgcgttgacattgattattgactagttattaatagtaatcaattacggggtcattagttcatagcccatatatggagttccgcgttacataacttacggtaaatggcccgcctggctgaccgcccaacgacccccgcccattgacgtcaataatgacgtatgttcccatagtaacgccaatagggactttccattgacgtcaatgggtggagtatttacggtaaactgcccacttggcagtacatcaagtgtatcatatgccaagtacgccccctattgacgtcaatgacggtaaatggcccgcctggcattatgcccagtacatgaccttatgggactttcctacttggcagtacatctacgtattagtcatcgctattaccatggtgatgcggttttggcagtacatcaatgggcgtggatagcggtttgactcacggggatttccaagtctccaccccattgacgtcaatgggagtttgttttggcaccaaaatcaacgggactttccaaaatgtcgtaacaactccgccccattgacgcaaatgggcggtaggcgtgtacggtgggaggtctatataagcagagctctctggctaactagagaacccactgcgccaccatggtgagcaagggcgaggaggataacatggccatcatcaaggagttcatgcgcttcaaggtgcacatggagggctccgtgaacggccacgagttcgagatcgagggcgagggcgagggccgcccctacgagggcacccagaccgccaagctgaaggtgaccaagggtggccccctgcccttcgcctgggacatcctgtcccctcagttcatgtacggctccaaggcctacgtgaagcaccccgccgacatccccgactacttgaagctgtccttccccgagggcttcaagtgggagcgcgtgatgaacttcgaggacggcggcgtggtgaccgtgacccaggactcctccctgcaggacggcgagttcatctacaaggtgaagctgcgcggcaccaacttcccctccgacggccccgtaatgcagaagaagaccatgggctgggaggcctcctccgagcggatgtaccccgaggacggcgccctgaagggcgagatcaagcagaggctgaagctgaaggacggcggccactacgacgctgaggtcaagaccacctacaaggccaagaagcccgtgcagctgcccggcgcctacaacgtcaacatcaagttggacatcacctcccacaacgaggactacaccatcgtggaacagtacgaacgcgccgagggccgccactccaccggcggcatggacgagctgtacaagtaactcgagtctagagggcccgtttaaacccgctgatcagcctcgactgtgccttctagttgccagccatctgttgtttgcccctcccccgtgccttccttgaccctggaaggtgccactcccactgtcctttcctaataaaatgaggaaattgcatcgcattgtctgagtaggtgtcattctattctggggggtggggtggggcaggacagcaagggggaggattgggaagacaatagcaggcatgctggggatgcggtgggctctatgggcggccgcggcgctcttccgcttcctcgctcactgactcgctgcgctcggtcgttcggctgcggcgagcggtatcagctcactcaaaggcggtaatacggttatccacagaatcaggggataacgcaggaaagaacatgtgagcaaaaggccagcaaaaggccaggaaccgtaaaaaggccgcgttgctggcgtttttccataggctccgcccccctgacgagcatcacaaaaatcgacgctcaagtcagaggtggcgaaacccgacaggactataaagataccaggcgtttccccctggaagctccctcgtgcgctctcctgttccgaccctgccgcttaccggatacctgtccgcctttctcccttcgggaagcgtggcgctttctcatagctcacgctgtaggtatctcagttcggtgtaggtcgttcgctccaagctgggctgtgtgcacgaaccccccgttcagcccgaccgctgcgccttatccggtaactatcgtcttgagtccaacccggtaagacacgacttatcgccactggcagcagccactggtaacaggattagcagagcgaggtatgtaggcggtgctacagagttcttgaagtggtggcctaactacggctacactagaagaacagtatttggtatctgcgctctgctgaagccagttaccttcggaaaaagagttggtagctcttgatccggcaaacaaaccaccgctggtagcggtggtttttttgtttgcaagcagcagattacgcgcagaaaaaaaggatctcaagaagatcctttgatcttttctacggggtctgacgctcagtggaacgaaaactcacgttaagggattttggtcatgagattatcaaaaaggatcttcacctagatccttttaaattaaaaatgaagttttaaatcaatctaaagtatatatgagtaaacttggtctgacagttaccaatgcttaatcagtgaggcacctatctcagcgatctgtctatttcgttcatccatagttgcctgactccccgtcgtgtagataactacgatacgggagggcttaccatctggccccagtgctgcaatgataccgcgagacccacgctcaccggctccagatttatcagcaataaaccagccagccggaagggccgagcgcagaagtggtcctgcaactttatccgcctccatccagtctattaattgttgccgggaagctagagtaagtagttcgccagttaatagtttgcgcaacgttgttgccattgctacaggcatcgtggtgtcacgctcgtcgtttggtatggcttcattcagctccggttcccaacgatcaaggcgagttacatgatcccccatgttgtgcaaaaaagcggttagctccttcggtcctccgatcgttgtcagaagtaagttggccgcagtgttatcactcatggttatggcagcactgcataattctcttactgtcatgccatccgtaagatgcttttctgtgactggtgagtactcaaccaagtcattctgagaatagtgtatgcggcgaccgagttgctcttgcccggcgtcaatacgggataataccgcgccacatagcagaactttaaaagtgctcatcattggaaaacgttcttcggggcgaaaactctcaaggatcttaccgctgttgagatccagttcgatgtaacccactcgtgcacccaactgatcttcagcatcttttactttcaccagcgtttctgggtgagcaaaaacaggaaggcaaaatgccgcaaaaaagggaataagggcgacacggaaatgttgaatactcatactcttcctttttcaatattattgaagcatttatcagggttattgtctcatgagcggatacatatttgaatgtatttagaaaaataaacaaataggggttccgcgcacatttccccgaaaagtgccacctgacgtctaagaaaccattattatcatgacattaacctataaaaataggcgtatcacgaggccctttcgtcggcgcgccgcggccgc

SEQ ID NO: 38 - DNA, 5866 bp, synthetic construct
  source 1..5866: mol_type = other DNA
caactttgtatagaaaagttgctcgacattgattattgactagttattaatagtaatcaattacggggtcattagttcatagcccatatatggagttccgcgttacataacttacggtaaatggcccgcctggctgaccgcccaacgacccccgcccattgacgtcaataatgacgtatgttcccatagtaacgccaatagggactttccattgacgtcaatgggtggagtatttacggtaaactgcccacttggcagtacatcaagtgtatcatatgccaagtacgccccctattgacgtcaatgacggtaaatggcccgcctggcattatgcccagtacatgaccttatgggactttcctacttggcagtacatctacgtattagtcatcgctattaccatggtcgaggtgagccccacgttctgcttcactctccccatctcccccccctccccacccccaattttgtatttatttattttttaattattttgtgcagcgatgggggcggggggggggggggggcgcgcgccaggcggggcggggcggggcgaggggcggggcggggcgaggcggagaggtgcggcggcagccaatcagagcggcgcgctccgaaagtttccttttatggcgaggcggcggcggcggcggccctataaaaagcgaagcgcgcggcgggcgggagtcgctgcgcgctgccttcgccccgtgccccgctccgccgccgcctcgcgccgcccgccccggctctgactgaccgcgttactcccacaggtgagcgggcgggacggcccttctcctccgggctgtaattagcgcttggtttaatgacggcttgtttcttttctgtggctgcgtgaaagccttgaggggctccgggagggccctttgtgcggggggagcggctcggggggtgcgtgcgtgtgtgtgtgcgtggggagcgccgcgtgcggctccgcgctgcccggcggctgtgagcgctgcgggcgcggcgcggggctttgtgcgctccgcagtgtgcgcgaggggagcgcggccgggggcggtgccccgcggtgcggggggggctgcgaggggaacaaaggctgcgtgcggggtgtgtgcgtgggggggtgagcagggggtgtgggcgcgtcggtcgggctgcaaccccccctgcacccccctccccgagttgctgagcacggcccggcttcgggtgcggggctccgtacggggcgtggcgcggggctcgccgtgccgggcggggggtggcggcaggtgggggtgccgggcggggcggggccgcctcgggccggggagggctcgggggaggggcgcggcggcccccggagcgccggcggctgtcgaggcgcggcgagccgcagccattgccttttatggtaatcgtgcgagagggcgcagggacttcctttgtcccaaatctgtgcggagccgaaatctgggaggcgccgccgcaccccctctagcgggcgcggggcgaagcggtgcggcgccggcaggaaggaaatgggcggggagggccttcgtgcgtcgccgcgccgccgtccccttctccctctccagcctcggggctgtccgcggggggacggctgccttcgggggggacggggcagggcggggttcggcttctggcgtgtgaccggcggctctagagcctctgctaaccatgttcatgccttcttctttttcctacagctcctgggcaacgtgctggttattgtgctgtctcatcattttggcaaagaattgcaagtttgtacaaaaaagcaggctgccaccatgggtagttctttagacgatgagcatatcctctctgctcttctgcaaagcgatgacgagcttgttggtgaggattctgacagtgaaatatcagatcacgtaagtgaagatgacgtccagagcgatacagaagaagcgtttatagatgaggtacatgaagtgcagccaacgtcaagcggtagtgaaatattagacgaacaaaatgttattgaacaaccaggttcttcattggcttctaacagaatcttgaccttgccacagaggactattagaggtaagaataaacattgttggtcaacttcaaagtccacgaggcgtagccgagtctctgcactgaacattgtcagatctcaaagaggtccgacgcgtatgtgccgcaatatatatgacccacttttatgcttcaaactattttttactgatgagataatttcggaaattgtaaaatggacaaatgctgagatatcattgaaacgtcgggaatctatgacaggtgctacatttcgtgacacgaatgaagatgaaatctatgctttctttggtattctggtaatgacagcagtgagaaaagataaccacatgtccacagatgacctctttgatcgatctttgtcaatggtgtacgtctctgtaatgagtcgtgatcgttttgattttttgatacgatgtcttagaatggatgacaaaagtatacggcccacacttcgagaaaacgatgtatttactcctgttagaaaaatatgggatctctttatccatcagtgcatacaaaattacactccaggggctcatttgaccatagatgaacagttacttggttttagaggacggtgtccgtttaggatgtatatcccaaacaagccaagtaagtatggaataaaaatcctcatgatgtgtgacagtggtacgaagtatatgataaatggaatgccttatttgggaagaggaacacagaccaacggagtaccactcggtgaatactacgtgaaggagttatcaaagcctgtgcacggtagttgtcgtaatattacgtgtgacaattggttcacctcaatccctttggcaaaaaacttactacaagaaccgtataagttaaccattgtgggaaccgtgcgatcaaacaaacgcgagataccggaagtactgaaaaacagtcgctccaggccagtgggaacatcgatgttttgttttgacggaccccttactctcgtctcatataaaccgaagccagctaagatggtatacttattatcatcttgtgatgaggatgcttctatcaacgaaagtaccggtaaaccgcaaatggttatgtattataatcaaactaaaggcggagtggacacgctagaccaaatgtgttctgtgatgacctgcagtaggaagacgaataggtggcctatggcattattgtacggaatgataaacattgcctgcataaattcttttattatatacagccataatgtcagtagcaagggagaaaaggttcaaagtcgcaaaaaatttatgagaaacctttacatgagcctgacgtcatcgtttatgcgtaagcgtttagaagctcctactttgaagagatatttgcgcgataatatctctaatattttgccaaatgaagtgcctggtacatcagatgacagtactgaagagccagtaatgaaaaaacgtacttactgtacttactgcccctctaaaataaggcgaaaggcaaatgcatcgtgcaaaaaatgcaaaaaagttatttgtcgagagcataatattgatatgtgccaaagttgtttctgaacccagctttcttgtacaaagtggtgatggccggccgcttcgagcagacatgataagatacattgatgagtttggacaaaccacaactagaatgcagtgaaaaaaatgctttatttgtgaaatttgtgatgctattgctttatttgtaaccattataagctgcaataaacaagttaacaacaacaattgcattcattttatgtttcaggttcagggggaggtgtgggaggttttttaaagcaagtaaaacctctacaaatgtggtagcggccgcggcgctcttccgcttcctcgctcactgactcgctgcgctcggtcgttcggctgcggcgagcggtatcagctcactcaaaggcggtaatacggttatccacagaatcaggggataacgcaggaaagaacatgtgagcaaaaggccagcaaaaggccaggaaccgtaaaaaggccgcgttgctggcgtttttccataggctccgcccccctgacgagcatcacaaaaatcgacgctcaagtcagaggtggcgaaacccgacaggactataaagataccaggcgtttccccctggaagctccctcgtgcgctctcctgttccgaccctgccgcttaccggatacctgtccgcctttctctcttcgggaagcgtggcgctttctcatagctcacgctgtaggtatctcagttcggtgtaggtcgttcgctccaagctgggctgtgtgcacgaaccccccgttcagcccgaccgctgcgccttatccggtaactatcgtcttgagtccaacccggtaagacacgacttatcgccactggcagcagccactggtaacaggattagcagagcgaggtatgtaggcggtgctacagagttcttgaagtggtggcctaactacggctacactagaagaacagtatttggtatctgcgctctgctgaagccagttaccttcggaaaaagagttggtagctcttgatccggcaaacaaaccaccgctggtagcggtggtttttttgtttgcaagcagcagattacgcgcagaaaaaaaggatctcaagaagatcctttgatcttttctacggggtctgacgctcagtggaacgaaaactcacgttaagggattttggtcatgagattatcaaaaaggatcttcacctagatccttttaaattaaaaatgaagttttaaatcaatctaaagtatatatgagtaaacttggtctgacagttaccaatgcttaatcagtgaggcacctatctcagcgatctgtctatttcgttcatccatagttgcctgactccccgtcgtgtagataactacgatacgggagggcttaccatctggccccagtgctgcaatgataccgcgagacccacgctcaccggctccagatttatcagcaataaaccagccagccggaagggccgagcgcagaagtggtcctgcaactttatccgcctccatccagtctattaattgttgccgggaagctagagtaagtagttcgccagttaatagtttgcgcaacgttgttgccattgctacaggcatcgtggtgtcacgctcgtcgtttggtatggcttcattcagctccggttcccaacgatcaaggcgagttacatgatcccccatgttgtgcaaaaaagcggttagctccttcggtcctccgatcgttgtcagaagtaagttggccgcagtgttatcactcatggttatggcagcactgcataattctcttactgtcatgccatccgtaagatgcttttctgtgactggtgagtactcaaccaagtcattctgagaatagtgtatgcggcgaccgagttgctcttgcccggcgtcaatacgggataataccgcgccacatagcagaactttaaaagtgctcatcattggaaaacgttcttcggggcgaaaactctcaaggatcttaccgctgttgagatccagttcgatgtaacccactcgtgcacccaactgatcttcagcatcttttactttcaccagcgtttctgggtgagcaaaaacaggaaggcaaaatgccgcaaaaaagggaataagggcgacacggaaatgttgaatactcatactcttcctttttcaatattattgaagcatttatcagggttattgtctcatgagcggatacatatttgaatgtatttagaaaaataaacaaataggggttccgcgcacatttccccgaaaagtgccacctgacgtctaagaaaccattattatcatgacattaacctataaaaataggcgtatcacgaggccctttcgtcggcgcgccgcggccgc

SEQ ID NO: 39 - protein, 803 aa, Homo sapiens
MDETSPRLEEDWKKVLQREAGWQCAALVGEDQPLCPDLPELDLSELDVNDLDTDSFLGGLKWCSDQSEIISNQYNNEPSNIFEKIDEENEANLLAVLTETLDSLPVDEDGLPSFDALTDGDVTTDNEASPSSMPDGTPPPQEAEEPSLLKKLLLAPANTQLSYNECSGLSTQNHANHNHRIRTNPAIVKTENSWSNKAKSICQQQKPQRRPCSELLKYLTTNDDPPHTKPTENRNSSRDKCTSKKKSHTQSQSQHLQAKPTTLSLPLTPESPNDPKGSPFENKTIERTLSVELSGTAGLTPPTTPPHKANQDNPFRASPKLKSSCKTVVPPPSKKPRYSESSGTQGNNSTKKGPEQSELYAQLSKSSVLTGGHEERKTKRPSLRLFGDHDYCQSINSKTEILINISQELQDSRQLENKDVSSDWQGQICSSTDSDQCYLRETLEASKQVSPCSTRKQLQDQEIRAELNKHFGHPSQAVFDDEADKTGELRDSDFSNEQFSKLPMFINSGLAMDGLFDDSEDESDKLSYPWDGTQSYSLFNVSPSCSSFNSPCRDSVSPPKSLFSQRPQRMRSRSRSFSRHRSCSRSPYSRSRSRSPGSRSSSRSCYYYESSHYRHRTHRNSPLYVRSRSRSPYSRRPRYDSYEEYQHERLKREEYRREYEKRESERAKQRERQRQKAIEERRVIYVGKIRPDTTRTELRDRFEVFGEIEECTVNLRDDGDSYGFITYRYTCDAFAALENGYTLRRSNETDFELYFCGRKQFFKSNYADLDSNSDDFDPASTKSKYDSLDFDSLLKEAQRSLRR

SEQ ID NO: 40 - protein, 798 aa, Homo sapiens
MAWDMCNQDSESVWSDIECAALVGEDQPLCPDLPELDLSELDVNDLDTDSFLGGLKWCSDQSEIISNQYNNEPSNIFEKIDEENEANLLAVLTETLDSLPVDEDGLPSFDALTDGDVTTDNEASPSSMPDGTPPPQEAEEPSLLKKLLLAPANTQLSYNECSGLSTQNHANHNHRIRTNPAIVKTENSWSNKAKSICQQQKPQRRPCSELLKYLTTNDDPPHTKPTENRNSSRDKCTSKKKSHTQSQSQHLQAKPTTLSLPLTPESPNDPKGSPFENKTIERTLSVELSGTAGLTPPTTPPHKANQDNPFRASPKLKSSCKTVVPPPSKKPRYSESSGTQGNNSTKKGPEQSELYAQLSKSSVLTGGHEERKTKRPSLRLFGDHDYCQSINSKTEILINISQELQDSRQLENKDVSSDWQGQICSSTDSDQCYLRETLEASKQVSPCSTRKQLQDQEIRAELNKHFGHPSQAVFDDEADKTGELRDSDFSNEQFSKLPMFINSGLAMDGLFDDSEDESDKLSYPWDGTQSYSLFNVSPSCSSFNSPCRDSVSPPKSLFSQRPQRMRSRSRSFSRHRSCSRSPYSRSRSRSPGSRSSSRSCYYYESSHYRHRTHRNSPLYVRSRSRSPYSRRPRYDSYEEYQHERLKREEYRREYEKRESERAKQRERQRQKAIEERRVIYVGKIRPDTTRTELRDRFEVFGEIEECTVNLRDDGDSYGFITYRYTCDAFAALENGYTLRRSNETDFELYFCGRKQFFKSNYADLDSNSDDFDPASTKSKYDSLDFDSLLKEAQRSLRR

SEQ ID NO: 41 - protein, 786 aa, Homo sapiens
MDEGYFCAALVGEDQPLCPDLPELDLSELDVNDLDTDSFLGGLKWCSDQSEIISNQYNNEPSNIFEKIDEENEANLLAVLTETLDSLPVDEDGLPSFDALTDGDVTTDNEASPSSMPDGTPPPQEAEEPSLLKKLLLAPANTQLSYNECSGLSTQNHANHNHRIRTNPAIVKTENSWSNKAKSICQQQKPQRRPCSELLKYLTTNDDPPHTKPTENRNSSRDKCTSKKKSHTQSQSQHLQAKPTTLSLPLTPESPNDPKGSPFENKTIERTLSVELSGTAGLTPPTTPPHKANQDNPFRASPKLKSSCKTVVPPPSKKPRYSESSGTQGNNSTKKGPEQSELYAQLSKSSVLTGGHEERKTKRPSLRLFGDHDYCQSINSKTEILINISQELQDSRQLENKDVSSDWQGQICSSTDSDQCYLRETLEASKQVSPCSTRKQLQDQEIRAELNKHFGHPSQAVFDDEADKTGELRDSDFSNEQFSKLPMFINSGLAMDGLFDDSEDESDKLSYPWDGTQSYSLFNVSPSCSSFNSPCRDSVSPPKSLFSQRPQRMRSRSRSFSRHRSCSRSPYSRSRSRSPGSRSSSRSCYYYESSHYRHRTHRNSPLYVRSRSRSPYSRRPRYDSYEEYQHERLKREEYRREYEKRESERAKQRERQRQKAIEERRVIYVGKIRPDTTRTELRDRFEVFGEIEECTVNLRDDGDSYGFITYRYTCDAFAALENGYTLRRSNETDFELYFCGRKQFFKSNYADLDSNSDDFDPASTKSKYDSLDFDSLLKEAQRSLRR

SEQ ID NO: 42 - protein, 671 aa, Homo sapiens
MPDGTPPPQEAEEPSLLKKLLLAPANTQLSYNECSGLSTQNHANHNHRIRTNPAIVKTENSWSNKAKSICQQQKPQRRPCSELLKYLTTNDDPPHTKPTENRNSSRDKCTSKKKSHTQSQSQHLQAKPTTLSLPLTPESPNDPKGSPFENKTIERTLSVELSGTAGLTPPTTPPHKANQDNPFRASPKLKSSCKTVVPPPSKKPRYSESSGTQGNNSTKKGPEQSELYAQLSKSSVLTGGHEERKTKRPSLRLFGDHDYCQSINSKTEILINISQELQDSRQLENKDVSSDWQGQICSSTDSDQCYLRETLEASKQVSPCSTRKQLQDQEIRAELNKHFGHPSQAVFDDEADKTGELRDSDFSNEQFSKLPMFINSGLAMDGLFDDSEDESDKLSYPWDGTQSYSLFNVSPSCSSFNSPCRDSVSPPKSLFSQRPQRMRSRSRSFSRHRSCSRSPYSRSRSRSPGSRSSSRSCYYYESSHYRHRTHRNSPLYVRSRSRSPYSRRPRYDSYEEYQHERLKREEYRREYEKRESERAKQRERQRQKAIEERRVIYVGKIRPDTTRTELRDRFEVFGEIEECTVNLRDDGDSYGFITYRYTCDAFAALENGYTLRRSNETDFELYFCGRKQFFKSNYADLDSNSDDFDPASTKSKYDSLDFDSLLKEAQRSLRR

SEQ ID NO: 43 - protein, 801 aa, Homo sapiens
MDETSPRLEEDWKKVLQREAGWQCAALVGEDQPLCPDLPELDLSELDVNDLDTDSFLGGLKWCSDQSEIISNQYNNEPSNIFEKIDEENEANLLAVLTETLDSLPVDEDGLPSFDALTDGDVTTDNEASPSSMPDGTPPPQEAEEPSLLKKLLLAPANTQLSYNECSGLSTQNHANHNHRIRTNPAIVKTENSWSNKAKSICQQQKPQRRPCSELLKYLTTNDDPPHTKPTENRNSSRDKCTSKKKSHTQSQSQHLQAKPTTLSLPLTPESPNDPKGSPFENKTIERTLSVELSGTAGLTPPTTPPHKANQDNPFRASPKLKSSCKTVVPPPSKKPRYSESSGTQGNNSTKKGPEQSELYAQLSKSSVLTGGHEERKTKRPSLRLFGDHDYCQSINSKTEILINISQELQDSRQLENKDVSSDWQGQICSSTDSDQCYLRETLEASKQVSPCSTRKQLQDQEIRAELNKHFGHPSQAVFDDEADKTGELRDSDFSNEQFSKLPMFINSGLAMDGLFDDSEDESDKLSYPWDGTQSYSLFNVSPSCSSFNSPCRDSVSPPKSLFSQRPQRMRSRSRSFSRHRSCSRSPYSRSRSRSPGSRSSSRSCYYYESSHYRHRTHRNSPLYVRSRSRSPYSRRPRYDSYEEYQHERLKREEYRREYEKRESERAKQRERQRQKAIEERRVIYVGKIRPDTTRTELRDRFEVFGEIEECTVNLRDDGYGFITYRYTCDAFAALENGYTLRRSNETDFELYFCGRKQFFKSNYADLDSNSDDFDPASTKSKYDSLDFDSLLKEAQRSLRR

SEQ ID NO: 44 - protein, 99 aa, Homo sapiens
MAWDMCNQDSESVWSDIECAALVGEDQPLCPDLPELDLSELDVNDLDTDSFLGGLKWCSDQSEIISNQYNNEPSNIFEVRTSFGNINFSLSLAWARLTW

SEQ ID NO: 45 - protein, 1023 aa, Homo sapiens
MAGNDCGALLDEELSSFFLNYLADTQGGGSGEEQLYADFPELDLSQLDASDFDSATCFGELQWCPENSETEPNQYSPDDSELFQIDSENEALLAELTKTLDDIPEDDVGLAAFPALDGGDALSCTSASPAPSSAPPSPAPEKPSAPAPEVDELSLLQKLLLATSYPTSSSDTQKEGTAWRQAGLRSKSQRPCVKADSTQDKKAPMMQSQSRSCTELHKHLTSAQCCLQDRGLQPPCLQSPRLPAKEDKEPGEDCPSPQPAPASPRDSLALGRADPGAPVSQEDMQAMVQLIRYMHTYCLPQRKLPPQTPEPLPKACSNPSQQVRSRPWSRHHSKASWAEFSILRELLAQDVLCDVSKPYRLATPVYASLTPRSRPRPPKDSQASPGRPSSVEEVRIAASPKSTGPRPSLRPLRLEVKREVRRPARLQQQEEEDEEEEEEEEEEEKEEEEEWGRKRPGRGLPWTKLGRKLESSVCPVRRSRRLNPELGPWLTFADEPLVPSEPQGALPSLCLAPKAYDVERELGSPTDEDSGQDQQLLRGPQIPALESPCESGCGDMDEDPSCPQLPPRDSPRCLMLALSQSDPTFGKKSFEQTLTVELCGTAGLTPPTTPPYKPTEEDPFKPDIKHSLGKEIALSLPSPEGLSLKATPGAAHKLPKKHPERSELLSHLRHATAQPASQAGQKRPFSCSFGDHDYCQVLRPEGVLQRKVLRSWEPSGVHLEDWPQQGAPWAEAQAPGREEDRSCDAGAPPKDSTLLRDHEIRASLTKHFGLLETALEEEDLASCKSPEYDTVFEDSSSSSGESSFLPEEEEEEGEEEEEDDEEEDSGVSPTCSDHCPYQSPPSKANRQLCSRSRSSSGSSPCHSWSPATRRNFRCESRGPCSDRTPSIRHARKRREKAIGEGRVVYIQNLSSDMSSRELKRRFEVFGEIEECEVLTRNRRGEKYGFITYRCSEHAALSLTKGAALRKRNEPSFQLSYGGLRHFCWPRYTDYDSNSEEALPASGKSKYEAMDFDSLLKEAQQSLH

SEQ ID NO: 46 - protein, 984 aa, Homo sapiens
MAGNDCGALLDEELSSFFLNYLADTQGGGSGEEQLYADFPELDLSQLDASDFDSATCFGELQWCPENSETEPNQYSPDDSELFQIDSENEALLAELTKTLDDIPEDDVGLAAFPALDGGDALSCTSASPAPSSAPPSPAPEKPSAPAPEVDELSLADSTQDKKAPMMQSQSRSCTELHKHLTSAQCCLQDRGLQPPCLQSPRLPAKEDKEPGEDCPSPQPAPASPRDSLALGRADPGAPVSQEDMQAMVQLIRYMHTYCLPQRKLPPQTPEPLPKACSNPSQQVRSRPWSRHHSKASWAEFSILRELLAQDVLCDVSKPYRLATPVYASLTPRSRPRPPKDSQASPGRPSSVEEVRIAASPKSTGPRPSLRPLRLEVKREVRRPARLQQQEEEDEEEEEEEEEEEKEEEEEWGRKRPGRGLPWTKLGRKLESSVCPVRRSRRLNPELGPWLTFADEPLVPSEPQGALPSLCLAPKAYDVERELGSPTDEDSGQDQQLLRGPQIPALESPCESGCGDMDEDPSCPQLPPRDSPRCLMLALSQSDPTFGKKSFEQTLTVELCGTAGLTPPTTPPYKPTEEDPFKPDIKHSLGKEIALSLPSPEGLSLKATPGAAHKLPKKHPERSELLSHLRHATAQPASQAGQKRPFSCSFGDHDYCQVLRPEGVLQRKVLRSWEPSGVHLEDWPQQGAPWAEAQAPGREEDRSCDAGAPPKDSTLLRDHEIRASLTKHFGLLETALEEEDLASCKSPEYDTVFEDSSSSSGESSFLPEEEEEEGEEEEEDDEEEDSGVSPTCSDHCPYQSPPSKANRQLCSRSRSSSGSSPCHSWSPATRRNFRCESRGPCSDRTPSIRHARKRREKAIGEGRVVYIQNLSSDMSSRELKRRFEVFGEIEECEVLTRNRRGEKYGFITYRCSEHAALSLTKGAALRKRNEPSFQLSYGGLRHFCWPRYTDYDSNSEEALPASGKSKYEAMDFDSLLKEAQQSLH

SEQ ID NO: 47 - protein, 959 aa, Homo sapiens
MGGGSGEEQLYADFPELDLSQLDASDFDSATCFGELQWCPENSETEPNQYSPDDSELFQIDSENEALLAELTKTLDDIPEDDVGLAAFPALDGGDALSCTSASPAPSSAPPSPAPEKPSAPAPEVDELSLADSTQDKKAPMMQSQSRSCTELHKHLTSAQCCLQDRGLQPPCLQSPRLPAKEDKEPGEDCPSPQPAPASPRDSLALGRADPGAPVSQEDMQAMVQLIRYMHTYCLPQRKLPPQTPEPLPKACSNPSQQVRSRPWSRHHSKASWAEFSILRELLAQDVLCDVSKPYRLATPVYASLTPRSRPRPPKDSQASPGRPSSVEEVRIAASPKSTGPRPSLRPLRLEVKREVRRPARLQQQEEEDEEEEEEEEEEEKEEEEEWGRKRPGRGLPWTKLGRKLESSVCPVRRSRRLNPELGPWLTFADEPLVPSEPQGALPSLCLAPKAYDVERELGSPTDEDSGQDQQLLRGPQIPALESPCESGCGDMDEDPSCPQLPPRDSPRCLMLALSQSDPTFGKKSFEQTLTVELCGTAGLTPPTTPPYKPTEEDPFKPDIKHSLGKEIALSLPSPEGLSLKATPGAAHKLPKKHPERSELLSHLRHATAQPASQAGQKRPFSCSFGDHDYCQVLRPEGVLQRKVLRSWEPSGVHLEDWPQQGAPWAEAQAPGREEDRSCDAGAPPKDSTLLRDHEIRASLTKHFGLLETALEEEDLASCKSPEYDTVFEDSSSSSGESSFLPEEEEEEGEEEEEDDEEEDSGVSPTCSDHCPYQSPPSKANRQLCSRSRSSSGSSPCHSWSPATRRNFRCESRGPCSDRTPSIRHARKRREKAIGEGRVVYIQNLSSDMSSRELKRRFEVFGEIEECEVLTRNRRGEKYGFITYRCSEHAALSLTKGAALRKRNEPSFQLSYGGLRHFCWPRYTDYDSNSEEALPASGKSKYEAMDFDSLLKEAQQSLH

SEQ ID NO: 48 - protein, 1132 aa, Homo sapiens
MPRAPRCRAVRSLLRSHYREVLPLATFVRRLGPQGWRLVQRGDPAAFRALVAQCLVCVPWDARPPPAAPSFRQVSCLKELVARVLQRLCERGAKNVLAFGFALLDGARGGPPEAFTTSVRSYLPNTVTDALRGSGAWGLLLRRVGDDVLVHLLARCALFVLVAPSCAYQVCGPPLYQLGAATQARPPPHASGPRRRLGCERAWNHSVREAGVPLGLPAPGARRRGGSASRSLPLPKRPRRGAAPEPERTPVGQGSWAHPGRTRGPSDRGFCVVSPARPAEEATSLEGALSGTRHSHPSVGRQHHAGPPSTSRPPRPWDTPCPPVYAETKHFLYSSGDKEQLRPSFLLSSLRPSLTGARRLVETIFLGSRPWMPGTPRRLPRLPQRYWQMRPLFLELLGNHAQCPYGVLLKTHCPLRAAVTPAAGVCAREKPQGSVAAPEEEDTDPRRLVQLLRQHSSPWQVYGFVRACLRRLVPPGLWGSRHNERRFLRNTKKFISLGKHAKLSLQELTWKMSVRDCAWLRRSPGVGCVPAAEHRLREEILAKFLHWLMSVYVVELLRSFFYVTETTFQKNRLFFYRKSVWSKLQSIGIRQHLKRVQLRELSEAEVRQHREARPALLTSRLRFIPKPDGLRPIVNMDYVVGARTFRREKRAERLTSRVKALFSVLNYERARRPGLLGASVLGLDDIHRAWRTFVLRVRAQDPPPELYFVKVDVTGAYDTIPQDRLTEVIASIIKPQNTYCVRRYAVVQKAAHGHVRKAFKSHVSTLTDLQPYMRQFVAHLQETSPLRDAVVIEQSSSLNEASSGLFDVFLRFMCHHAVRIRGKSYVQCQGIPQGSILSTLLCSLCYGDMENKLFAGIRRDGLLLRLVDDFLLVTPHLTHAKTFLRTLVRGVPEYGCVVNLRKTVVNFPVEDEALGGTAFVQMPAHGLFPWCGLLLDTRTLEVQSDYSSYARTSIRASLTFNRGFKAGRNMRRKLFGVLRLKCHSLFLDLQVNSLQTVCTNIYKILLLQAYRFHACVLQLPFHQQVWKNPTFFLRVISDTASLCYSILKAKNAGMSLGAKGAAGPLPSEAVQWLCHQAFLLKLTRHRVTYVPLLGSLRTAQTQLSRKLPGTTLTALEAAANPALPSDFKTILD

SEQ ID NO: 49 - protein, 1069 aa, Homo sapiens
MPRAPRCRAVRSLLRSHYREVLPLATFVRRLGPQGWRLVQRGDPAAFRALVAQCLVCVPWDARPPPAAPSFRQVSCLKELVARVLQRLCERGAKNVLAFGFALLDGARGGPPEAFTTSVRSYLPNTVTDALRGSGAWGLLLRRVGDDVLVHLLARCALFVLVAPSCAYQVCGPPLYQLGAATQARPPPHASGPRRRLGCERAWNHSVREAGVPLGLPAPGARRRGGSASRSLPLPKRPRRGAAPEPERTPVGQGSWAHPGRTRGPSDRGFCVVSPARPAEEATSLEGALSGTRHSHPSVGRQHHAGPPSTSRPPRPWDTPCPPVYAETKHFLYSSGDKEQLRPSFLLSSLRPSLTGARRLVETIFLGSRPWMPGTPRRLPRLPQRYWQMRPLFLELLGNHAQCPYGVLLKTHCPLRAAVTPAAGVCAREKPQGSVAAPEEEDTDPRRLVQLLRQHSSPWQVYGFVRACLRRLVPPGLWGSRHNERRFLRNTKKFISLGKHAKLSLQELTWKMSVRDCAWLRRSPGVGCVPAAEHRLREEILAKFLHWLMSVYVVELLRSFFYVTETTFQKNRLFFYRKSVWSKLQSIGIRQHLKRVQLRELSEAEVRQHREARPALLTSRLRFIPKPDGLRPIVNMDYVVGARTFRREKRAERLTSRVKALFSVLNYERARRPGLLGASVLGLDDIHRAWRTFVLRVRAQDPPPELYFVKVDVTGAYDTIPQDRLTEVIASIIKPQNTYCVRRYAVVQKAAHGHVRKAFKSHVSTLTDLQPYMRQFVAHLQETSPLRDAVVIEQSSSLNEASSGLFDVFLRFMCHHAVRIRGKSYVQCQGIPQGSILSTLLCSLCYGDMENKLFAGIRRDGLLLRLVDDFLLVTPHLTHAKTFLSYARTSIRASLTFNRGFKAGRNMRRKLFGVLRLKCHSLFLDLQVNSLQTVCTNIYKILLLQAYRFHACVLQLPFHQQVWKNPTFFLRVISDTASLCYSILKAKNAGMSLGAKGAAGPLPSEAVQWLCHQAFLLKLTRHRVTYVPLLGSLRTAQTQLSRKLPGTTLTALEAAANPALPSDFKTILD

SEQ ID NO: 50 - protein, 199 aa, Streptomyces alboniger
MTEYKPTVRLATRDDVPRAVRTLAAAFADYPATRHTVDPDRHIERVTELQELFLTRVGLDIGKVWVADDGAAVAVWTTPESVEAGAVFAEIGPRMAELSGSRLAAQQQMEGLLAPHRPKEPAWFLATVGVSPDHQGKGLGSAVVLPGVEAAERAGVPAFLETSAPRNLPFYERLGFTVTADVEVPEGPRTWCMTRKPGA

SEQ ID NO: 51 - protein, 286 aa, Escherichia coli
MSIQHFRVALIPFFAAFCLPVFAHPETLVKVKDAEDQLGARVGYIELDLNSGKILESFRPEERFPMMSTFKVLLCGAVLSRIDAGQEQLGRRIHYSQNDLVEYSPVTEKHLTDGMTVRELCSAAITMSDNTAANLLLTTIGGPKELTAFLHNMGDHVTRLDRWEPELNEAIPNDERDTTMPVAMATTLRKLLTGELLTLASRQQLIDWMEADKVAGPLLRSALPAGWFIADKSGAGERGSRGIIAALGPDGKPSRIVVIYTTGSQATMDERNRQIAEIGASLIKHW

SEQ ID NO: 52 - protein, 239 aa, synthetic construct
MVSKGEELFTGVVPILVELDGDVNGHKFSVSGEGEGDATYGKLTLKFICTTGKLPVPWPTLVTTLTYGVQCFSRYPDHMKQHDFFKSAMPEGYVQERTIFFKDDGNYKTRAEVKFEGDTLVNRIELKGIDFKEDGNILGHKLEYNYNSHNVYIMADKQKNGIKVNFKIRHNIEDGSVQLADHYQQNTPIGDGPVLLPDNHYLSTQSALSKDPNEKRDHMVLLEFVTAAGITLGMDELYK

SEQ ID NO: 53 - protein, 550 aa, Photinus pyralis
MEDAKNIKKGPAPFYPLEDGTAGEQLHKAMKRYALVPGTIAFTDAHIEVNITYAEYFEMSVRLAEAMKRYGLNTNHRIVVCSENSLQFFMPVLGALFIGVAVAPANDIYNERELLNSMNISQPTVVFVSKKGLQKILNVQKKLPIIQKIIIMDSKTDYQGFQSMYTFVTSHLPPGFNEYDFVPESFDRDKTIALIMNSSGSTGLPKGVALPHRTACVRFSHARDPIFGNQIIPDTAILSVVPFHHGFGMFTTLGYLICGFRVVLMYRFEEELFLRSLQDYKIQSALLVPTLFSFFAKSTLIDKYDLSNLHEIASGGAPLSKEVGEAVAKRFHLPGIRQGYGLTETTSAILITPEGDDKPGAVGKVVPFFEAKVVDLDTGKTLGVNQRGELCVRGPMIMSGYVNNPEATNALIDKDGWLHSGDIAYWDEDEHFFIVDRLKSLIKYKGYQVAPAELESILLQHPNIFDAGVAGLPDDDAGELPAAVVVLEHGKTMTEKEIVDYVASQVTTAKKLRGGVVFVDEVPKGLTGKLDARKIREILIKAKKGGKSKL

SEQ ID NO: 54 - protein, 236 aa, synthetic construct
MVSKGEEDNMAIIKEFMRFKVHMEGSVNGHEFEIEGEGEGRPYEGTQTAKLKVTKGGPLPFAWDILSPQFMYGSKAYVKHPADIPDYLKLSFPEGFKWERVMNFEDGGVVTVTQDSSLQDGEFIYKVKLRGTNFPSDGPVMQKKTMGWEASSERMYPEDGALKGEIKQRLKLKDGGHYDAEVKTTYKAKKPVQLPGAYNVNIKLDITSHNEDYTIVEQYERAEGRHSTGGMDELYK

SEQ ID NO: 55 - protein, 594 aa, Trichoplusia ni
MGSSLDDEHILSALLQSDDELVGEDSDSEISDHVSEDDVQSDTEEAFIDEVHEVQPTSSGSEILDEQNVIEQPGSSLASNRILTLPQRTIRGKNKHCWSTSKSTRRSRVSALNIVRSQRGPTRMCRNIYDPLLCFKLFFTDEIISEIVKWTNAEISLKRRESMTGATFRDTNEDEIYAFFGILVMTAVRKDNHMSTDDLFDRSLSMVYVSVMSRDRFDFLIRCLRMDDKSIRPTLRENDVFTPVRKIWDLFIHQCIQNYTPGAHLTIDEQLLGFRGRCPFRMYIPNKPSKYGIKILMMCDSGTKYMINGMPYLGRGTQTNGVPLGEYYVKELSKPVHGSCRNITCDNWFTSIPLAKNLLQEPYKLTIVGTVRSNKREIPEVLKNSRSRPVGTSMFCFDGPLTLVSYKPKPAKMVYLLSSCDEDASINESTGKPQMVMYYNQTKGGVDTLDQMCSVMTCSRKTNRWPMALLYGMINIACINSFIIYSHNVSSKGEKVQSRKKFMRNLYMSLTSSFMRKRLEAPTLKRYLRDNISNILPNEVPGTSDDSTEEPVMKKRTYCTYCPSKIRRKANASCKKCKKVICREHNIDMCQSCF

SEQ ID NO: 56 - protein, 594 aa, synthetic construct
MGSSLDDEHILSALLQSDDELVGEDSDSEVSDHVSEDDVQSDTEEAFIDEVHEVQPTSSGSEILDEQNVIEQPGSSLASNRILTLPQRTIRGKNKHCWSTSKPTRRSRVSALNIVRSQRGPTRMCRNIYDPLLCFKLFFTDEIISEIVKWTNAEISLKRRESMTSATFRDTNEDEIYAFFGILVMTAVRKDNHMSTDDLFDRSLSMVYVSVMSRDRFDFLIRCLRMDDKSIRPTLRENDVFTPVRKIWDLFIHQCIQNYTPGAHLTIDEQLLGFRGRCPFRVYIPNKPSKYGIKILMMCDSGTKYMINGMPYLGRGTQTNGVPLGEYYVKELSKPVHGSCRNITCDNWFTSIPLAKNLLQEPYKLTIVGTVRSNKREIPEVLKNSRSRPVGTSMFCFDGPLTLVSYKPKPAKMVYLLSSCDEDASINESTGKPQMVMYYNQTKGGVDTLDQMCSVMTCSRKTNRWPMALLYGMINIACINSFIIYSHNVSSKGEKVQSRKKFMRNLYMGLTSSFMRKRLEAPTLKRYLRDNISNILPKEVPGTSDDSTEEPVMKKRTYCTYCPSKIRRKASASCKKCKKVICREHNIDMCQSCF